European Patent Application EP 4 722 230 A1, published April 8, 2026. Title: CORONAVIRUS VACCINE COMPOSITION, METHOD AND USE THEREOF. Applicant: Sichuan Clover Biopharmaceuticals, Inc. The sequence listing filed with the application follows.

SEQUENCE LISTING (127 sequences)

SEQ ID NO: 1 - protein, 1509 aa, synthetic construct
  source 1..1509: note; note (original language) = Hu-1 SARS-CoV-2 S-trimer fusion polypeptide without signal peptide, 1509 aa; organism (original language) = Synthetic construct
QCVNLTTRTQLPPAYTNSFTRGVYYPDKVFRSSVLHSTQDLFLPFFSNVTWFHAIHVSGTNGTKRFDNPVLPFNDGVYFASTEKSNIIRGWIFGTTLDSKTQSLLIVNNATNVVIKVCEFQFCNDPFLGVYYHKNNKSWMESEFRVYSSANNCTFEYVSQPFLMDLEGKQGNFKNLREFVFKNIDGYFKIYSKHTPINLVRDLPQGFSALEPLVDLPIGINITRFQTLLALHRSYLTPGDSSSGWTAGAAAYYVGYLQPRTFLLKYNENGTITDAVDCALDPLSETKCTLKSFTVEKGIYQTSNFRVQPTESIVRFPNITNLCPFGEVFNATRFASVYAWNRKRISNCVADYSVLYNSASFSTFKCYGVSPTKLNDLCFTNVYADSFVIRGDEVRQIAPGQTGKIADYNYKLPDDFTGCVIAWNSNNLDSKVGGNYNYLYRLFRKSNLKPFERDISTEIYQAGSTPCNGVEGFNCYFPLQSYGFQPTNGVGYQPYRVVVLSFELLHAPATVCGPKKSTNLVKNKCVNFNFNGLTGTGVLTESNKKFLPFQQFGRDIADTTDAVRDPQTLEILDITPCSFGGVSVITPGTNTSNQVAVLYQDVNCTEVPVAIHADQLTPTWRVYSTGSNVFQTRAGCLIGAEHVNNSYECDIPIGAGICASYQTQTNSPRRARSVASQSIIAYTMSLGAENSVAYSNNSIAIPTNFTISVTTEILPVSMTKTSVDCTMYICGDSTECSNLLLQYGSFCTQLNRALTGIAVEQDKNTQEVFAQVKQIYKTPPIKDFGGFNFSQILPDPSKPSKRSFIEDLLFNKVTLADAGFIKQYGDCLGDIAARDLICAQKFNGLTVLPPLLTDEMIAQYTSALLAGTITSGWTFGAGAALQIPFAMQMAYRFNGIGVTQNVLYENQKLIANQFNSAIGKIQDSLSSTASALGKLQDVVNQNAQALNTLVKQLSSNFGAISSVLNDILSRLDKVEAEVQIDRLITGRLQSLQTYVTQQLIRAAEIRASANLAATKMSECVLGQSKRVDFCGKGYHLMSFPQSAPHGVVFLHVTYVPAQEKNFTTAPAICHDGKAHFPREGVFVSNGTHWFVTQRNFYEPQIITTDNTFVSGNCDVVIGIVNNTVYDPLQPELDSFKEELDKYFKNHTSPDVDLGDISGINASVVNIQKEIDRLNEVAKNLNESLIDLQELGKYEQYIKRSNGLPGPIGPPGPRGRTGDAGPVGPPGPPGPPGPPGPPSAGFDFSFLPQPPQEKAHDGGRYYRANDANVVRDRDLEVDTTLKSLSQQIENIRSPEGSRKNPARTCRDLKMCHSDWKSGEYWIDPNQGCNLDAIKVFCNMETGETCVYPTQPSVAQKNWYISKNPKDKRHVWFGESMTDGFQFEYGGQGSDPADVAIQLTFLRLMSTEASQNITYHCKNSVAYMDQQTGNLKKALLLQGSNEIEIRAEGNSRFTYSVTVDGCTSHTGAWGKTVIEYKTTKTSRLPIIDVAPLDVGAPDQEFGFDVGPVCFL

SEQ ID NO: 2 - protein, 1509 aa, synthetic construct
  source 1..1509: note; note (original language) = Hu-1 SARS-CoV-2 spike S-trimer fusion polypeptide without signal peptide, 1509 aa, S1/S2 furin cleavage site 1 mutant (685R→685A); organism (original language) = Synthetic construct
QCVNLTTRTQLPPAYTNSFTRGVYYPDKVFRSSVLHSTQDLFLPFFSNVTWFHAIHVSGTNGTKRFDNPVLPFNDGVYFASTEKSNIIRGWIFGTTLDSKTQSLLIVNNATNVVIKVCEFQFCNDPFLGVYYHKNNKSWMESEFRVYSSANNCTFEYVSQPFLMDLEGKQGNFKNLREFVFKNIDGYFKIYSKHTPINLVRDLPQGFSALEPLVDLPIGINITRFQTLLALHRSYLTPGDSSSGWTAGAAAYYVGYLQPRTFLLKYNENGTITDAVDCALDPLSETKCTLKSFTVEKGIYQTSNFRVQPTESIVRFPNITNLCPFGEVFNATRFASVYAWNRKRISNCVADYSVLYNSASFSTFKCYGVSPTKLNDLCFTNVYADSFVIRGDEVRQIAPGQTGKIADYNYKLPDDFTGCVIAWNSNNLDSKVGGNYNYLYRLFRKSNLKPFERDISTEIYQAGSTPCNGVEGFNCYFPLQSYGFQPTNGVGYQPYRVVVLSFELLHAPATVCGPKKSTNLVKNKCVNFNFNGLTGTGVLTESNKKFLPFQQFGRDIADTTDAVRDPQTLEILDITPCSFGGVSVITPGTNTSNQVAVLYQDVNCTEVPVAIHADQLTPTWRVYSTGSNVFQTRAGCLIGAEHVNNSYECDIPIGAGICASYQTQTNSPRRAASVASQSIIAYTMSLGAENSVAYSNNSIAIPTNFTISVTTEILPVSMTKTSVDCTMYICGDSTECSNLLLQYGSFCTQLNRALTGIAVEQDKNTQEVFAQVKQIYKTPPIKDFGGFNFSQILPDPSKPSKRSFIEDLLFNKVTLADAGFIKQYGDCLGDIAARDLICAQKFNGLTVLPPLLTDEMIAQYTSALLAGTITSGWTFGAGAALQIPFAMQMAYRFNGIGVTQNVLYENQKLIANQFNSAIGKIQDSLSSTASALGKLQDVVNQNAQALNTLVKQLSSNFGAISSVLNDILSRLDKVEAEVQIDRLITGRLQSLQTYVTQQLIRAAEIRASANLAATKMSECVLGQSKRVDFCGKGYHLMSFPQSAPHGVVFLHVTYVPAQEKNFTTAPAICHDGKAHFPREGVFVSNGTHWFVTQRNFYEPQIITTDNTFVSGNCDVVIGIVNNTVYDPLQPELDSFKEELDKYFKNHTSPDVDLGDISGINASVVNIQKEIDRLNEVAKNLNESLIDLQELGKYEQYIKRSNGLPGPIGPPGPRGRTGDAGPVGPPGPPGPPGPPGPPSAGFDFSFLPQPPQEKAHDGGRYYRANDANVVRDRDLEVDTTLKSLSQQIENIRSPEGSRKNPARTCRDLKMCHSDWKSGEYWIDPNQGCNLDAIKVFCNMETGETCVYPTQPSVAQKNWYISKNPKDKRHVWFGESMTDGFQFEYGGQGSDPADVAIQLTFLRLMSTEASQNITYHCKNSVAYMDQQTGNLKKALLLQGSNEIEIRAEGNSRFTYSVTVDGCTSHTGAWGKTVIEYKTTKTSRLPIIDVAPLDVGAPDQEFGFDVGPVCFL

SEQ ID NO: 3 - protein, 1509 aa, synthetic construct
  source 1..1509: note; note (original language) = Hu-1 SARS-CoV-2 S-trimer fusion polypeptide without signal peptide, 1509 aa, proline mutant (986K/987V→986P/987P); organism (original language) = Synthetic construct
QCVNLTTRTQLPPAYTNSFTRGVYYPDKVFRSSVLHSTQDLFLPFFSNVTWFHAIHVSGTNGTKRFDNPVLPFNDGVYFASTEKSNIIRGWIFGTTLDSKTQSLLIVNNATNVVIKVCEFQFCNDPFLGVYYHKNNKSWMESEFRVYSSANNCTFEYVSQPFLMDLEGKQGNFKNLREFVFKNIDGYFKIYSKHTPINLVRDLPQGFSALEPLVDLPIGINITRFQTLLALHRSYLTPGDSSSGWTAGAAAYYVGYLQPRTFLLKYNENGTITDAVDCALDPLSETKCTLKSFTVEKGIYQTSNFRVQPTESIVRFPNITNLCPFGEVFNATRFASVYAWNRKRISNCVADYSVLYNSASFSTFKCYGVSPTKLNDLCFTNVYADSFVIRGDEVRQIAPGQTGKIADYNYKLPDDFTGCVIAWNSNNLDSKVGGNYNYLYRLFRKSNLKPFERDISTEIYQAGSTPCNGVEGFNCYFPLQSYGFQPTNGVGYQPYRVVVLSFELLHAPATVCGPKKSTNLVKNKCVNFNFNGLTGTGVLTESNKKFLPFQQFGRDIADTTDAVRDPQTLEILDITPCSFGGVSVITPGTNTSNQVAVLYQDVNCTEVPVAIHADQLTPTWRVYSTGSNVFQTRAGCLIGAEHVNNSYECDIPIGAGICASYQTQTNSPRRARSVASQSIIAYTMSLGAENSVAYSNNSIAIPTNFTISVTTEILPVSMTKTSVDCTMYICGDSTECSNLLLQYGSFCTQLNRALTGIAVEQDKNTQEVFAQVKQIYKTPPIKDFGGFNFSQILPDPSKPSKRSFIEDLLFNKVTLADAGFIKQYGDCLGDIAARDLICAQKFNGLTVLPPLLTDEMIAQYTSALLAGTITSGWTFGAGAALQIPFAMQMAYRFNGIGVTQNVLYENQKLIANQFNSAIGKIQDSLSSTASALGKLQDVVNQNAQALNTLVKQLSSNFGAISSVLNDILSRLDPPEAEVQIDRLITGRLQSLQTYVTQQLIRAAEIRASANLAATKMSECVLGQSKRVDFCGKGYHLMSFPQSAPHGVVFLHVTYVPAQEKNFTTAPAICHDGKAHFPREGVFVSNGTHWFVTQRNFYEPQIITTDNTFVSGNCDVVIGIVNNTVYDPLQPELDSFKEELDKYFKNHTSPDVDLGDISGINASVVNIQKEIDRLNEVAKNLNESLIDLQELGKYEQYIKRSNGLPGPIGPPGPRGRTGDAGPVGPPGPPGPPGPPGPPSAGFDFSFLPQPPQEKAHDGGRYYRANDANVVRDRDLEVDTTLKSLSQQIENIRSPEGSRKNPARTCRDLKMCHSDWKSGEYWIDPNQGCNLDAIKVFCNMETGETCVYPTQPSVAQKNWYISKNPKDKRHVWFGESMTDGFQFEYGGQGSDPADVAIQLTFLRLMSTEASQNITYHCKNSVAYMDQQTGNLKKALLLQGSNEIEIRAEGNSRFTYSVTVDGCTSHTGAWGKTVIEYKTTKTSRLPIIDVAPLDVGAPDQEFGFDVGPVCFL

SEQ ID NO: 4 - protein, 1509 aa, synthetic construct
  source 1..1509: note; note (original language) = Hu-1 SARS-CoV-2 S-trimer fusion polypeptide without signal peptide, 1509 aa, S1/S2 furin cleavage site 1 and proline mutant (685R→685A, 986K/987V→986P/987P); organism (original language) = Synthetic construct
QCVNLTTRTQLPPAYTNSFTRGVYYPDKVFRSSVLHSTQDLFLPFFSNVTWFHAIHVSGTNGTKRFDNPVLPFNDGVYFASTEKSNIIRGWIFGTTLDSKTQSLLIVNNATNVVIKVCEFQFCNDPFLGVYYHKNNKSWMESEFRVYSSANNCTFEYVSQPFLMDLEGKQGNFKNLREFVFKNIDGYFKIYSKHTPINLVRDLPQGFSALEPLVDLPIGINITRFQTLLALHRSYLTPGDSSSGWTAGAAAYYVGYLQPRTFLLKYNENGTITDAVDCALDPLSETKCTLKSFTVEKGIYQTSNFRVQPTESIVRFPNITNLCPFGEVFNATRFASVYAWNRKRISNCVADYSVLYNSASFSTFKCYGVSPTKLNDLCFTNVYADSFVIRGDEVRQIAPGQTGKIADYNYKLPDDFTGCVIAWNSNNLDSKVGGNYNYLYRLFRKSNLKPFERDISTEIYQAGSTPCNGVEGFNCYFPLQSYGFQPTNGVGYQPYRVVVLSFELLHAPATVCGPKKSTNLVKNKCVNFNFNGLTGTGVLTESNKKFLPFQQFGRDIADTTDAVRDPQTLEILDITPCSFGGVSVITPGTNTSNQVAVLYQDVNCTEVPVAIHADQLTPTWRVYSTGSNVFQTRAGCLIGAEHVNNSYECDIPIGAGICASYQTQTNSPRRAASVASQSIIAYTMSLGAENSVAYSNNSIAIPTNFTISVTTEILPVSMTKTSVDCTMYICGDSTECSNLLLQYGSFCTQLNRALTGIAVEQDKNTQEVFAQVKQIYKTPPIKDFGGFNFSQILPDPSKPSKRSFIEDLLFNKVTLADAGFIKQYGDCLGDIAARDLICAQKFNGLTVLPPLLTDEMIAQYTSALLAGTITSGWTFGAGAALQIPFAMQMAYRFNGIGVTQNVLYENQKLIANQFNSAIGKIQDSLSSTASALGKLQDVVNQNAQALNTLVKQLSSNFGAISSVLNDILSRLDPPEAEVQIDRLITGRLQSLQTYVTQQLIRAAEIRASANLAATKMSECVLGQSKRVDFCGKGYHLMSFPQSAPHGVVFLHVTYVPAQEKNFTTAPAICHDGKAHFPREGVFVSNGTHWFVTQRNFYEPQIITTDNTFVSGNCDVVIGIVNNTVYDPLQPELDSFKEELDKYFKNHTSPDVDLGDISGINASVVNIQKEIDRLNEVAKNLNESLIDLQELGKYEQYIKRSNGLPGPIGPPGPRGRTGDAGPVGPPGPPGPPGPPGPPSAGFDFSFLPQPPQEKAHDGGRYYRANDANVVRDRDLEVDTTLKSLSQQIENIRSPEGSRKNPARTCRDLKMCHSDWKSGEYWIDPNQGCNLDAIKVFCNMETGETCVYPTQPSVAQKNWYISKNPKDKRHVWFGESMTDGFQFEYGGQGSDPADVAIQLTFLRLMSTEASQNITYHCKNSVAYMDQQTGNLKKALLLQGSNEIEIRAEGNSRFTYSVTVDGCTSHTGAWGKTVIEYKTTKTSRLPIIDVAPLDVGAPDQEFGFDVGPVCFL

SEQ ID NO: 5 - protein, 836 aa, synthetic construct
  source 1..836: note; note (original language) = Hu-1 SARS-CoV-2 spike NTD/RBD-trimeric fusion protein without fusion peptide, 836 aa; organism (original language) = Synthetic construct
QCVNLTTRTQLPPAYTNSFTRGVYYPDKVFRSSVLHSTQDLFLPFFSNVTWFHAIHVSGTNGTKRFDNPVLPFNDGVYFASTEKSNIIRGWIFGTTLDSKTQSLLIVNNATNVVIKVCEFQFCNDPFLGVYYHKNNKSWMESEFRVYSSANNCTFEYVSQPFLMDLEGKQGNFKNLREFVFKNIDGYFKIYSKHTPINLVRDLPQGFSALEPLVDLPIGINITRFQTLLALHRSYLTPGDSSSGWTAGAAAYYVGYLQPRTFLLKYNENGTITDAVDCALDPLSETKCTLKSFTVEKGIYQTSNFRVQPTESIVRFPNITNLCPFGEVFNATRFASVYAWNRKRISNCVADYSVLYNSASFSTFKCYGVSPTKLNDLCFTNVYADSFVIRGDEVRQIAPGQTGKIADYNYKLPDDFTGCVIAWNSNNLDSKVGGNYNYLYRLFRKSNLKPFERDISTEIYQAGSTPCNGVEGFNCYFPLQSYGFQPTNGVGYQPYRVVVLSFELLHAPATVCGPKKSTNLVKNKCRSNGLPGPIGPPGPRGRTGDAGPVGPPGPPGPPGPPGPPSAGFDFSFLPQPPQEKAHDGGRYYRANDANVVRDRDLEVDTTLKSLSQQIENIRSPEGSRKNPARTCRDLKMCHSDWKSGEYWIDPNQGCNLDAIKVFCNMETGETCVYPTQPSVAQKNWYISKNPKDKRHVWFGESMTDGFQFEYGGQGSDPADVAIQLTFLRLMSTEASQNITYHCKNSVAYMDQQTGNLKKALLLQGSNEIEIRAEGNSRFTYSVTVDGCTSHTGAWGKTVIEYKTTKTSRLPIIDVAPLDVGAPDQEFGFDVGPVCFL

SEQ ID NO: 6 - protein, 979 aa, synthetic construct
  source 1..979: note; note (original language) = Hu-1 SARS-CoV-2 spike S1-trimer fusion polypeptide without signal peptide, 979 aa; organism (original language) = Synthetic construct
QCVNLTTRTQLPPAYTNSFTRGVYYPDKVFRSSVLHSTQDLFLPFFSNVTWFHAIHVSGTNGTKRFDNPVLPFNDGVYFASTEKSNIIRGWIFGTTLDSKTQSLLIVNNATNVVIKVCEFQFCNDPFLGVYYHKNNKSWMESEFRVYSSANNCTFEYVSQPFLMDLEGKQGNFKNLREFVFKNIDGYFKIYSKHTPINLVRDLPQGFSALEPLVDLPIGINITRFQTLLALHRSYLTPGDSSSGWTAGAAAYYVGYLQPRTFLLKYNENGTITDAVDCALDPLSETKCTLKSFTVEKGIYQTSNFRVQPTESIVRFPNITNLCPFGEVFNATRFASVYAWNRKRISNCVADYSVLYNSASFSTFKCYGVSPTKLNDLCFTNVYADSFVIRGDEVRQIAPGQTGKIADYNYKLPDDFTGCVIAWNSNNLDSKVGGNYNYLYRLFRKSNLKPFERDISTEIYQAGSTPCNGVEGFNCYFPLQSYGFQPTNGVGYQPYRVVVLSFELLHAPATVCGPKKSTNLVKNKCVNFNFNGLTGTGVLTESNKKFLPFQQFGRDIADTTDAVRDPQTLEILDITPCSFGGVSVITPGTNTSNQVAVLYQDVNCTEVPVAIHADQLTPTWRVYSTGSNVFQTRAGCLIGAEHVNNSYECDIPIGAGICASYQTQTNSPRSNGLPGPIGPPGPRGRTGDAGPVGPPGPPGPPGPPGPPSAGFDFSFLPQPPQEKAHDGGRYYRANDANVVRDRDLEVDTTLKSLSQQIENIRSPEGSRKNPARTCRDLKMCHSDWKSGEYWIDPNQGCNLDAIKVFCNMETGETCVYPTQPSVAQKNWYISKNPKDKRHVWFGESMTDGFQFEYGGQGSDPADVAIQLTFLRLMSTEASQNITYHCKNSVAYMDQQTGNLKKALLLQGSNEIEIRAEGNSRFTYSVTVDGCTSHTGAWGKTVIEYKTTKTSRLPIIDVAPLDVGAPDQEFGFDVGPVCFL

SEQ ID NO: 7 - protein, 837 aa, synthetic construct
  source 1..837: note; note (original language) = Hu-1 SARS-CoV-2 spike S2-trimer fusion polypeptide, 837 aa (cleaved at site 1, S1/S2); organism (original language) = Synthetic construct
SVASQSIIAYTMSLGAENSVAYSNNSIAIPTNFTISVTTEILPVSMTKTSVDCTMYICGDSTECSNLLLQYGSFCTQLNRALTGIAVEQDKNTQEVFAQVKQIYKTPPIKDFGGFNFSQILPDPSKPSKRSFIEDLLFNKVTLADAGFIKQYGDCLGDIAARDLICAQKFNGLTVLPPLLTDEMIAQYTSALLAGTITSGWTFGAGAALQIPFAMQMAYRFNGIGVTQNVLYENQKLIANQFNSAIGKIQDSLSSTASALGKLQDVVNQNAQALNTLVKQLSSNFGAISSVLNDILSRLDKVEAEVQIDRLITGRLQSLQTYVTQQLIRAAEIRASANLAATKMSECVLGQSKRVDFCGKGYHLMSFPQSAPHGVVFLHVTYVPAQEKNFTTAPAICHDGKAHFPREGVFVSNGTHWFVTQRNFYEPQIITTDNTFVSGNCDVVIGIVNNTVYDPLQPELDSFKEELDKYFKNHTSPDVDLGDISGINASVVNIQKEIDRLNEVAKNLNESLIDLQELGKYEQYIKRSNGLPGPIGPPGPRGRTGDAGPVGPPGPPGPPGPPGPPSAGFDFSFLPQPPQEKAHDGGRYYRANDANVVRDRDLEVDTTLKSLSQQIENIRSPEGSRKNPARTCRDLKMCHSDWKSGEYWIDPNQGCNLDAIKVFCNMETGETCVYPTQPSVAQKNWYISKNPKDKRHVWFGESMTDGFQFEYGGQGSDPADVAIQLTFLRLMSTEASQNITYHCKNSVAYMDQQTGNLKKALLLQGSNEIEIRAEGNSRFTYSVTVDGCTSHTGAWGKTVIEYKTTKTSRLPIIDVAPLDVGAPDQEFGFDVGPVCFL

SEQ ID NO: 8 - protein, 827 aa, synthetic construct
  source 1..827: note; note (original language) = Hu-1 SARS-CoV-2 spike S2-trimer fusion polypeptide, 827 aa (cleaved at site 2, S1/S2); organism (original language) = Synthetic construct
TMSLGAENSVAYSNNSIAIPTNFTISVTTEILPVSMTKTSVDCTMYICGDSTECSNLLLQYGSFCTQLNRALTGIAVEQDKNTQEVFAQVKQIYKTPPIKDFGGFNFSQILPDPSKPSKRSFIEDLLFNKVTLADAGFIKQYGDCLGDIAARDLICAQKFNGLTVLPPLLTDEMIAQYTSALLAGTITSGWTFGAGAALQIPFAMQMAYRFNGIGVTQNVLYENQKLIANQFNSAIGKIQDSLSSTASALGKLQDVVNQNAQALNTLVKQLSSNFGAISSVLNDILSRLDKVEAEVQIDRLITGRLQSLQTYVTQQLIRAAEIRASANLAATKMSECVLGQSKRVDFCGKGYHLMSFPQSAPHGVVFLHVTYVPAQEKNFTTAPAICHDGKAHFPREGVFVSNGTHWFVTQRNFYEPQIITTDNTFVSGNCDVVIGIVNNTVYDPLQPELDSFKEELDKYFKNHTSPDVDLGDISGINASVVNIQKEIDRLNEVAKNLNESLIDLQELGKYEQYIKRSNGLPGPIGPPGPRGRTGDAGPVGPPGPPGPPGPPGPPSAGFDFSFLPQPPQEKAHDGGRYYRANDANVVRDRDLEVDTTLKSLSQQIENIRSPEGSRKNPARTCRDLKMCHSDWKSGEYWIDPNQGCNLDAIKVFCNMETGETCVYPTQPSVAQKNWYISKNPKDKRHVWFGESMTDGFQFEYGGQGSDPADVAIQLTFLRLMSTEASQNITYHCKNSVAYMDQQTGNLKKALLLQGSNEIEIRAEGNSRFTYSVTVDGCTSHTGAWGKTVIEYKTTKTSRLPIIDVAPLDVGAPDQEFGFDVGPVCFL

SEQ ID NO: 9 - protein, 707 aa, synthetic construct
  source 1..707: note; note (original language) = Hu-1 SARS-CoV-2 spike S2-trimer fusion polypeptide, 707 aa (cleaved at S2'); organism (original language) = Synthetic construct
SFIEDLLFNKVTLADAGFIKQYGDCLGDIAARDLICAQKFNGLTVLPPLLTDEMIAQYTSALLAGTITSGWTFGAGAALQIPFAMQMAYRFNGIGVTQNVLYENQKLIANQFNSAIGKIQDSLSSTASALGKLQDVVNQNAQALNTLVKQLSSNFGAISSVLNDILSRLDKVEAEVQIDRLITGRLQSLQTYVTQQLIRAAEIRASANLAATKMSECVLGQSKRVDFCGKGYHLMSFPQSAPHGVVFLHVTYVPAQEKNFTTAPAICHDGKAHFPREGVFVSNGTHWFVTQRNFYEPQIITTDNTFVSGNCDVVIGIVNNTVYDPLQPELDSFKEELDKYFKNHTSPDVDLGDISGINASVVNIQKEIDRLNEVAKNLNESLIDLQELGKYEQYIKRSNGLPGPIGPPGPRGRTGDAGPVGPPGPPGPPGPPGPPSAGFDFSFLPQPPQEKAHDGGRYYRANDANVVRDRDLEVDTTLKSLSQQIENIRSPEGSRKNPARTCRDLKMCHSDWKSGEYWIDPNQGCNLDAIKVFCNMETGETCVYPTQPSVAQKNWYISKNPKDKRHVWFGESMTDGFQFEYGGQGSDPADVAIQLTFLRLMSTEASQNITYHCKNSVAYMDQQTGNLKKALLLQGSNEIEIRAEGNSRFTYSVTVDGCTSHTGAWGKTVIEYKTTKTSRLPIIDVAPLDVGAPDQEFGFDVGPVCFL

SEQ ID NO: 10 - protein, 1509 aa, synthetic construct
  source 1..1509: note; note (original language) = SARS-CoV-2 South African variant B.1.351 S-trimer fusion polypeptide without signal peptide, 1509 aa; organism (original language) = Synthetic construct
QCVNLTTRTQLPPAYTNSFTRGVYYPDKVFRSSVLHSTQDLFLPFFSNVTWFHAIHVSGTNGTKRFDNPVLPFNDGVYFASTEKSNIIRGWIFGTTLDSKTQSLLIVNNATNVVIKVCEFQFCNDPFLGVYYHKNNKSWMESEFRVYSSANNCTFEYVSQPFLMDLEGKQGNFKNLREFVFKNIDGYFKIYSKHTPINLVRDLPQGFSALEPLVDLPIGINITRFQTLLALHRSYLTPGDSSSGWTAGAAAYYVGYLQPRTFLLKYNENGTITDAVDCALDPLSETKCTLKSFTVEKGIYQTSNFRVQPTESIVRFPNITNLCPFGEVFNATRFASVYAWNRKRISNCVADYSVLYNSASFSTFKCYGVSPTKLNDLCFTNVYADSFVIRGDEVRQIAPGQTGNIADYNYKLPDDFTGCVIAWNSNNLDSKVGGNYNYLYRLFRKSNLKPFERDISTEIYQAGSTPCNGVKGFNCYFPLQSYGFQPTYGVGYQPYRVVVLSFELLHAPATVCGPKKSTNLVKNKCVNFNFNGLTGTGVLTESNKKFLPFQQFGRDIADTTDAVRDPQTLEILDITPCSFGGVSVITPGTNTSNQVAVLYQGVNCTEVPVAIHADQLTPTWRVYSTGSNVFQTRAGCLIGAEHVNNSYECDIPIGAGICASYQTQTNSPRRARSVASQSIIAYTMSLGAENSVAYSNNSIAIPTNFTISVTTEILPVSMTKTSVDCTMYICGDSTECSNLLLQYGSFCTQLNRALTGIAVEQDKNTQEVFAQVKQIYKTPPIKDFGGFNFSQILPDPSKPSKRSFIEDLLFNKVTLADAGFIKQYGDCLGDIAARDLICAQKFNGLTVLPPLLTDEMIAQYTSALLAGTITSGWTFGAGAALQIPFAMQMAYRFNGIGVTQNVLYENQKLIANQFNSAIGKIQDSLSSTASALGKLQDVVNQNAQALNTLVKQLSSNFGAISSVLNDILSRLDKVEAEVQIDRLITGRLQSLQTYVTQQLIRAAEIRASANLAATKMSECVLGQSKRVDFCGKGYHLMSFPQSAPHGVVFLHVTYVPAQEKNFTTAPAICHDGKAHFPREGVFVSNGTHWFVTQRNFYEPQIITTDNTFVSGNCDVVIGIVNNTVYDPLQPELDSFKEELDKYFKNHTSPDVDLGDISGINASVVNIQKEIDRLNEVAKNLNESLIDLQELGKYEQYIKRSNGLPGPIGPPGPRGRTGDAGPVGPPGPPGPPGPPGPPSAGFDFSFLPQPPQEKAHDGGRYYRANDANVVRDRDLEVDTTLKSLSQQIENIRSPEGSRKNPARTCRDLKMCHSDWKSGEYWIDPNQGCNLDAIKVFCNMETGETCVYPTQPSVAQKNWYISKNPKDKRHVWFGESMTDGFQFEYGGQGSDPADVAIQLTFLRLMSTEASQNITYHCKNSVAYMDQQTGNLKKALLLQGSNEIEIRAEGNSRFTYSVTVDGCTSHTGAWGKTVIEYKTTKTSRLPIIDVAPLDVGAPDQEFGFDVGPVCFL

SEQ ID NO: 11 - protein, 1509 aa, synthetic construct
  source 1..1509: note; note (original language) = SARS-CoV-2 South African variant B.1.351 S-trimer fusion polypeptide without signal peptide, 1509 aa, S1/S2 furin cleavage site 1 mutant (685R→685A); organism (original language) = Synthetic construct
QCVNLTTRTQLPPAYTNSFTRGVYYPDKVFRSSVLHSTQDLFLPFFSNVTWFHAIHVSGTNGTKRFDNPVLPFNDGVYFASTEKSNIIRGWIFGTTLDSKTQSLLIVNNATNVVIKVCEFQFCNDPFLGVYYHKNNKSWMESEFRVYSSANNCTFEYVSQPFLMDLEGKQGNFKNLREFVFKNIDGYFKIYSKHTPINLVRDLPQGFSALEPLVDLPIGINITRFQTLLALHRSYLTPGDSSSGWTAGAAAYYVGYLQPRTFLLKYNENGTITDAVDCALDPLSETKCTLKSFTVEKGIYQTSNFRVQPTESIVRFPNITNLCPFGEVFNATRFASVYAWNRKRISNCVADYSVLYNSASFSTFKCYGVSPTKLNDLCFTNVYADSFVIRGDEVRQIAPGQTGNIADYNYKLPDDFTGCVIAWNSNNLDSKVGGNYNYLYRLFRKSNLKPFERDISTEIYQAGSTPCNGVKGFNCYFPLQSYGFQPTYGVGYQPYRVVVLSFELLHAPATVCGPKKSTNLVKNKCVNFNFNGLTGTGVLTESNKKFLPFQQFGRDIADTTDAVRDPQTLEILDITPCSFGGVSVITPGTNTSNQVAVLYQGVNCTEVPVAIHADQLTPTWRVYSTGSNVFQTRAGCLIGAEHVNNSYECDIPIGAGICASYQTQTNSPRRAASVASQSIIAYTMSLGAENSVAYSNNSIAIPTNFTISVTTEILPVSMTKTSVDCTMYICGDSTECSNLLLQYGSFCTQLNRALTGIAVEQDKNTQEVFAQVKQIYKTPPIKDFGGFNFSQILPDPSKPSKRSFIEDLLFNKVTLADAGFIKQYGDCLGDIAARDLICAQKFNGLTVLPPLLTDEMIAQYTSALLAGTITSGWTFGAGAALQIPFAMQMAYRFNGIGVTQNVLYENQKLIANQFNSAIGKIQDSLSSTASALGKLQDVVNQNAQALNTLVKQLSSNFGAISSVLNDILSRLDKVEAEVQIDRLITGRLQSLQTYVTQQLIRAAEIRASANLAATKMSECVLGQSKRVDFCGKGYHLMSFPQSAPHGVVFLHVTYVPAQEKNFTTAPAICHDGKAHFPREGVFVSNGTHWFVTQRNFYEPQIITTDNTFVSGNCDVVIGIVNNTVYDPLQPELDSFKEELDKYFKNHTSPDVDLGDISGINASVVNIQKEIDRLNEVAKNLNESLIDLQELGKYEQYIKRSNGLPGPIGPPGPRGRTGDAGPVGPPGPPGPPGPPGPPSAGFDFSFLPQPPQEKAHDGGRYYRANDANVVRDRDLEVDTTLKSLSQQIENIRSPEGSRKNPARTCRDLKMCHSDWKSGEYWIDPNQGCNLDAIKVFCNMETGETCVYPTQPSVAQKNWYISKNPKDKRHVWFGESMTDGFQFEYGGQGSDPADVAIQLTFLRLMSTEASQNITYHCKNSVAYMDQQTGNLKKALLLQGSNEIEIRAEGNSRFTYSVTVDGCTSHTGAWGKTVIEYKTTKTSRLPIIDVAPLDVGAPDQEFGFDVGPVCFL

SEQ ID NO: 12 - protein, 1509 aa, synthetic construct
  source 1..1509: note; note (original language) = SARS-CoV-2 South African variant B.1.351 S-trimer fusion polypeptide without signal peptide, 1509 aa, proline mutant (986K/987V→986P/987P); organism (original language) = Synthetic construct
QCVNLTTRTQLPPAYTNSFTRGVYYPDKVFRSSVLHSTQDLFLPFFSNVTWFHAIHVSGTNGTKRFDNPVLPFNDGVYFASTEKSNIIRGWIFGTTLDSKTQSLLIVNNATNVVIKVCEFQFCNDPFLGVYYHKNNKSWMESEFRVYSSANNCTFEYVSQPFLMDLEGKQGNFKNLREFVFKNIDGYFKIYSKHTPINLVRDLPQGFSALEPLVDLPIGINITRFQTLLALHRSYLTPGDSSSGWTAGAAAYYVGYLQPRTFLLKYNENGTITDAVDCALDPLSETKCTLKSFTVEKGIYQTSNFRVQPTESIVRFPNITNLCPFGEVFNATRFASVYAWNRKRISNCVADYSVLYNSASFSTFKCYGVSPTKLNDLCFTNVYADSFVIRGDEVRQIAPGQTGNIADYNYKLPDDFTGCVIAWNSNNLDSKVGGNYNYLYRLFRKSNLKPFERDISTEIYQAGSTPCNGVKGFNCYFPLQSYGFQPTYGVGYQPYRVVVLSFELLHAPATVCGPKKSTNLVKNKCVNFNFNGLTGTGVLTESNKKFLPFQQFGRDIADTTDAVRDPQTLEILDITPCSFGGVSVITPGTNTSNQVAVLYQGVNCTEVPVAIHADQLTPTWRVYSTGSNVFQTRAGCLIGAEHVNNSYECDIPIGAGICASYQTQTNSPRRARSVASQSIIAYTMSLGAENSVAYSNNSIAIPTNFTISVTTEILPVSMTKTSVDCTMYICGDSTECSNLLLQYGSFCTQLNRALTGIAVEQDKNTQEVFAQVKQIYKTPPIKDFGGFNFSQILPDPSKPSKRSFIEDLLFNKVTLADAGFIKQYGDCLGDIAARDLICAQKFNGLTVLPPLLTDEMIAQYTSALLAGTITSGWTFGAGAALQIPFAMQMAYRFNGIGVTQNVLYENQKLIANQFNSAIGKIQDSLSSTASALGKLQDVVNQNAQALNTLVKQLSSNFGAISSVLNDILSRLDPPEAEVQIDRLITGRLQSLQTYVTQQLIRAAEIRASANLAATKMSECVLGQSKRVDFCGKGYHLMSFPQSAPHGVVFLHVTYVPAQEKNFTTAPAICHDGKAHFPREGVFVSNGTHWFVTQRNFYEPQIITTDNTFVSGNCDVVIGIVNNTVYDPLQPELDSFKEELDKYFKNHTSPDVDLGDISGINASVVNIQKEIDRLNEVAKNLNESLIDLQELGKYEQYIKRSNGLPGPIGPPGPRGRTGDAGPVGPPGPPGPPGPPGPPSAGFDFSFLPQPPQEKAHDGGRYYRANDANVVRDRDLEVDTTLKSLSQQIENIRSPEGSRKNPARTCRDLKMCHSDWKSGEYWIDPNQGCNLDAIKVFCNMETGETCVYPTQPSVAQKNWYISKNPKDKRHVWFGESMTDGFQFEYGGQGSDPADVAIQLTFLRLMSTEASQNITYHCKNSVAYMDQQTGNLKKALLLQGSNEIEIRAEGNSRFTYSVTVDGCTSHTGAWGKTVIEYKTTKTSRLPIIDVAPLDVGAPDQEFGFDVGPVCFL

SEQ ID NO: 13 - protein, 1509 aa, synthetic construct
  source 1..1509: note; note (original language) = SARS-CoV-2 South African variant B.1.351 S-trimer fusion polypeptide without signal peptide, 1509 aa, S1/S2 furin cleavage site 1 and proline mutant (685R→685A, 986K/987V→986P/987P); organism (original language) = Synthetic construct
QCVNLTTRTQLPPAYTNSFTRGVYYPDKVFRSSVLHSTQDLFLPFFSNVTWFHAIHVSGTNGTKRFDNPVLPFNDGVYFASTEKSNIIRGWIFGTTLDSKTQSLLIVNNATNVVIKVCEFQFCNDPFLGVYYHKNNKSWMESEFRVYSSANNCTFEYVSQPFLMDLEGKQGNFKNLREFVFKNIDGYFKIYSKHTPINLVRDLPQGFSALEPLVDLPIGINITRFQTLLALHRSYLTPGDSSSGWTAGAAAYYVGYLQPRTFLLKYNENGTITDAVDCALDPLSETKCTLKSFTVEKGIYQTSNFRVQPTESIVRFPNITNLCPFGEVFNATRFASVYAWNRKRISNCVADYSVLYNSASFSTFKCYGVSPTKLNDLCFTNVYADSFVIRGDEVRQIAPGQTGNIADYNYKLPDDFTGCVIAWNSNNLDSKVGGNYNYLYRLFRKSNLKPFERDISTEIYQAGSTPCNGVKGFNCYFPLQSYGFQPTYGVGYQPYRVVVLSFELLHAPATVCGPKKSTNLVKNKCVNFNFNGLTGTGVLTESNKKFLPFQQFGRDIADTTDAVRDPQTLEILDITPCSFGGVSVITPGTNTSNQVAVLYQGVNCTEVPVAIHADQLTPTWRVYSTGSNVFQTRAGCLIGAEHVNNSYECDIPIGAGICASYQTQTNSPRRAASVASQSIIAYTMSLGAENSVAYSNNSIAIPTNFTISVTTEILPVSMTKTSVDCTMYICGDSTECSNLLLQYGSFCTQLNRALTGIAVEQDKNTQEVFAQVKQIYKTPPIKDFGGFNFSQILPDPSKPSKRSFIEDLLFNKVTLADAGFIKQYGDCLGDIAARDLICAQKFNGLTVLPPLLTDEMIAQYTSALLAGTITSGWTFGAGAALQIPFAMQMAYRFNGIGVTQNVLYENQKLIANQFNSAIGKIQDSLSSTASALGKLQDVVNQNAQALNTLVKQLSSNFGAISSVLNDILSRLDPPEAEVQIDRLITGRLQSLQTYVTQQLIRAAEIRASANLAATKMSECVLGQSKRVDFCGKGYHLMSFPQSAPHGVVFLHVTYVPAQEKNFTTAPAICHDGKAHFPREGVFVSNGTHWFVTQRNFYEPQIITTDNTFVSGNCDVVIGIVNNTVYDPLQPELDSFKEELDKYFKNHTSPDVDLGDISGINASVVNIQKEIDRLNEVAKNLNESLIDLQELGKYEQYIKRSNGLPGPIGPPGPRGRTGDAGPVGPPGPPGPPGPPGPPSAGFDFSFLPQPPQEKAHDGGRYYRANDANVVRDRDLEVDTTLKSLSQQIENIRSPEGSRKNPARTCRDLKMCHSDWKSGEYWIDPNQGCNLDAIKVFCNMETGETCVYPTQPSVAQKNWYISKNPKDKRHVWFGESMTDGFQFEYGGQGSDPADVAIQLTFLRLMSTEASQNITYHCKNSVAYMDQQTGNLKKALLLQGSNEIEIRAEGNSRFTYSVTVDGCTSHTGAWGKTVIEYKTTKTSRLPIIDVAPLDVGAPDQEFGFDVGPVCFL

SEQ ID NO: 14 - protein, 1509 aa, synthetic construct
  source 1..1509: note; note (original language) = SARS-CoV-2 Brazilian variant P.1 S-trimer fusion polypeptide without signal peptide, 1509 aa; organism (original language) = Synthetic construct
QCVNFTNRTQLPSAYTNSFTRGVYYPDKVFRSSVLHSTQDLFLPFFSNVTWFHAIHVSGTNGTKRFDNPVLPFNDGVYFASTEKSNIIRGWIFGTTLDSKTQSLLIVNNATNVVIKVCEFQFCNYPFLGVYYHKNNKSWMESEFRVYSSANNCTFEYVSQPFLMDLEGKQGNFKNLSEFVFKNIDGYFKIYSKHTPINLVRDLPQGFSALEPLVDLPIGINITRFQTLLALHRSYLTPGDSSSGWTAGAAAYYVGYLQPRTFLLKYNENGTITDAVDCALDPLSETKCTLKSFTVEKGIYQTSNFRVQPTESIVRFPNITNLCPFGEVFNATRFASVYAWNRKRISNCVADYSVLYNSASFSTFKCYGVSPTKLNDLCFTNVYADSFVIRGDEVRQIAPGQTGTIADYNYKLPDDFTGCVIAWNSNNLDSKVGGNYNYLYRLFRKSNLKPFERDISTEIYQAGSTPCNGVKGFNCYFPLQSYGFQPTYGVGYQPYRVVVLSFELLHAPATVCGPKKSTNLVKNKCVNFNFNGLTGTGVLTESNKKFLPFQQFGRDIADTTDAVRDPQTLEILDITPCSFGGVSVITPGTNTSNQVAVLYQGVNCTEVPVAIHADQLTPTWRVYSTGSNVFQTRAGCLIGAEYVNNSYECDIPIGAGICASYQTQTNSPRRARSVASQSIIAYTMSLGAENSVAYSNNSIAIPTNFTISVTTEILPVSMTKTSVDCTMYICGDSTECSNLLLQYGSFCTQLNRALTGIAVEQDKNTQEVFAQVKQIYKTPPIKDFGGFNFSQILPDPSKPSKRSFIEDLLFNKVTLADAGFIKQYGDCLGDIAARDLICAQKFNGLTVLPPLLTDEMIAQYTSALLAGTITSGWTFGAGAALQIPFAMQMAYRFNGIGVTQNVLYENQKLIANQFNSAIGKIQDSLSSTASALGKLQDVVNQNAQALNTLVKQLSSNFGAISSVLNDILSRLDKVEAEVQIDRLITGRLQSLQTYVTQQLIRAAEIRASANLAAIKMSECVLGQSKRVDFCGKGYHLMSFPQSAPHGVVFLHVTYVPAQEKNFTTAPAICHDGKAHFPREGVFVSNGTHWFVTQRNFYEPQIITTDNTFVSGNCDVVIGIVNNTVYDPLQPELDSFKEELDKYFKNHTSPDVDLGDISGINASVVNIQKEIDRLNEVAKNLNESLIDLQELGKYEQYIKRSNGLPGPIGPPGPRGRTGDAGPVGPPGPPGPPGPPGPPSAGFDFSFLPQPPQEKAHDGGRYYRANDANVVRDRDLEVDTTLKSLSQQIENIRSPEGSRKNPARTCRDLKMCHSDWKSGEYWIDPNQGCNLDAIKVFCNMETGETCVYPTQPSVAQKNWYISKNPKDKRHVWFGESMTDGFQFEYGGQGSDPADVAIQLTFLRLMSTEASQNITYHCKNSVAYMDQQTGNLKKALLLQGSNEIEIRAEGNSRFTYSVTVDGCTSHTGAWGKTVIEYKTTKTSRLPIIDVAPLDVGAPDQEFGFDVGPVCFL

SEQ ID NO: 15 - protein, 1509 aa, synthetic construct
  source 1..1509: note; note (original language) = SARS-CoV-2 Brazilian variant P.1 S-trimer fusion polypeptide without signal peptide, 1509 aa, S1/S2 furin cleavage site 1 mutant (685R→685A); organism (original language) = Synthetic construct
QCVNFTNRTQLPSAYTNSFTRGVYYPDKVFRSSVLHSTQDLFLPFFSNVTWFHAIHVSGTNGTKRFDNPVLPFNDGVYFASTEKSNIIRGWIFGTTLDSKTQSLLIVNNATNVVIKVCEFQFCNYPFLGVYYHKNNKSWMESEFRVYSSANNCTFEYVSQPFLMDLEGKQGNFKNLSEFVFKNIDGYFKIYSKHTPINLVRDLPQGFSALEPLVDLPIGINITRFQTLLALHRSYLTPGDSSSGWTAGAAAYYVGYLQPRTFLLKYNENGTITDAVDCALDPLSETKCTLKSFTVEKGIYQTSNFRVQPTESIVRFPNITNLCPFGEVFNATRFASVYAWNRKRISNCVADYSVLYNSASFSTFKCYGVSPTKLNDLCFTNVYADSFVIRGDEVRQIAPGQTGTIADYNYKLPDDFTGCVIAWNSNNLDSKVGGNYNYLYRLFRKSNLKPFERDISTEIYQAGSTPCNGVKGFNCYFPLQSYGFQPTYGVGYQPYRVVVLSFELLHAPATVCGPKKSTNLVKNKCVNFNFNGLTGTGVLTESNKKFLPFQQFGRDIADTTDAVRDPQTLEILDITPCSFGGVSVITPGTNTSNQVAVLYQGVNCTEVPVAIHADQLTPTWRVYSTGSNVFQTRAGCLIGAEYVNNSYECDIPIGAGICASYQTQTNSPRRAASVASQSIIAYTMSLGAENSVAYSNNSIAIPTNFTISVTTEILPVSMTKTSVDCTMYICGDSTECSNLLLQYGSFCTQLNRALTGIAVEQDKNTQEVFAQVKQIYKTPPIKDFGGFNFSQILPDPSKPSKRSFIEDLLFNKVTLADAGFIKQYGDCLGDIAARDLICAQKFNGLTVLPPLLTDEMIAQYTSALLAGTITSGWTFGAGAALQIPFAMQMAYRFNGIGVTQNVLYENQKLIANQFNSAIGKIQDSLSSTASALGKLQDVVNQNAQALNTLVKQLSSNFGAISSVLNDILSRLDKVEAEVQIDRLITGRLQSLQTYVTQQLIRAAEIRASANLAAIKMSECVLGQSKRVDFCGKGYHLMSFPQSAPHGVVFLHVTYVPAQEKNFTTAPAICHDGKAHFPREGVFVSNGTHWFVTQRNFYEPQIITTDNTFVSGNCDVVIGIVNNTVYDPLQPELDSFKEELDKYFKNHTSPDVDLGDISGINASVVNIQKEIDRLNEVAKNLNESLIDLQELGKYEQYIKRSNGLPGPIGPPGPRGRTGDAGPVGPPGPPGPPGPPGPPSAGFDFSFLPQPPQEKAHDGGRYYRANDANVVRDRDLEVDTTLKSLSQQIENIRSPEGSRKNPARTCRDLKMCHSDWKSGEYWIDPNQGCNLDAIKVFCNMETGETCVYPTQPSVAQKNWYISKNPKDKRHVWFGESMTDGFQFEYGGQGSDPADVAIQLTFLRLMSTEASQNITYHCKNSVAYMDQQTGNLKKALLLQGSNEIEIRAEGNSRFTYSVTVDGCTSHTGAWGKTVIEYKTTKTSRLPIIDVAPLDVGAPDQEFGFDVGPVCFL

SEQ ID NO: 16 - protein, 1509 aa, synthetic construct
  source 1..1509: note; note (original language) = SARS-CoV-2 Brazilian variant P.1 S-trimer fusion polypeptide without signal peptide, 1509 aa, proline mutant (986K/987V→986P/987P); organism (original language) = Synthetic construct
QCVNFTNRTQLPSAYTNSFTRGVYYPDKVFRSSVLHSTQDLFLPFFSNVTWFHAIHVSGTNGTKRFDNPVLPFNDGVYFASTEKSNIIRGWIFGTTLDSKTQSLLIVNNATNVVIKVCEFQFCNYPFLGVYYHKNNKSWMESEFRVYSSANNCTFEYVSQPFLMDLEGKQGNFKNLSEFVFKNIDGYFKIYSKHTPINLVRDLPQGFSALEPLVDLPIGINITRFQTLLALHRSYLTPGDSSSGWTAGAAAYYVGYLQPRTFLLKYNENGTITDAVDCALDPLSETKCTLKSFTVEKGIYQTSNFRVQPTESIVRFPNITNLCPFGEVFNATRFASVYAWNRKRISNCVADYSVLYNSASFSTFKCYGVSPTKLNDLCFTNVYADSFVIRGDEVRQIAPGQTGTIADYNYKLPDDFTGCVIAWNSNNLDSKVGGNYNYLYRLFRKSNLKPFERDISTEIYQAGSTPCNGVKGFNCYFPLQSYGFQPTYGVGYQPYRVVVLSFELLHAPATVCGPKKSTNLVKNKCVNFNFNGLTGTGVLTESNKKFLPFQQFGRDIADTTDAVRDPQTLEILDITPCSFGGVSVITPGTNTSNQVAVLYQGVNCTEVPVAIHADQLTPTWRVYSTGSNVFQTRAGCLIGAEYVNNSYECDIPIGAGICASYQTQTNSPRRARSVASQSIIAYTMSLGAENSVAYSNNSIAIPTNFTISVTTEILPVSMTKTSVDCTMYICGDSTECSNLLLQYGSFCTQLNRALTGIAVEQDKNTQEVFAQVKQIYKTPPIKDFGGFNFSQILPDPSKPSKRSFIEDLLFNKVTLADAGFIKQYGDCLGDIAARDLICAQKFNGLTVLPPLLTDEMIAQYTSALLAGTITSGWTFGAGAALQIPFAMQMAYRFNGIGVTQNVLYENQKLIANQFNSAIGKIQDSLSSTASALGKLQDVVNQNAQALNTLVKQLSSNFGAISSVLNDILSRLDPPEAEVQIDRLITGRLQSLQTYVTQQLIRAAEIRASANLAAIKMSECVLGQSKRVDFCGKGYHLMSFPQSAPHGVVFLHVTYVPAQEKNFTTAPAICHDGKAHFPREGVFVSNGTHWFVTQRNFYEPQIITTDNTFVSGNCDVVIGIVNNTVYDPLQPELDSFKEELDKYFKNHTSPDVDLGDISGINASVVNIQKEIDRLNEVAKNLNESLIDLQELGKYEQYIKRSNGLPGPIGPPGPRGRTGDAGPVGPPGPPGPPGPPGPPSAGFDFSFLPQPPQEKAHDGGRYYRANDANVVRDRDLEVDTTLKSLSQQIENIRSPEGSRKNPARTCRDLKMCHSDWKSGEYWIDPNQGCNLDAIKVFCNMETGETCVYPTQPSVAQKNWYISKNPKDKRHVWFGESMTDGFQFEYGGQGSDPADVAIQLTFLRLMSTEASQNITYHCKNSVAYMDQQTGNLKKALLLQGSNEIEIRAEGNSRFTYSVTVDGCTSHTGAWGKTVIEYKTTKTSRLPIIDVAPLDVGAPDQEFGFDVGPVCFL

SEQ ID NO: 17 - protein, 1509 aa, synthetic construct
  source 1..1509: note; note (original language) = SARS-CoV-2 Brazilian variant P.1 S-trimer fusion polypeptide without signal peptide, 1509 aa, S1/S2 furin cleavage site 1 and proline mutant (685R→685A, 986K/987V→986P/987P); organism (original language) = Synthetic construct
QCVNFTNRTQLPSAYTNSFTRGVYYPDKVFRSSVLHSTQDLFLPFFSNVTWFHAIHVSGTNGTKRFDNPVLPFNDGVYFASTEKSNIIRGWIFGTTLDSKTQSLLIVNNATNVVIKVCEFQFCNYPFLGVYYHKNNKSWMESEFRVYSSANNCTFEYVSQPFLMDLEGKQGNFKNLSEFVFKNIDGYFKIYSKHTPINLVRDLPQGFSALEPLVDLPIGINITRFQTLLALHRSYLTPGDSSSGWTAGAAAYYVGYLQPRTFLLKYNENGTITDAVDCALDPLSETKCTLKSFTVEKGIYQTSNFRVQPTESIVRFPNITNLCPFGEVFNATRFASVYAWNRKRISNCVADYSVLYNSASFSTFKCYGVSPTKLNDLCFTNVYADSFVIRGDEVRQIAPGQTGTIADYNYKLPDDFTGCVIAWNSNNLDSKVGGNYNYLYRLFRKSNLKPFERDISTEIYQAGSTPCNGVKGFNCYFPLQSYGFQPTYGVGYQPYRVVVLSFELLHAPATVCGPKKSTNLVKNKCVNFNFNGLTGTGVLTESNKKFLPFQQFGRDIADTTDAVRDPQTLEILDITPCSFGGVSVITPGTNTSNQVAVLYQGVNCTEVPVAIHADQLTPTWRVYSTGSNVFQTRAGCLIGAEYVNNSYECDIPIGAGICASYQTQTNSPRRAASVASQSIIAYTMSLGAENSVAYSNNSIAIPTNFTISVTTEILPVSMTKTSVDCTMYICGDSTECSNLLLQYGSFCTQLNRALTGIAVEQDKNTQEVFAQVKQIYKTPPIKDFGGFNFSQILPDPSKPSKRSFIEDLLFNKVTLADAGFIKQYGDCLGDIAARDLICAQKFNGLTVLPPLLTDEMIAQYTSALLAGTITSGWTFGAGAALQIPFAMQMAYRFNGIGVTQNVLYENQKLIANQFNSAIGKIQDSLSSTASALGKLQDVVNQNAQALNTLVKQLSSNFGAISSVLNDILSRLDPPEAEVQIDRLITGRLQSLQTYVTQQLIRAAEIRASANLAAIKMSECVLGQSKRVDFCGKGYHLMSFPQSAPHGVVFLHVTYVPAQEKNFTTAPAICHDGKAHFPREGVFVSNGTHWFVTQRNFYEPQIITTDNTFVSGNCDVVIGIVNNTVYDPLQPELDSFKEELDKYFKNHTSPDVDLGDISGINASVVNIQKEIDRLNEVAKNLNESLIDLQELGKYEQYIKRSNGLPGPIGPPGPRGRTGDAGPVGPPGPPGPPGPPGPPSAGFDFSFLPQPPQEKAHDGGRYYRANDANVVRDRDLEVDTTLKSLSQQIENIRSPEGSRKNPARTCRDLKMCHSDWKSGEYWIDPNQGCNLDAIKVFCNMETGETCVYPTQPSVAQKNWYISKNPKDKRHVWFGESMTDGFQFEYGGQGSDPADVAIQLTFLRLMSTEASQNITYHCKNSVAYMDQQTGNLKKALLLQGSNEIEIRAEGNSRFTYSVTVDGCTSHTGAWGKTVIEYKTTKTSRLPIIDVAPLDVGAPDQEFGFDVGPVCFL

SEQ ID NO: 18 - protein, 1507 aa, synthetic construct
  source 1..1507: note; note (original language) = SARS-CoV-2 British variant B.1.1.7 S-trimer fusion polypeptide without signal peptide, 1507 aa; organism (original language) = Synthetic construct
QCVNLTTRTQLPPAYTNSFTRGVYYPDKVFRSSVLHSTQDLFLPFFSNVTWFHAISGTNGTKRFDNPVLPFNDGVYFASTEKSNIIRGWIFGTTLDSKTQSLLIVNNATNVVIKVCEFQFCNDPFLGVYYHKNNKSWMESEFRVYSSANNCTFEYVSQPFLMDLEGKQGNFKNLREFVFKNIDGYFKIYSKHTPINLVRDLPQGFSALEPLVDLPIGINITRFQTLLALHRSYLTPGDSSSGWTAGAAAYYVGYLQPRTFLLKYNENGTITDAVDCALDPLSETKCTLKSFTVEKGIYQTSNFRVQPTESIVRFPNITNLCPFGEVFNATRFASVYAWNRKRISNCVADYSVLYNSASFSTFKCYGVSPTKLNDLCFTNVYADSFVIRGDEVRQIAPGQTGKIADYNYKLPDDFTGCVIAWNSNNLDSKVGGNYNYLYRLFRKSNLKPFERDISTEIYQAGSTPCNGVEGFNCYFPLQSYGFQPTYGVGYQPYRVVVLSFELLHAPATVCGPKKSTNLVKNKCVNFNFNGLTGTGVLTESNKKFLPFQQFGRDIADTTDAVRDPQTLEILDITPCSFGGVSVITPGTNTSNQVAVLYQGVNCTEVPVAIHADQLTPTWRVYSTGSNVFQTRAGCLIGAEHVNNSYECDIPIGAGICASYQTQTNSHRRARSVASQSIIAYTMSLGAENSVAYSNNSIAIPTNFTISVTTEILPVSMTKTSVDCTMYICGDSTECSNLLLQYGSFCTQLNRALTGIAVEQDKNTQEVFAQVKQIYKTPPIKDFGGFNFSQILPDPSKPSKRSFIEDLLFNKVTLADAGFIKQYGDCLGDIAARDLICAQKFNGLTVLPPLLTDEMIAQYTSALLAGTITSGWTFGAGAALQIPFAMQMAYRFNGIGVTQNVLYENQKLIANQFNSAIGKIQDSLSSTASALGKLQDVVNQNAQALNTLVKQLSSNFGAISSVLNDILSRLDKVEAEVQIDRLITGRLQSLQTYVTQQLIRAAEIRASANLAATKMSECVLGQSKRVDFCGKGYHLMSFPQSAPHGVVFLHVTYVPAQEKNFTTAPAICHDGKAHFPREGVFVSNGTHWFVTQRNFYEPQIITTDNTFVSGNCDVVIGIVNNTVYDPLQPELDSFKEELDKYFKNHTSPDVDLGDISGINASVVNIQKEIDRLNEVAKNLNESLIDLQELGKYEQYIKRSNGLPGPIGPPGPRGRTGDAGPVGPPGPPGPPGPPGPPSAGFDFSFLPQPPQEKAHDGGRYYRANDANVVRDRDLEVDTTLKSLSQQIENIRSPEGSRKNPARTCRDLKMCHSDWKSGEYWIDPNQGCNLDAIKVFCNMETGETCVYPTQPSVAQKNWYISKNPKDKRHVWFGESMTDGFQFEYGGQGSDPADVAIQLTFLRLMSTEASQNITYHCKNSVAYMDQQTGNLKKALLLQGSNEIEIRAEGNSRFTYSVTVDGCTSHTGAWGKTVIEYKTTKTSRLPIIDVAPLDVGAPDQEFGFDVGPVCFL

SEQ ID NO: 19 - protein, 1507 aa, synthetic construct
  source 1..1507: note; note (original language) = SARS-CoV-2 British variant B.1.1.7 S-trimer fusion polypeptide without signal peptide, 1507 aa, S1/S2 furin cleavage site 1 mutant (685R→685A); organism (original language) = Synthetic construct
QCVNLTTRTQLPPAYTNSFTRGVYYPDKVFRSSVLHSTQDLFLPFFSNVTWFHAISGTNGTKRFDNPVLPFNDGVYFASTEKSNIIRGWIFGTTLDSKTQSLLIVNNATNVVIKVCEFQFCNDPFLGVYYHKNNKSWMESEFRVYSSANNCTFEYVSQPFLMDLEGKQGNFKNLREFVFKNIDGYFKIYSKHTPINLVRDLPQGFSALEPLVDLPIGINITRFQTLLALHRSYLTPGDSSSGWTAGAAAYYVGYLQPRTFLLKYNENGTITDAVDCALDPLSETKCTLKSFTVEKGIYQTSNFRVQPTESIVRFPNITNLCPFGEVFNATRFASVYAWNRKRISNCVADYSVLYNSASFSTFKCYGVSPTKLNDLCFTNVYADSFVIRGDEVRQIAPGQTGKIADYNYKLPDDFTGCVIAWNSNNLDSKVGGNYNYLYRLFRKSNLKPFERDISTEIYQAGSTPCNGVEGFNCYFPLQSYGFQPTYGVGYQPYRVVVLSFELLHAPATVCGPKKSTNLVKNKCVNFNFNGLTGTGVLTESNKKFLPFQQFGRDIADTTDAVRDPQTLEILDITPCSFGGVSVITPGTNTSNQVAVLYQGVNCTEVPVAIHADQLTPTWRVYSTGSNVFQTRAGCLIGAEHVNNSYECDIPIGAGICASYQTQTNSHRRAASVASQSIIAYTMSLGAENSVAYSNNSIAIPTNFTISVTTEILPVSMTKTSVDCTMYICGDSTECSNLLLQYGSFCTQLNRALTGIAVEQDKNTQEVFAQVKQIYKTPPIKDFGGFNFSQILPDPSKPSKRSFIEDLLFNKVTLADAGFIKQYGDCLGDIAARDLICAQKFNGLTVLPPLLTDEMIAQYTSALLAGTITSGWTFGAGAALQIPFAMQMAYRFNGIGVTQNVLYENQKLIANQFNSAIGKIQDSLSSTASALGKLQDVVNQNAQALNTLVKQLSSNFGAISSVLNDILSRLDKVEAEVQIDRLITGRLQSLQTYVTQQLIRAAEIRASANLAATKMSECVLGQSKRVDFCGKGYHLMSFPQSAPHGVVFLHVTYVPAQEKNFTTAPAICHDGKAHFPREGVFVSNGTHWFVTQRNFYEPQIITTDNTFVSGNCDVVIGIVNNTVYDPLQPELDSFKEELDKYFKNHTSPDVDLGDISGINASVVNIQKEIDRLNEVAKNLNESLIDLQELGKYEQYIKRSNGLPGPIGPPGPRGRTGDAGPVGPPGPPGPPGPPGPPSAGFDFSFLPQPPQEKAHDGGRYYRANDANVVRDRDLEVDTTLKSLSQQIENIRSPEGSRKNPARTCRDLKMCHSDWKSGEYWIDPNQGCNLDAIKVFCNMETGETCVYPTQPSVAQKNWYISKNPKDKRHVWFGESMTDGFQFEYGGQGSDPADVAIQLTFLRLMSTEASQNITYHCKNSVAYMDQQTGNLKKALLLQGSNEIEIRAEGNSRFTYSVTVDGCTSHTGAWGKTVIEYKTTKTSRLPIIDVAPLDVGAPDQEFGFDVGPVCFL

SEQ ID NO: 20 - protein, 1507 aa, synthetic construct
  source 1..1507: note; note (original language) = SARS-CoV-2 British variant B.1.1.7 S-trimer fusion polypeptide without signal peptide, 1507 aa, proline mutant (986K/987V→986P/987P); organism (original language) = Synthetic construct
QCVNLTTRTQLPPAYTNSFTRGVYYPDKVFRSSVLHSTQDLFLPFFSNVTWFHAISGTNGTKRFDNPVLPFNDGVYFASTEKSNIIRGWIFGTTLDSKTQSLLIVNNATNVVIKVCEFQFCNDPFLGVYYHKNNKSWMESEFRVYSSANNCTFEYVSQPFLMDLEGKQGNFKNLREFVFKNIDGYFKIYSKHTPINLVRDLPQGFSALEPLVDLPIGINITRFQTLLALHRSYLTPGDSSSGWTAGAAAYYVGYLQPRTFLLKYNENGTITDAVDCALDPLSETKCTLKSFTVEKGIYQTSNFRVQPTESIVRFPNITNLCPFGEVFNATRFASVYAWNRKRISNCVADYSVLYNSASFSTFKCYGVSPTKLNDLCFTNVYADSFVIRGDEVRQIAPGQTGKIADYNYKLPDDFTGCVIAWNSNNLDSKVGGNYNYLYRLFRKSNLKPFERDISTEIYQAGSTPCNGVEGFNCYFPLQSYGFQPTYGVGYQPYRVVVLSFELLHAPATVCGPKKSTNLVKNKCVNFNFNGLTGTGVLTESNKKFLPFQQFGRDIADTTDAVRDPQTLEILDITPCSFGGVSVITPGTNTSNQVAVLYQGVNCTEVPVAIHADQLTPTWRVYSTGSNVFQTRAGCLIGAEHVNNSYECDIPIGAGICASYQTQTNSHRRARSVASQSIIAYTMSLGAENSVAYSNNSIAIPTNFTISVTTEILPVSMTKTSVDCTMYICGDSTECSNLLLQYGSFCTQLNRALTGIAVEQDKNTQEVFAQVKQIYKTPPIKDFGGFNFSQILPDPSKPSKRSFIEDLLFNKVTLADAGFIKQYGDCLGDIAARDLICAQKFNGLTVLPPLLTDEMIAQYTSALLAGTITSGWTFGAGAALQIPFAMQMAYRFNGIGVTQNVLYENQKLIANQFNSAIGKIQDSLSSTASALGKLQDVVNQNAQALNTLVKQLSSNFGAISSVLNDILSRLDPPEAEVQIDRLITGRLQSLQTYVTQQLIRAAEIRASANLAATKMSECVLGQSKRVDFCGKGYHLMSFPQSAPHGVVFLHVTYVPAQEKNFTTAPAICHDGKAHFPREGVFVSNGTHWFVTQRNFYEPQIITTDNTFVSGNCDVVIGIVNNTVYDPLQPELDSFKEELDKYFKNHTSPDVDLGDISGINASVVNIQKEIDRLNEVAKNLNESLIDLQELGKYEQYIKRSNGLPGPIGPPGPRGRTGDAGPVGPPGPPGPPGPPGPPSAGFDFSFLPQPPQEKAHDGGRYYRANDANVVRDRDLEVDTTLKSLSQQIENIRSPEGSRKNPARTCRDLKMCHSDWKSGEYWIDPNQGCNLDAIKVFCNMETGETCVYPTQPSVAQKNWYISKNPKDKRHVWFGESMTDGFQFEYGGQGSDPADVAIQLTFLRLMSTEASQNITYHCKNSVAYMDQQTGNLKKALLLQGSNEIEIRAEGNSRFTYSVTVDGCTSHTGAWGKTVIEYKTTKTSRLPIIDVAPLDVGAPDQEFGFDVGPVCFL

SEQ ID NO: 21 - protein, 1507 aa, synthetic construct
  source 1..1507: note; note (original language) = SARS-CoV-2 British variant B.1.1.7 S-trimer fusion polypeptide without signal peptide, 1507 aa, S1/S2 furin cleavage site 1 and proline mutant (685R→685A, 986K/987V→986P/987P); organism (original language) = Synthetic construct
QCVNLTTRTQLPPAYTNSFTRGVYYPDKVFRSSVLHSTQDLFLPFFSNVTWFHAISGTNGTKRFDNPVLPFNDGVYFASTEKSNIIRGWIFGTTLDSKTQSLLIVNNATNVVIKVCEFQFCNDPFLGVYYHKNNKSWMESEFRVYSSANNCTFEYVSQPFLMDLEGKQGNFKNLREFVFKNIDGYFKIYSKHTPINLVRDLPQGFSALEPLVDLPIGINITRFQTLLALHRSYLTPGDSSSGWTAGAAAYYVGYLQPRTFLLKYNENGTITDAVDCALDPLSETKCTLKSFTVEKGIYQTSNFRVQPTESIVRFPNITNLCPFGEVFNATRFASVYAWNRKRISNCVADYSVLYNSASFSTFKCYGVSPTKLNDLCFTNVYADSFVIRGDEVRQIAPGQTGKIADYNYKLPDDFTGCVIAWNSNNLDSKVGGNYNYLYRLFRKSNLKPFERDISTEIYQAGSTPCNGVEGFNCYFPLQSYGFQPTYGVGYQPYRVVVLSFELLHAPATVCGPKKSTNLVKNKCVNFNFNGLTGTGVLTESNKKFLPFQQFGRDIADTTDAVRDPQTLEILDITPCSFGGVSVITPGTNTSNQVAVLYQGVNCTEVPVAIHADQLTPTWRVYSTGSNVFQTRAGCLIGAEHVNNSYECDIPIGAGICASYQTQTNSHRRAASVASQSIIAYTMSLGAENSVAYSNNSIAIPTNFTISVTTEILPVSMTKTSVDCTMYICGDSTECSNLLLQYGSFCTQLNRALTGIAVEQDKNTQEVFAQVKQIYKTPPIKDFGGFNFSQILPDPSKPSKRSFIEDLLFNKVTLADAGFIKQYGDCLGDIAARDLICAQKFNGLTVLPPLLTDEMIAQYTSALLAGTITSGWTFGAGAALQIPFAMQMAYRFNGIGVTQNVLYENQKLIANQFNSAIGKIQDSLSSTASALGKLQDVVNQNAQALNTLVKQLSSNFGAISSVLNDILSRLDPPEAEVQIDRLITGRLQSLQTYVTQQLIRAAEIRASANLAATKMSECVLGQSKRVDFCGKGYHLMSFPQSAPHGVVFLHVTYVPAQEKNFTTAPAICHDGKAHFPREGVFVSNGTHWFVTQRNFYEPQIITTDNTFVSGNCDVVIGIVNNTVYDPLQPELDSFKEELDKYFKNHTSPDVDLGDISGINASVVNIQKEIDRLNEVAKNLNESLIDLQELGKYEQYIKRSNGLPGPIGPPGPRGRTGDAGPVGPPGPPGPPGPPGPPSAGFDFSFLPQPPQEKAHDGGRYYRANDANVVRDRDLEVDTTLKSLSQQIENIRSPEGSRKNPARTCRDLKMCHSDWKSGEYWIDPNQGCNLDAIKVFCNMETGETCVYPTQPSVAQKNWYISKNPKDKRHVWFGESMTDGFQFEYGGQGSDPADVAIQLTFLRLMSTEASQNITYHCKNSVAYMDQQTGNLKKALLLQGSNEIEIRAEGNSRFTYSVTVDGCTSHTGAWGKTVIEYKTTKTSRLPIIDVAPLDVGAPDQEFGFDVGPVCFL

SEQ ID NO: 22 - protein, 1509 aa, synthetic construct
  source 1..1509: note; note (original language) = SARS-CoV-2 variant D614G S-trimer fusion polypeptide without signal peptide, 1509 aa; organism (original language) = Synthetic construct
QCVNLTTRTQLPPAYTNSFTRGVYYPDKVFRSSVLHSTQDLFLPFFSNVTWFHAIHVSGTNGTKRFDNPVLPFNDGVYFASTEKSNIIRGWIFGTTLDSKTQSLLIVNNATNVVIKVCEFQFCNDPFLGVYYHKNNKSWMESEFRVYSSANNCTFEYVSQPFLMDLEGKQGNFKNLREFVFKNIDGYFKIYSKHTPINLVRDLPQGFSALEPLVDLPIGINITRFQTLLALHRSYLTPGDSSSGWTAGAAAYYVGYLQPRTFLLKYNENGTITDAVDCALDPLSETKCTLKSFTVEKGIYQTSNFRVQPTESIVRFPNITNLCPFGEVFNATRFASVYAWNRKRISNCVADYSVLYNSASFSTFKCYGVSPTKLNDLCFTNVYADSFVIRGDEVRQIAPGQTGKIADYNYKLPDDFTGCVIAWNSNNLDSKVGGNYNYLYRLFRKSNLKPFERDISTEIYQAGSTPCNGVEGFNCYFPLQSYGFQPTNGVGYQPYRVVVLSFELLHAPATVCGPKKSTNLVKNKCVNFNFNGLTGTGVLTESNKKFLPFQQFGRDIADTTDAVRDPQTLEILDITPCSFGGVSVITPGTNTSNQVAVLYQGVNCTEVPVAIHADQLTPTWRVYSTGSNVFQTRAGCLIGAEHVNNSYECDIPIGAGICASYQTQTNSPRRARSVASQSIIAYTMSLGAENSVAYSNNSIAIPTNFTISVTTEILPVSMTKTSVDCTMYICGDSTECSNLLLQYGSFCTQLNRALTGIAVEQDKNTQEVFAQVKQIYKTPPIKDFGGFNFSQILPDPSKPSKRSFIEDLLFNKVTLADAGFIKQYGDCLGDIAARDLICAQKFNGLTVLPPLLTDEMIAQYTSALLAGTITSGWTFGAGAALQIPFAMQMAYRFNGIGVTQNVLYENQKLIANQFNSAIGKIQDSLSSTASALGKLQDVVNQNAQALNTLVKQLSSNFGAISSVLNDILSRLDKVEAEVQIDRLITGRLQSLQTYVTQQLIRAAEIRASANLAATKMSECVLGQSKRVDFCGKGYHLMSFPQSAPHGVVFLHVTYVPAQEKNFTTAPAICHDGKAHFPREGVFVSNGTHWFVTQRNFYEPQIITTDNTFVSGNCDVVIGIVNNTVYDPLQPELDSFKEELDKYFKNHTSPDVDLGDISGINASVVNIQKEIDRLNEVAKNLNESLIDLQELGKYEQYIKRSNGLPGPIGPPGPRGRTGDAGPVGPPGPPGPPGPPGPPSAGFDFSFLPQPPQEKAHDGGRYYRANDANVVRDRDLEVDTTLKSLSQQIENIRSPEGSRKNPARTCRDLKMCHSDWKSGEYWIDPNQGCNLDAIKVFCNMETGETCVYPTQPSVAQKNWYISKNPKDKRHVWFGESMTDGFQFEYGGQGSDPADVAIQLTFLRLMSTEASQNITYHCKNSVAYMDQQTGNLKKALLLQGSNEIEIRAEGNSRFTYSVTVDGCTSHTGAWGKTVIEYKTTKTSRLPIIDVAPLDVGAPDQEFGFDVGPVCFL

SEQ ID NO: 23 - protein, 1509 aa, synthetic construct
  source 1..1509: note; note (original language) = SARS-CoV-2 variant D614G S-trimer fusion polypeptide without signal peptide, 1509 aa, S1/S2 furin cleavage site 1 mutant (685R→685A); organism (original language) = Synthetic construct
QCVNLTTRTQLPPAYTNSFTRGVYYPDKVFRSSVLHSTQDLFLPFFSNVTWFHAIHVSGTNGTKRFDNPVLPFNDGVYFASTEKSNIIRGWIFGTTLDSKTQSLLIVNNATNVVIKVCEFQFCNDPFLGVYYHKNNKSWMESEFRVYSSANNCTFEYVSQPFLMDLEGKQGNFKNLREFVFKNIDGYFKIYSKHTPINLVRDLPQGFSALEPLVDLPIGINITRFQTLLALHRSYLTPGDSSSGWTAGAAAYYVGYLQPRTFLLKYNENGTITDAVDCALDPLSETKCTLKSFTVEKGIYQTSNFRVQPTESIVRFPNITNLCPFGEVFNATRFASVYAWNRKRISNCVADYSVLYNSASFSTFKCYGVSPTKLNDLCFTNVYADSFVIRGDEVRQIAPGQTGKIADYNYKLPDDFTGCVIAWNSNNLDSKVGGNYNYLYRLFRKSNLKPFERDISTEIYQAGSTPCNGVEGFNCYFPLQSYGFQPTNGVGYQPYRVVVLSFELLHAPATVCGPKKSTNLVKNKCVNFNFNGLTGTGVLTESNKKFLPFQQFGRDIADTTDAVRDPQTLEILDITPCSFGGVSVITPGTNTSNQVAVLYQGVNCTEVPVAIHADQLTPTWRVYSTGSNVFQTRAGCLIGAEHVNNSYECDIPIGAGICASYQTQTNSPRRAASVASQSIIAYTMSLGAENSVAYSNNSIAIPTNFTISVTTEILPVSMTKTSVDCTMYICGDSTECSNLLLQYGSFCTQLNRALTGIAVEQDKNTQEVFAQVKQIYKTPPIKDFGGFNFSQILPDPSKPSKRSFIEDLLFNKVTLADAGFIKQYGDCLGDIAARDLICAQKFNGLTVLPPLLTDEMIAQYTSALLAGTITSGWTFGAGAALQIPFAMQMAYRFNGIGVTQNVLYENQKLIANQFNSAIGKIQDSLSSTASALGKLQDVVNQNAQALNTLVKQLSSNFGAISSVLNDILSRLDKVEAEVQIDRLITGRLQSLQTYVTQQLIRAAEIRASANLAATKMSECVLGQSKRVDFCGKGYHLMSFPQSAPHGVVFLHVTYVPAQEKNFTTAPAICHDGKAHFPREGVFVSNGTHWFVTQRNFYEPQIITTDNTFVSGNCDVVIGIVNNTVYDPLQPELDSFKEELDKYFKNHTSPDVDLGDISGINASVVNIQKEIDRLNEVAKNLNESLIDLQELGKYEQYIKRSNGLPGPIGPPGPRGRTGDAGPVGPPGPPGPPGPPGPPSAGFDFSFLPQPPQEKAHDGGRYYRANDANVVRDRDLEVDTTLKSLSQQIENIRSPEGSRKNPARTCRDLKMCHSDWKSGEYWIDPNQGCNLDAIKVFCNMETGETCVYPTQPSVAQKNWYISKNPKDKRHVWFGESMTDGFQFEYGGQGSDPADVAIQLTFLRLMSTEASQNITYHCKNSVAYMDQQTGNLKKALLLQGSNEIEIRAEGNSRFTYSVTVDGCTSHTGAWGKTVIEYKTTKTSRLPIIDVAPLDVGAPDQEFGFDVGPVCFL

SEQ ID NO: 24 - protein, 1509 aa, synthetic construct
  source 1..1509: note; note (original language) = SARS-CoV-2 variant D614G S-trimer fusion polypeptide without signal peptide, 1509 aa, proline mutant (986K/987V→986P/987P); organism (original language) = Synthetic construct
QCVNLTTRTQLPPAYTNSFTRGVYYPDKVFRSSVLHSTQDLFLPFFSNVTWFHAIHVSGTNGTKRFDNPVLPFNDGVYFASTEKSNIIRGWIFGTTLDSKTQSLLIVNNATNVVIKVCEFQFCNDPFLGVYYHKNNKSWMESEFRVYSSANNCTFEYVSQPFLMDLEGKQGNFKNLREFVFKNIDGYFKIYSKHTPINLVRDLPQGFSALEPLVDLPIGINITRFQTLLALHRSYLTPGDSSSGWTAGAAAYYVGYLQPRTFLLKYNENGTITDAVDCALDPLSETKCTLKSFTVEKGIYQTSNFRVQPTESIVRFPNITNLCPFGEVFNATRFASVYAWNRKRISNCVADYSVLYNSASFSTFKCYGVSPTKLNDLCFTNVYADSFVIRGDEVRQIAPGQTGKIADYNYKLPDDFTGCVIAWNSNNLDSKVGGNYNYLYRLFRKSNLKPFERDISTEIYQAGSTPCNGVEGFNCYFPLQSYGFQPTNGVGYQPYRVVVLSFELLHAPATVCGPKKSTNLVKNKCVNFNFNGLTGTGVLTESNKKFLPFQQFGRDIADTTDAVRDPQTLEILDITPCSFGGVSVITPGTNTSNQVAVLYQGVNCTEVPVAIHADQLTPTWRVYSTGSNVFQTRAGCLIGAEHVNNSYECDIPIGAGICASYQTQTNSPRRARSVASQSIIAYTMSLGAENSVAYSNNSIAIPTNFTISVTTEILPVSMTKTSVDCTMYICGDSTECSNLLLQYGSFCTQLNRALTGIAVEQDKNTQEVFAQVKQIYKTPPIKDFGGFNFSQILPDPSKPSKRSFIEDLLFNKVTLADAGFIKQYGDCLGDIAARDLICAQKFNGLTVLPPLLTDEMIAQYTSALLAGTITSGWTFGAGAALQIPFAMQMAYRFNGIGVTQNVLYENQKLIANQFNSAIGKIQDSLSSTASALGKLQDVVNQNAQALNTLVKQLSSNFGAISSVLNDILSRLDPPEAEVQIDRLITGRLQSLQTYVTQQLIRAAEIRASANLAATKMSECVLGQSKRVDFCGKGYHLMSFPQSAPHGVVFLHVTYVPAQEKNFTTAPAICHDGKAHFPREGVFVSNGTHWFVTQRNFYEPQIITTDNTFVSGNCDVVIGIVNNTVYDPLQPELDSFKEELDKYFKNHTSPDVDLGDISGINASVVNIQKEIDRLNEVAKNLNESLIDLQELGKYEQYIKRSNGLPGPIGPPGPRGRTGDAGPVGPPGPPGPPGPPGPPSAGFDFSFLPQPPQEKAHDGGRYYRANDANVVRDRDLEVDTTLKSLSQQIENIRSPEGSRKNPARTCRDLKMCHSDWKSGEYWIDPNQGCNLDAIKVFCNMETGETCVYPTQPSVAQKNWYISKNPKDKRHVWFGESMTDGFQFEYGGQGSDPADVAIQLTFLRLMSTEASQNITYHCKNSVAYMDQQTGNLKKALLLQGSNEIEIRAEGNSRFTYSVTVDGCTSHTGAWGKTVIEYKTTKTSRLPIIDVAPLDVGAPDQEFGFDVGPVCFL

SEQ ID NO: 25 - protein, 1509 aa, synthetic construct
  source 1..1509: note; note (original language) = SARS-CoV-2 variant D614G S-trimer fusion polypeptide without signal peptide, 1509 aa, S1/S2 furin cleavage site 1 and proline mutant (685R→685A, 986K/987V→986P/987P); organism (original language) = Synthetic construct
QCVNLTTRTQLPPAYTNSFTRGVYYPDKVFRSSVLHSTQDLFLPFFSNVTWFHAIHVSGTNGTKRFDNPVLPFNDGVYFASTEKSNIIRGWIFGTTLDSKTQSLLIVNNATNVVIKVCEFQFCNDPFLGVYYHKNNKSWMESEFRVYSSANNCTFEYVSQPFLMDLEGKQGNFKNLREFVFKNIDGYFKIYSKHTPINLVRDLPQGFSALEPLVDLPIGINITRFQTLLALHRSYLTPGDSSSGWTAGAAAYYVGYLQPRTFLLKYNENGTITDAVDCALDPLSETKCTLKSFTVEKGIYQTSNFRVQPTESIVRFPNITNLCPFGEVFNATRFASVYAWNRKRISNCVADYSVLYNSASFSTFKCYGVSPTKLNDLCFTNVYADSFVIRGDEVRQIAPGQTGKIADYNYKLPDDFTGCVIAWNSNNLDSKVGGNYNYLYRLFRKSNLKPFERDISTEIYQAGSTPCNGVEGFNCYFPLQSYGFQPTNGVGYQPYRVVVLSFELLHAPATVCGPKKSTNLVKNKCVNFNFNGLTGTGVLTESNKKFLPFQQFGRDIADTTDAVRDPQTLEILDITPCSFGGVSVITPGTNTSNQVAVLYQGVNCTEVPVAIHADQLTPTWRVYSTGSNVFQTRAGCLIGAEHVNNSYECDIPIGAGICASYQTQTNSPRRAASVASQSIIAYTMSLGAENSVAYSNNSIAIPTNFTISVTTEILPVSMTKTSVDCTMYICGDSTECSNLLLQYGSFCTQLNRALTGIAVEQDKNTQEVFAQVKQIYKTPPIKDFGGFNFSQILPDPSKPSKRSFIEDLLFNKVTLADAGFIKQYGDCLGDIAARDLICAQKFNGLTVLPPLLTDEMIAQYTSALLAGTITSGWTFGAGAALQIPFAMQMAYRFNGIGVTQNVLYENQKLIANQFNSAIGKIQDSLSSTASALGKLQDVVNQNAQALNTLVKQLSSNFGAISSVLNDILSRLDPPEAEVQIDRLITGRLQSLQTYVTQQLIRAAEIRASANLAATKMSECVLGQSKRVDFCGKGYHLMSFPQSAPHGVVFLHVTYVPAQEKNFTTAPAICHDGKAHFPREGVFVSNGTHWFVTQRNFYEPQIITTDNTFVSGNCDVVIGIVNNTVYDPLQPELDSFKEELDKYFKNHTSPDVDLGDISGINASVVNIQKEIDRLNEVAKNLNESLIDLQELGKYEQYIKRSNGLPGPIGPPGPRGRTGDAGPVGPPGPPGPPGPPGPPSAGFDFSFLPQPPQEKAHDGGRYYRANDANVVRDRDLEVDTTLKSLSQQIENIRSPEGSRKNPARTCRDLKMCHSDWKSGEYWIDPNQGCNLDAIKVFCNMETGETCVYPTQPSVAQKNWYISKNPKDKRHVWFGESMTDGFQFEYGGQGSDPADVAIQLTFLRLMSTEASQNITYHCKNSVAYMDQQTGNLKKALLLQGSNEIEIRAEGNSRFTYSVTVDGCTSHTGAWGKTVIEYKTTKTSRLPIIDVAPLDVGAPDQEFGFDVGPVCFL

SEQ ID NO: 26 - protein, 1491 aa, synthetic construct
  source 1..1491: note; note (original language) = SARS-CoV-1 S-trimer fusion polypeptide without signal peptide, 1491 aa; organism (original language) = Synthetic construct
SDLDRCTTFDDVQAPNYTQHTSSMRGVYYPDEIFRSDTLYLTQDLFLPFYSNVTGFHTINHTFDNPVIPFKDGIYFAATEKSNVVRGWVFGSTMNNKSQSVIIINNSTNVVIRACNFELCDNPFFAVSKPMGTQTHTMIFDNAFNCTFEYISDAFSLDVSEKSGNFKHLREFVFKNKDGFLYVYKGYQPIDVVRDLPSGFNTLKPIFKLPLGINITNFRAILTAFLPAQDTWGTSAAAYFVGYLKPTTFMLKYDENGTITDAVDCSQNPLAELKCSVKSFEIDKGIYQTSNFRVVPSRDVVRFPNITNLCPFGEVFNATKFPSVYAWERKRISNCVADYSVLYNSTFFSTFKCYGVSATKLNDLCFSNVYADSFVVKGDDVRQIAPGQTGVIADYNYKLPDDFMGCVLAWNTRNIDATSTGNYNYKYRYLRHGKLRPFERDISNVPFSPDGKPCTPPALNCYWPLNDYGFYTTTGIGYQPYRVVVLSFELLNAPATVCGPKLSTDLIKNQCVNFNFNGLTGTGVLTPSSKRFQPFQQFGRDVSDFTDSVRDPKTSEILDISPCSFGGVSVITPGTNASSEVAVLYQDVNCTDVSTAIHADQLTPAWRIYSTGNNVFQTQAGCLIGAEHVDTSYECDIPIGAGICASYHTVSLLRSTSQKSIVAYTMSLGADSSIAYSNNTIAIPTNFSISITTEVMPVSMAKTSVDCNMYICGDSTECANLLLQYGSFCTQLNRALSGIAAEQDRNTREVFAQVKQMYKTPTLKDFGGFNFSQILPDPLKPTKRSFIEDLLFNKVTLADAGFMKQYGECLGDINARDLICAQKFNGLTVLPPLLTDDMIAAYTAALVSGTATAGWTFGAGAALQIPFAMQMAYRFNGIGVTQNVLYENQKQIANQFNKAISQIQESLTTTSTALGKLQDVVNQNAQALNTLVKQLSSNFGAISSVLNDILSRLDKVEAEVQIDRLITGRLQSLQTYVTQQLIRAAEIRASANLAATKMSECVLGQSKRVDFCGKGYHLMSFPQAAPHGVVFLHVTYVPSQERNFTTAPAICHEGKAYFPREGVFVFNGTSWFITQRNFFSPQIITTDNTFVSGNCDVVIGIINNTVYDPLQPELDSFKEELDKYFKNHTSPDVDLGDISGINASVVNIQEEIDRLNEVAKNLNESLIDLQELGKYEQYIKRSNGLPGPIGPPGPRGRTGDAGPVGPPGPPGPPGPPGPPSAGFDFSFLPQPPQEKAHDGGRYYRANDANVVRDRDLEVDTTLKSLSQQIENIRSPEGSRKNPARTCRDLKMCHSDWKSGEYWIDPNQGCNLDAIKVFCNMETGETCVYPTQPSVAQKNWYISKNPKDKRHVWFGESMTDGFQFEYGGQGSDPADVAIQLTFLRLMSTEASQNITYHCKNSVAYMDQQTGNLKKALLLQGSNEIEIRAEGNSRFTYSVTVDGCTSHTGAWGKTVIEYKTTKTSRLPIIDVAPLDVGAPDQEFGFDVGPVCFL

SEQ ID NO: 27 - protein, 1195 aa, synthetic construct
  source 1..1195: note; note (original language) = Hu-1 SARS-CoV-2 spike protein extracellular domain without signal peptide; organism (original language) = Synthetic construct
QCVNLTTRTQLPPAYTNSFTRGVYYPDKVFRSSVLHSTQDLFLPFFSNVTWFHAIHVSGTNGTKRFDNPVLPFNDGVYFASTEKSNIIRGWIFGTTLDSKTQSLLIVNNATNVVIKVCEFQFCNDPFLGVYYHKNNKSWMESEFRVYSSANNCTFEYVSQPFLMDLEGKQGNFKNLREFVFKNIDGYFKIYSKHTPINLVRDLPQGFSALEPLVDLPIGINITRFQTLLALHRSYLTPGDSSSGWTAGAAAYYVGYLQPRTFLLKYNENGTITDAVDCALDPLSETKCTLKSFTVEKGIYQTSNFRVQPTESIVRFPNITNLCPFGEVFNATRFASVYAWNRKRISNCVADYSVLYNSASFSTFKCYGVSPTKLNDLCFTNVYADSFVIRGDEVRQIAPGQTGKIADYNYKLPDDFTGCVIAWNSNNLDSKVGGNYNYLYRLFRKSNLKPFERDISTEIYQAGSTPCNGVEGFNCYFPLQSYGFQPTNGVGYQPYRVVVLSFELLHAPATVCGPKKSTNLVKNKCVNFNFNGLTGTGVLTESNKKFLPFQQFGRDIADTTDAVRDPQTLEILDITPCSFGGVSVITPGTNTSNQVAVLYQDVNCTEVPVAIHADQLTPTWRVYSTGSNVFQTRAGCLIGAEHVNNSYECDIPIGAGICASYQTQTNSPRRARSVASQSIIAYTMSLGAENSVAYSNNSIAIPTNFTISVTTEILPVSMTKTSVDCTMYICGDSTECSNLLLQYGSFCTQLNRALTGIAVEQDKNTQEVFAQVKQIYKTPPIKDFGGFNFSQILPDPSKPSKRSFIEDLLFNKVTLADAGFIKQYGDCLGDIAARDLICAQKFNGLTVLPPLLTDEMIAQYTSALLAGTITSGWTFGAGAALQIPFAMQMAYRFNGIGVTQNVLYENQKLIANQFNSAIGKIQDSLSSTASALGKLQDVVNQNAQALNTLVKQLSSNFGAISSVLNDILSRLDKVEAEVQIDRLITGRLQSLQTYVTQQLIRAAEIRASANLAATKMSECVLGQSKRVDFCGKGYHLMSFPQSAPHGVVFLHVTYVPAQEKNFTTAPAICHDGKAHFPREGVFVSNGTHWFVTQRNFYEPQIITTDNTFVSGNCDVVIGIVNNTVYDPLQPELDSFKEELDKYFKNHTSPDVDLGDISGINASVVNIQKEIDRLNEVAKNLNESLIDLQELGKYEQ

SEQ ID NO: 28 - protein, 1195 aa, synthetic construct
  source 1..1195: note; note (original language) = Hu-1 SARS-CoV-2 spike protein extracellular domain without signal peptide, S1/S2 furin cleavage site 1 mutant (685R→685A); organism (original language) = Synthetic construct
QCVNLTTRTQLPPAYTNSFTRGVYYPDKVFRSSVLHSTQDLFLPFFSNVTWFHAIHVSGTNGTKRFDNPVLPFNDGVYFASTEKSNIIRGWIFGTTLDSKTQSLLIVNNATNVVIKVCEFQFCNDPFLGVYYHKNNKSWMESEFRVYSSANNCTFEYVSQPFLMDLEGKQGNFKNLREFVFKNIDGYFKIYSKHTPINLVRDLPQGFSALEPLVDLPIGINITRFQTLLALHRSYLTPGDSSSGWTAGAAAYYVGYLQPRTFLLKYNENGTITDAVDCALDPLSETKCTLKSFTVEKGIYQTSNFRVQPTESIVRFPNITNLCPFGEVFNATRFASVYAWNRKRISNCVADYSVLYNSASFSTFKCYGVSPTKLNDLCFTNVYADSFVIRGDEVRQIAPGQTGKIADYNYKLPDDFTGCVIAWNSNNLDSKVGGNYNYLYRLFRKSNLKPFERDISTEIYQAGSTPCNGVEGFNCYFPLQSYGFQPTNGVGYQPYRVVVLSFELLHAPATVCGPKKSTNLVKNKCVNFNFNGLTGTGVLTESNKKFLPFQQFGRDIADTTDAVRDPQTLEILDITPCSFGGVSVITPGTNTSNQVAVLYQDVNCTEVPVAIHADQLTPTWRVYSTGSNVFQTRAGCLIGAEHVNNSYECDIPIGAGICASYQTQTNSPRRAASVASQSIIAYTMSLGAENSVAYSNNSIAIPTNFTISVTTEILPVSMTKTSVDCTMYICGDSTECSNLLLQYGSFCTQLNRALTGIAVEQDKNTQEVFAQVKQIYKTPPIKDFGGFNFSQILPDPSKPSKRSFIEDLLFNKVTLADAGFIKQYGDCLGDIAARDLICAQKFNGLTVLPPLLTDEMIAQYTSALLAGTITSGWTFGAGAALQIPFAMQMAYRFNGIGVTQNVLYENQKLIANQFNSAIGKIQDSLSSTASALGKLQDVVNQNAQALNTLVKQLSSNFGAISSVLNDILSRLDKVEAEVQIDRLITGRLQSLQTYVTQQLIRAAEIRASANLAATKMSECVLGQSKRVDFCGKGYHLMSFPQSAPHGVVFLHVTYVPAQEKNFTTAPAICHDGKAHFPREGVFVSNGTHWFVTQRNFYEPQIITTDNTFVSGNCDVVIGIVNNTVYDPLQPELDSFKEELDKYFKNHTSPDVDLGDISGINASVVNIQKEIDRLNEVAKNLNESLIDLQELGKYEQ

SEQ ID NO: 29 - protein, 1195 aa, synthetic construct
  source 1..1195: note; note (original language) = Hu-1 SARS-CoV-2 spike protein extracellular domain without signal peptide, proline mutant (986K/987V→986P/987P); organism (original language) = Synthetic construct
QCVNLTTRTQLPPAYTNSFTRGVYYPDKVFRSSVLHSTQDLFLPFFSNVTWFHAIHVSGTNGTKRFDNPVLPFNDGVYFASTEKSNIIRGWIFGTTLDSKTQSLLIVNNATNVVIKVCEFQFCNDPFLGVYYHKNNKSWMESEFRVYSSANNCTFEYVSQPFLMDLEGKQGNFKNLREFVFKNIDGYFKIYSKHTPINLVRDLPQGFSALEPLVDLPIGINITRFQTLLALHRSYLTPGDSSSGWTAGAAAYYVGYLQPRTFLLKYNENGTITDAVDCALDPLSETKCTLKSFTVEKGIYQTSNFRVQPTESIVRFPNITNLCPFGEVFNATRFASVYAWNRKRISNCVADYSVLYNSASFSTFKCYGVSPTKLNDLCFTNVYADSFVIRGDEVRQIAPGQTGKIADYNYKLPDDFTGCVIAWNSNNLDSKVGGNYNYLYRLFRKSNLKPFERDISTEIYQAGSTPCNGVEGFNCYFPLQSYGFQPTNGVGYQPYRVVVLSFELLHAPATVCGPKKSTNLVKNKCVNFNFNGLTGTGVLTESNKKFLPFQQFGRDIADTTDAVRDPQTLEILDITPCSFGGVSVITPGTNTSNQVAVLYQDVNCTEVPVAIHADQLTPTWRVYSTGSNVFQTRAGCLIGAEHVNNSYECDIPIGAGICASYQTQTNSPRRARSVASQSIIAYTMSLGAENSVAYSNNSIAIPTNFTISVTTEILPVSMTKTSVDCTMYICGDSTECSNLLLQYGSFCTQLNRALTGIAVEQDKNTQEVFAQVKQIYKTPPIKDFGGFNFSQILPDPSKPSKRSFIEDLLFNKVTLADAGFIKQYGDCLGDIAARDLICAQKFNGLTVLPPLLTDEMIAQYTSALLAGTITSGWTFGAGAALQIPFAMQMAYRFNGIGVTQNVLYENQKLIANQFNSAIGKIQDSLSSTASALGKLQDVVNQNAQALNTLVKQLSSNFGAISSVLNDILSRLDPPEAEVQIDRLITGRLQSLQTYVTQQLIRAAEIRASANLAATKMSECVLGQSKRVDFCGKGYHLMSFPQSAPHGVVFLHVTYVPAQEKNFTTAPAICHDGKAHFPREGVFVSNGTHWFVTQRNFYEPQIITTDNTFVSGNCDVVIGIVNNTVYDPLQPELDSFKEELDKYFKNHTSPDVDLGDISGINASVVNIQKEIDRLNEVAKNLNESLIDLQELGKYEQ

SEQ ID NO: 30 - protein, 1195 aa, synthetic construct
  source 1..1195: note; note (original language) = Hu-1 SARS-CoV-2 spike protein extracellular domain without signal peptide, S1/S2 furin cleavage site 1 and proline mutant (685R→685A, 986K/987V→986P/987P); organism (original language) = Synthetic construct
QCVNLTTRTQLPPAYTNSFTRGVYYPDKVFRSSVLHSTQDLFLPFFSNVTWFHAIHVSGTNGTKRFDNPVLPFNDGVYFASTEKSNIIRGWIFGTTLDSKTQSLLIVNNATNVVIKVCEFQFCNDPFLGVYYHKNNKSWMESEFRVYSSANNCTFEYVSQPFLMDLEGKQGNFKNLREFVFKNIDGYFKIYSKHTPINLVRDLPQGFSALEPLVDLPIGINITRFQTLLALHRSYLTPGDSSSGWTAGAAAYYVGYLQPRTFLLKYNENGTITDAVDCALDPLSETKCTLKSFTVEKGIYQTSNFRVQPTESIVRFPNITNLCPFGEVFNATRFASVYAWNRKRISNCVADYSVLYNSASFSTFKCYGVSPTKLNDLCFTNVYADSFVIRGDEVRQIAPGQTGKIADYNYKLPDDFTGCVIAWNSNNLDSKVGGNYNYLYRLFRKSNLKPFERDISTEIYQAGSTPCNGVEGFNCYFPLQSYGFQPTNGVGYQPYRVVVLSFELLHAPATVCGPKKSTNLVKNKCVNFNFNGLTGTGVLTESNKKFLPFQQFGRDIADTTDAVRDPQTLEILDITPCSFGGVSVITPGTNTSNQVAVLYQDVNCTEVPVAIHADQLTPTWRVYSTGSNVFQTRAGCLIGAEHVNNSYECDIPIGAGICASYQTQTNSPRRAASVASQSIIAYTMSLGAENSVAYSNNSIAIPTNFTISVTTEILPVSMTKTSVDCTMYICGDSTECSNLLLQYGSFCTQLNRALTGIAVEQDKNTQEVFAQVKQIYKTPPIKDFGGFNFSQILPDPSKPSKRSFIEDLLFNKVTLADAGFIKQYGDCLGDIAARDLICAQKFNGLTVLPPLLTDEMIAQYTSALLAGTITSGWTFGAGAALQIPFAMQMAYRFNGIGVTQNVLYENQKLIANQFNSAIGKIQDSLSSTASALGKLQDVVNQNAQALNTLVKQLSSNFGAISSVLNDILSRLDPPEAEVQIDRLITGRLQSLQTYVTQQLIRAAEIRASANLAATKMSECVLGQSKRVDFCGKGYHLMSFPQSAPHGVVFLHVTYVPAQEKNFTTAPAICHDGKAHFPREGVFVSNGTHWFVTQRNFYEPQIITTDNTFVSGNCDVVIGIVNNTVYDPLQPELDSFKEELDKYFKNHTSPDVDLGDISGINASVVNIQKEIDRLNEVAKNLNESLIDLQELGKYEQ

SEQ ID NO: 31 - protein, 525 aa, synthetic construct
  source 1..525: note; note (original language) = Hu-1 SARS-CoV-2 spike protein NTD/RBD fragment without signal peptide; organism (original language) = Synthetic construct
QCVNLTTRTQLPPAYTNSFTRGVYYPDKVFRSSVLHSTQDLFLPFFSNVTWFHAIHVSGTNGTKRFDNPVLPFNDGVYFASTEKSNIIRGWIFGTTLDSKTQSLLIVNNATNVVIKVCEFQFCNDPFLGVYYHKNNKSWMESEFRVYSSANNCTFEYVSQPFLMDLEGKQGNFKNLREFVFKNIDGYFKIYSKHTPINLVRDLPQGFSALEPLVDLPIGINITRFQTLLALHRSYLTPGDSSSGWTAGAAAYYVGYLQPRTFLLKYNENGTITDAVDCALDPLSETKCTLKSFTVEKGIYQTSNFRVQPTESIVRFPNITNLCPFGEVFNATRFASVYAWNRKRISNCVADYSVLYNSASFSTFKCYGVSPTKLNDLCFTNVYADSFVIRGDEVRQIAPGQTGKIADYNYKLPDDFTGCVIAWNSNNLDSKVGGNYNYLYRLFRKSNLKPFERDISTEIYQAGSTPCNGVEGFNCYFPLQSYGFQPTNGVGYQPYRVVVLSFELLHAPATVCGPKKSTNLVKNKC

SEQ ID NO: 32 - protein, 668 aa, synthetic construct
  source 1..668: note; note (original language) = Hu-1 SARS-CoV-2 spike protein S1 fragment without signal peptide; organism (original language) = Synthetic construct
QCVNLTTRTQLPPAYTNSFTRGVYYPDKVFRSSVLHSTQDLFLPFFSNVTWFHAIHVSGTNGTKRFDNPVLPFNDGVYFASTEKSNIIRGWIFGTTLDSKTQSLLIVNNATNVVIKVCEFQFCNDPFLGVYYHKNNKSWMESEFRVYSSANNCTFEYVSQPFLMDLEGKQGNFKNLREFVFKNIDGYFKIYSKHTPINLVRDLPQGFSALEPLVDLPIGINITRFQTLLALHRSYLTPGDSSSGWTAGAAAYYVGYLQPRTFLLKYNENGTITDAVDCALDPLSETKCTLKSFTVEKGIYQTSNFRVQPTESIVRFPNITNLCPFGEVFNATRFASVYAWNRKRISNCVADYSVLYNSASFSTFKCYGVSPTKLNDLCFTNVYADSFVIRGDEVRQIAPGQTGKIADYNYKLPDDFTGCVIAWNSNNLDSKVGGNYNYLYRLFRKSNLKPFERDISTEIYQAGSTPCNGVEGFNCYFPLQSYGFQPTNGVGYQPYRVVVLSFELLHAPATVCGPKKSTNLVKNKCVNFNFNGLTGTGVLTESNKKFLPFQQFGRDIADTTDAVRDPQTLEILDITPCSFGGVSVITPGTNTSNQVAVLYQDVNCTEVPVAIHADQLTPTWRVYSTGSNVFQTRAGCLIGAEHVNNSYECDIPIGAGICASYQTQTNSP

SEQ ID NO: 33 - protein, 523 aa, synthetic construct
  source 1..523: note; note (original language) = Hu-1 SARS-CoV-2 spike protein S2 fragment (cleaved at site 1, S1/S2); organism (original language) = Synthetic construct
SVASQSIIAYTMSLGAENSVAYSNNSIAIPTNFTISVTTEILPVSMTKTSVDCTMYICGDSTECSNLLLQYGSFCTQLNRALTGIAVEQDKNTQEVFAQVKQIYKTPPIKDFGGFNFSQILPDPSKPSKRSFIEDLLFNKVTLADAGFIKQYGDCLGDIAARDLICAQKFNGLTVLPPLLTDEMIAQYTSALLAGTITSGWTFGAGAALQIPFAMQMAYRFNGIGVTQNVLYENQKLIANQFNSAIGKIQDSLSSTASALGKLQDVVNQNAQALNTLVKQLSSNFGAISSVLNDILSRLDKVEAEVQIDRLITGRLQSLQTYVTQQLIRAAEIRASANLAATKMSECVLGQSKRVDFCGKGYHLMSFPQSAPHGVVFLHVTYVPAQEKNFTTAPAICHDGKAHFPREGVFVSNGTHWFVTQRNFYEPQIITTDNTFVSGNCDVVIGIVNNTVYDPLQPELDSFKEELDKYFKNHTSPDVDLGDISGINASVVNIQKEIDRLNEVAKNLNESLIDLQELGKYEQ

SEQ ID NO: 34 - protein, 513 aa, synthetic construct
  source 1..513: note; note (original language) = Hu-1 SARS-CoV-2 spike protein S2 fragment (cleaved at site 2, S1/S2); organism (original language) = Synthetic construct
TMSLGAENSVAYSNNSIAIPTNFTISVTTEILPVSMTKTSVDCTMYICGDSTECSNLLLQYGSFCTQLNRALTGIAVEQDKNTQEVFAQVKQIYKTPPIKDFGGFNFSQILPDPSKPSKRSFIEDLLFNKVTLADAGFIKQYGDCLGDIAARDLICAQKFNGLTVLPPLLTDEMIAQYTSALLAGTITSGWTFGAGAALQIPFAMQMAYRFNGIGVTQNVLYENQKLIANQFNSAIGKIQDSLSSTASALGKLQDVVNQNAQALNTLVKQLSSNFGAISSVLNDILSRLDKVEAEVQIDRLITGRLQSLQTYVTQQLIRAAEIRASANLAATKMSECVLGQSKRVDFCGKGYHLMSFPQSAPHGVVFLHVTYVPAQEKNFTTAPAICHDGKAHFPREGVFVSNGTHWFVTQRNFYEPQIITTDNTFVSGNCDVVIGIVNNTVYDPLQPELDSFKEELDKYFKNHTSPDVDLGDISGINASVVNIQKEIDRLNEVAKNLNESLIDLQELGKYEQ

SEQ ID NO: 35 - protein, 393 aa, synthetic construct
  source 1..393: note; note (original language) = Hu-1 SARS-CoV-2 spike protein S2 fragment (cleaved at S2'); organism (original language) = Synthetic construct
SFIEDLLFNKVTLADAGFIKQYGDCLGDIAARDLICAQKFNGLTVLPPLLTDEMIAQYTSALLAGTITSGWTFGAGAALQIPFAMQMAYRFNGIGVTQNVLYENQKLIANQFNSAIGKIQDSLSSTASALGKLQDVVNQNAQALNTLVKQLSSNFGAISSVLNDILSRLDKVEAEVQIDRLITGRLQSLQTYVTQQLIRAAEIRASANLAATKMSECVLGQSKRVDFCGKGYHLMSFPQSAPHGVVFLHVTYVPAQEKNFTTAPAICHDGKAHFPREGVFVSNGTHWFVTQRNFYEPQIITTDNTFVSGNCDVVIGIVNNTVYDPLQPELDSFKEELDKYFKNHTSPDVDLGDISGINASVVNIQKEIDRLNEVAKNLNESLIDLQELGKYEQ

SEQ ID NO: 36 - protein, 1195 aa, synthetic construct
  source 1..1195: note; note (original language) = SARS-CoV-2 South African variant B.1.351 spike protein extracellular domain without signal peptide; organism (original language) = Synthetic construct
QCVNLTTRTQLPPAYTNSFTRGVYYPDKVFRSSVLHSTQDLFLPFFSNVTWFHAIHVSGTNGTKRFDNPVLPFNDGVYFASTEKSNIIRGWIFGTTLDSKTQSLLIVNNATNVVIKVCEFQFCNDPFLGVYYHKNNKSWMESEFRVYSSANNCTFEYVSQPFLMDLEGKQGNFKNLREFVFKNIDGYFKIYSKHTPINLVRDLPQGFSALEPLVDLPIGINITRFQTLLALHRSYLTPGDSSSGWTAGAAAYYVGYLQPRTFLLKYNENGTITDAVDCALDPLSETKCTLKSFTVEKGIYQTSNFRVQPTESIVRFPNITNLCPFGEVFNATRFASVYAWNRKRISNCVADYSVLYNSASFSTFKCYGVSPTKLNDLCFTNVYADSFVIRGDEVRQIAPGQTGNIADYNYKLPDDFTGCVIAWNSNNLDSKVGGNYNYLYRLFRKSNLKPFERDISTEIYQAGSTPCNGVKGFNCYFPLQSYGFQPTYGVGYQPYRVVVLSFELLHAPATVCGPKKSTNLVKNKCVNFNFNGLTGTGVLTESNKKFLPFQQFGRDIADTTDAVRDPQTLEILDITPCSFGGVSVITPGTNTSNQVAVLYQGVNCTEVPVAIHADQLTPTWRVYSTGSNVFQTRAGCLIGAEHVNNSYECDIPIGAGICASYQTQTNSPRRARSVASQSIIAYTMSLGAENSVAYSNNSIAIPTNFTISVTTEILPVSMTKTSVDCTMYICGDSTECSNLLLQYGSFCTQLNRALTGIAVEQDKNTQEVFAQVKQIYKTPPIKDFGGFNFSQILPDPSKPSKRSFIEDLLFNKVTLADAGFIKQYGDCLGDIAARDLICAQKFNGLTVLPPLLTDEMIAQYTSALLAGTITSGWTFGAGAALQIPFAMQMAYRFNGIGVTQNVLYENQKLIANQFNSAIGKIQDSLSSTASALGKLQDVVNQNAQALNTLVKQLSSNFGAISSVLNDILSRLDKVEAEVQIDRLITGRLQSLQTYVTQQLIRAAEIRASANLAATKMSECVLGQSKRVDFCGKGYHLMSFPQSAPHGVVFLHVTYVPAQEKNFTTAPAICHDGKAHFPREGVFVSNGTHWFVTQRNFYEPQIITTDNTFVSGNCDVVIGIVNNTVYDPLQPELDSFKEELDKYFKNHTSPDVDLGDISGINASVVNIQKEIDRLNEVAKNLNESLIDLQELGKYEQ

SEQ ID NO: 37 - protein, 1195 aa, synthetic construct
  source 1..1195: note; note (original language) = SARS-CoV-2 South African variant B.1.351 spike protein extracellular domain without signal peptide, S1/S2 furin cleavage site 1 mutant (685R→685A); organism (original language) = Synthetic construct
QCVNLTTRTQLPPAYTNSFTRGVYYPDKVFRSSVLHSTQDLFLPFFSNVTWFHAIHVSGTNGTKRFDNPVLPFNDGVYFASTEKSNIIRGWIFGTTLDSKTQSLLIVNNATNVVIKVCEFQFCNDPFLGVYYHKNNKSWMESEFRVYSSANNCTFEYVSQPFLMDLEGKQGNFKNLREFVFKNIDGYFKIYSKHTPINLVRDLPQGFSALEPLVDLPIGINITRFQTLLALHRSYLTPGDSSSGWTAGAAAYYVGYLQPRTFLLKYNENGTITDAVDCALDPLSETKCTLKSFTVEKGIYQTSNFRVQPTESIVRFPNITNLCPFGEVFNATRFASVYAWNRKRISNCVADYSVLYNSASFSTFKCYGVSPTKLNDLCFTNVYADSFVIRGDEVRQIAPGQTGNIADYNYKLPDDFTGCVIAWNSNNLDSKVGGNYNYLYRLFRKSNLKPFERDISTEIYQAGSTPCNGVKGFNCYFPLQSYGFQPTYGVGYQPYRVVVLSFELLHAPATVCGPKKSTNLVKNKCVNFNFNGLTGTGVLTESNKKFLPFQQFGRDIADTTDAVRDPQTLEILDITPCSFGGVSVITPGTNTSNQVAVLYQGVNCTEVPVAIHADQLTPTWRVYSTGSNVFQTRAGCLIGAEHVNNSYECDIPIGAGICASYQTQTNSPRRAASVASQSIIAYTMSLGAENSVAYSNNSIAIPTNFTISVTTEILPVSMTKTSVDCTMYICGDSTECSNLLLQYGSFCTQLNRALTGIAVEQDKNTQEVFAQVKQIYKTPPIKDFGGFNFSQILPDPSKPSKRSFIEDLLFNKVTLADAGFIKQYGDCLGDIAARDLICAQKFNGLTVLPPLLTDEMIAQYTSALLAGTITSGWTFGAGAALQIPFAMQMAYRFNGIGVTQNVLYENQKLIANQFNSAIGKIQDSLSSTASALGKLQDVVNQNAQALNTLVKQLSSNFGAISSVLNDILSRLDKVEAEVQIDRLITGRLQSLQTYVTQQLIRAAEIRASANLAATKMSECVLGQSKRVDFCGKGYHLMSFPQSAPHGVVFLHVTYVPAQEKNFTTAPAICHDGKAHFPREGVFVSNGTHWFVTQRNFYEPQIITTDNTFVSGNCDVVIGIVNNTVYDPLQPELDSFKEELDKYFKNHTSPDVDLGDISGINASVVNIQKEIDRLNEVAKNLNESLIDLQELGKYEQ

SEQ ID NO: 38 - protein, 1195 aa, synthetic construct
  source 1..1195: note; note (original language) = SARS-CoV-2 South African variant B.1.351 spike protein extracellular domain without signal peptide, proline mutant (986K/987V→986P/987P); organism (original language) = Synthetic construct
QCVNLTTRTQLPPAYTNSFTRGVYYPDKVFRSSVLHSTQDLFLPFFSNVTWFHAIHVSGTNGTKRFDNPVLPFNDGVYFASTEKSNIIRGWIFGTTLDSKTQSLLIVNNATNVVIKVCEFQFCNDPFLGVYYHKNNKSWMESEFRVYSSANNCTFEYVSQPFLMDLEGKQGNFKNLREFVFKNIDGYFKIYSKHTPINLVRDLPQGFSALEPLVDLPIGINITRFQTLLALHRSYLTPGDSSSGWTAGAAAYYVGYLQPRTFLLKYNENGTITDAVDCALDPLSETKCTLKSFTVEKGIYQTSNFRVQPTESIVRFPNITNLCPFGEVFNATRFASVYAWNRKRISNCVADYSVLYNSASFSTFKCYGVSPTKLNDLCFTNVYADSFVIRGDEVRQIAPGQTGNIADYNYKLPDDFTGCVIAWNSNNLDSKVGGNYNYLYRLFRKSNLKPFERDISTEIYQAGSTPCNGVKGFNCYFPLQSYGFQPTYGVGYQPYRVVVLSFELLHAPATVCGPKKSTNLVKNKCVNFNFNGLTGTGVLTESNKKFLPFQQFGRDIADTTDAVRDPQTLEILDITPCSFGGVSVITPGTNTSNQVAVLYQGVNCTEVPVAIHADQLTPTWRVYSTGSNVFQTRAGCLIGAEHVNNSYECDIPIGAGICASYQTQTNSPRRARSVASQSIIAYTMSLGAENSVAYSNNSIAIPTNFTISVTTEILPVSMTKTSVDCTMYICGDSTECSNLLLQYGSFCTQLNRALTGIAVEQDKNTQEVFAQVKQIYKTPPIKDFGGFNFSQILPDPSKPSKRSFIEDLLFNKVTLADAGFIKQYGDCLGDIAARDLICAQKFNGLTVLPPLLTDEMIAQYTSALLAGTITSGWTFGAGAALQIPFAMQMAYRFNGIGVTQNVLYENQKLIANQFNSAIGKIQDSLSSTASALGKLQDVVNQNAQALNTLVKQLSSNFGAISSVLNDILSRLDPPEAEVQIDRLITGRLQSLQTYVTQQLIRAAEIRASANLAATKMSECVLGQSKRVDFCGKGYHLMSFPQSAPHGVVFLHVTYVPAQEKNFTTAPAICHDGKAHFPREGVFVSNGTHWFVTQRNFYEPQIITTDNTFVSGNCDVVIGIVNNTVYDPLQPELDSFKEELDKYFKNHTSPDVDLGDISGINASVVNIQKEIDRLNEVAKNLNESLIDLQELGKYEQ

SEQ ID NO: 39 - protein, 1195 aa, synthetic construct
  source 1..1195: note; note (original language) = SARS-CoV-2 South African variant B.1.351 spike protein extracellular domain without signal peptide, S1/S2 furin cleavage site 1 and proline mutant (685R→685A, 986K/987V→986P/987P); organism (original language) = Synthetic construct
QCVNLTTRTQLPPAYTNSFTRGVYYPDKVFRSSVLHSTQDLFLPFFSNVTWFHAIHVSGTNGTKRFDNPVLPFNDGVYFASTEKSNIIRGWIFGTTLDSKTQSLLIVNNATNVVIKVCEFQFCNDPFLGVYYHKNNKSWMESEFRVYSSANNCTFEYVSQPFLMDLEGKQGNFKNLREFVFKNIDGYFKIYSKHTPINLVRDLPQGFSALEPLVDLPIGINITRFQTLLALHRSYLTPGDSSSGWTAGAAAYYVGYLQPRTFLLKYNENGTITDAVDCALDPLSETKCTLKSFTVEKGIYQTSNFRVQPTESIVRFPNITNLCPFGEVFNATRFASVYAWNRKRISNCVADYSVLYNSASFSTFKCYGVSPTKLNDLCFTNVYADSFVIRGDEVRQIAPGQTGNIADYNYKLPDDFTGCVIAWNSNNLDSKVGGNYNYLYRLFRKSNLKPFERDISTEIYQAGSTPCNGVKGFNCYFPLQSYGFQPTYGVGYQPYRVVVLSFELLHAPATVCGPKKSTNLVKNKCVNFNFNGLTGTGVLTESNKKFLPFQQFGRDIADTTDAVRDPQTLEILDITPCSFGGVSVITPGTNTSNQVAVLYQGVNCTEVPVAIHADQLTPTWRVYSTGSNVFQTRAGCLIGAEHVNNSYECDIPIGAGICASYQTQTNSPRRAASVASQSIIAYTMSLGAENSVAYSNNSIAIPTNFTISVTTEILPVSMTKTSVDCTMYICGDSTECSNLLLQYGSFCTQLNRALTGIAVEQDKNTQEVFAQVKQIYKTPPIKDFGGFNFSQILPDPSKPSKRSFIEDLLFNKVTLADAGFIKQYGDCLGDIAARDLICAQKFNGLTVLPPLLTDEMIAQYTSALLAGTITSGWTFGAGAALQIPFAMQMAYRFNGIGVTQNVLYENQKLIANQFNSAIGKIQDSLSSTASALGKLQDVVNQNAQALNTLVKQLSSNFGAISSVLNDILSRLDPPEAEVQIDRLITGRLQSLQTYVTQQLIRAAEIRASANLAATKMSECVLGQSKRVDFCGKGYHLMSFPQSAPHGVVFLHVTYVPAQEKNFTTAPAICHDGKAHFPREGVFVSNGTHWFVTQRNFYEPQIITTDNTFVSGNCDVVIGIVNNTVYDPLQPELDSFKEELDKYFKNHTSPDVDLGDISGINASVVNIQKEIDRLNEVAKNLNESLIDLQELGKYEQ

SEQ ID NO: 40 - protein, 1195 aa, synthetic construct
  source 1..1195: note; note (original language) = SARS-CoV-2 Brazilian variant P.1 spike protein extracellular domain without signal peptide; organism (original language) = Synthetic construct
QCVNFTNRTQLPSAYTNSFTRGVYYPDKVFRSSVLHSTQDLFLPFFSNVTWFHAIHVSGTNGTKRFDNPVLPFNDGVYFASTEKSNIIRGWIFGTTLDSKTQSLLIVNNATNVVIKVCEFQFCNYPFLGVYYHKNNKSWMESEFRVYSSANNCTFEYVSQPFLMDLEGKQGNFKNLSEFVFKNIDGYFKIYSKHTPINLVRDLPQGFSALEPLVDLPIGINITRFQTLLALHRSYLTPGDSSSGWTAGAAAYYVGYLQPRTFLLKYNENGTITDAVDCALDPLSETKCTLKSFTVEKGIYQTSNFRVQPTESIVRFPNITNLCPFGEVFNATRFASVYAWNRKRISNCVADYSVLYNSASFSTFKCYGVSPTKLNDLCFTNVYADSFVIRGDEVRQIAPGQTGTIADYNYKLPDDFTGCVIAWNSNNLDSKVGGNYNYLYRLFRKSNLKPFERDISTEIYQAGSTPCNGVKGFNCYFPLQSYGFQPTYGVGYQPYRVVVLSFELLHAPATVCGPKKSTNLVKNKCVNFNFNGLTGTGVLTESNKKFLPFQQFGRDIADTTDAVRDPQTLEILDITPCSFGGVSVITPGTNTSNQVAVLYQGVNCTEVPVAIHADQLTPTWRVYSTGSNVFQTRAGCLIGAEYVNNSYECDIPIGAGICASYQTQTNSPRRARSVASQSIIAYTMSLGAENSVAYSNNSIAIPTNFTISVTTEILPVSMTKTSVDCTMYICGDSTECSNLLLQYGSFCTQLNRALTGIAVEQDKNTQEVFAQVKQIYKTPPIKDFGGFNFSQILPDPSKPSKRSFIEDLLFNKVTLADAGFIKQYGDCLGDIAARDLICAQKFNGLTVLPPLLTDEMIAQYTSALLAGTITSGWTFGAGAALQIPFAMQMAYRFNGIGVTQNVLYENQKLIANQFNSAIGKIQDSLSSTASALGKLQDVVNQNAQALNTLVKQLSSNFGAISSVLNDILSRLDKVEAEVQIDRLITGRLQSLQTYVTQQLIRAAEIRASANLAAIKMSECVLGQSKRVDFCGKGYHLMSFPQSAPHGVVFLHVTYVPAQEKNFTTAPAICHDGKAHFPREGVFVSNGTHWFVTQRNFYEPQIITTDNTFVSGNCDVVIGIVNNTVYDPLQPELDSFKEELDKYFKNHTSPDVDLGDISGINASVVNIQKEIDRLNEVAKNLNESLIDLQELGKYEQ

SEQ ID NO: 41 - protein, 1195 aa, synthetic construct
  source 1..1195: note; note (original language) = SARS-CoV-2 Brazilian variant P.1 spike protein extracellular domain without signal peptide, S1/S2 furin cleavage site 1 mutant (685R→685A); organism (original language) = Synthetic construct
QCVNFTNRTQLPSAYTNSFTRGVYYPDKVFRSSVLHSTQDLFLPFFSNVTWFHAIHVSGTNGTKRFDNPVLPFNDGVYFASTEKSNIIRGWIFGTTLDSKTQSLLIVNNATNVVIKVCEFQFCNYPFLGVYYHKNNKSWMESEFRVYSSANNCTFEYVSQPFLMDLEGKQGNFKNLSEFVFKNIDGYFKIYSKHTPINLVRDLPQGFSALEPLVDLPIGINITRFQTLLALHRSYLTPGDSSSGWTAGAAAYYVGYLQPRTFLLKYNENGTITDAVDCALDPLSETKCTLKSFTVEKGIYQTSNFRVQPTESIVRFPNITNLCPFGEVFNATRFASVYAWNRKRISNCVADYSVLYNSASFSTFKCYGVSPTKLNDLCFTNVYADSFVIRGDEVRQIAPGQTGTIADYNYKLPDDFTGCVIAWNSNNLDSKVGGNYNYLYRLFRKSNLKPFERDISTEIYQAGSTPCNGVKGFNCYFPLQSYGFQPTYGVGYQPYRVVVLSFELLHAPATVCGPKKSTNLVKNKCVNFNFNGLTGTGVLTESNKKFLPFQQFGRDIADTTDAVRDPQTLEILDITPCSFGGVSVITPGTNTSNQVAVLYQGVNCTEVPVAIHADQLTPTWRVYSTGSNVFQTRAGCLIGAEYVNNSYECDIPIGAGICASYQTQTNSPRRAASVASQSIIAYTMSLGAENSVAYSNNSIAIPTNFTISVTTEILPVSMTKTSVDCTMYICGDSTECSNLLLQYGSFCTQLNRALTGIAVEQDKNTQEVFAQVKQIYKTPPIKDFGGFNFSQILPDPSKPSKRSFIEDLLFNKVTLADAGFIKQYGDCLGDIAARDLICAQKFNGLTVLPPLLTDEMIAQYTSALLAGTITSGWTFGAGAALQIPFAMQMAYRFNGIGVTQNVLYENQKLIANQFNSAIGKIQDSLSSTASALGKLQDVVNQNAQALNTLVKQLSSNFGAISSVLNDILSRLDKVEAEVQIDRLITGRLQSLQTYVTQQLIRAAEIRASANLAAIKMSECVLGQSKRVDFCGKGYHLMSFPQSAPHGVVFLHVTYVPAQEKNFTTAPAICHDGKAHFPREGVFVSNGTHWFVTQRNFYEPQIITTDNTFVSGNCDVVIGIVNNTVYDPLQPELDSFKEELDKYFKNHTSPDVDLGDISGINASVVNIQKEIDRLNEVAKNLNESLIDLQELGKYEQ

SEQ ID NO: 42 - protein, 1195 aa, synthetic construct
  source 1..1195: note; note (original language) = SARS-CoV-2 Brazilian variant P.1 spike protein extracellular domain without signal peptide, proline mutant (986K/987V→986P/987P); organism (original language) = Synthetic construct
QCVNFTNRTQLPSAYTNSFTRGVYYPDKVFRSSVLHSTQDLFLPFFSNVTWFHAIHVSGTNGTKRFDNPVLPFNDGVYFASTEKSNIIRGWIFGTTLDSKTQSLLIVNNATNVVIKVCEFQFCNYPFLGVYYHKNNKSWMESEFRVYSSANNCTFEYVSQPFLMDLEGKQGNFKNLSEFVFKNIDGYFKIYSKHTPINLVRDLPQGFSALEPLVDLPIGINITRFQTLLALHRSYLTPGDSSSGWTAGAAAYYVGYLQPRTFLLKYNENGTITDAVDCALDPLSETKCTLKSFTVEKGIYQTSNFRVQPTESIVRFPNITNLCPFGEVFNATRFASVYAWNRKRISNCVADYSVLYNSASFSTFKCYGVSPTKLNDLCFTNVYADSFVIRGDEVRQIAPGQTGTIADYNYKLPDDFTGCVIAWNSNNLDSKVGGNYNYLYRLFRKSNLKPFERDISTEIYQAGSTPCNGVKGFNCYFPLQSYGFQPTYGVGYQPYRVVVLSFELLHAPATVCGPKKSTNLVKNKCVNFNFNGLTGTGVLTESNKKFLPFQQFGRDIADTTDAVRDPQTLEILDITPCSFGGVSVITPGTNTSNQVAVLYQGVNCTEVPVAIHADQLTPTWRVYSTGSNVFQTRAGCLIGAEYVNNSYECDIPIGAGICASYQTQTNSPRRARSVASQSIIAYTMSLGAENSVAYSNNSIAIPTNFTISVTTEILPVSMTKTSVDCTMYICGDSTECSNLLLQYGSFCTQLNRALTGIAVEQDKNTQEVFAQVKQIYKTPPIKDFGGFNFSQILPDPSKPSKRSFIEDLLFNKVTLADAGFIKQYGDCLGDIAARDLICAQKFNGLTVLPPLLTDEMIAQYTSALLAGTITSGWTFGAGAALQIPFAMQMAYRFNGIGVTQNVLYENQKLIANQFNSAIGKIQDSLSSTASALGKLQDVVNQNAQALNTLVKQLSSNFGAISSVLNDILSRLDPPEAEVQIDRLITGRLQSLQTYVTQQLIRAAEIRASANLAAIKMSECVLGQSKRVDFCGKGYHLMSFPQSAPHGVVFLHVTYVPAQEKNFTTAPAICHDGKAHFPREGVFVSNGTHWFVTQRNFYEPQIITTDNTFVSGNCDVVIGIVNNTVYDPLQPELDSFKEELDKYFKNHTSPDVDLGDISGINASVVNIQKEIDRLNEVAKNLNESLIDLQELGKYEQ

SEQ ID NO: 43 - protein, 1195 aa, synthetic construct
  source 1..1195: note; note (original language) = SARS-CoV-2 Brazilian variant P.1 spike protein extracellular domain without signal peptide, S1/S2 furin cleavage site 1 and proline mutant (685R→685A, 986K/987V→986P/987P); organism (original language) = Synthetic construct
QCVNFTNRTQLPSAYTNSFTRGVYYPDKVFRSSVLHSTQDLFLPFFSNVTWFHAIHVSGTNGTKRFDNPVLPFNDGVYFASTEKSNIIRGWIFGTTLDSKTQSLLIVNNATNVVIKVCEFQFCNYPFLGVYYHKNNKSWMESEFRVYSSANNCTFEYVSQPFLMDLEGKQGNFKNLSEFVFKNIDGYFKIYSKHTPINLVRDLPQGFSALEPLVDLPIGINITRFQTLLALHRSYLTPGDSSSGWTAGAAAYYVGYLQPRTFLLKYNENGTITDAVDCALDPLSETKCTLKSFTVEKGIYQTSNFRVQPTESIVRFPNITNLCPFGEVFNATRFASVYAWNRKRISNCVADYSVLYNSASFSTFKCYGVSPTKLNDLCFTNVYADSFVIRGDEVRQIAPGQTGTIADYNYKLPDDFTGCVIAWNSNNLDSKVGGNYNYLYRLFRKSNLKPFERDISTEIYQAGSTPCNGVKGFNCYFPLQSYGFQPTYGVGYQPYRVVVLSFELLHAPATVCGPKKSTNLVKNKCVNFNFNGLTGTGVLTESNKKFLPFQQFGRDIADTTDAVRDPQTLEILDITPCSFGGVSVITPGTNTSNQVAVLYQGVNCTEVPVAIHADQLTPTWRVYSTGSNVFQTRAGCLIGAEYVNNSYECDIPIGAGICASYQTQTNSPRRAASVASQSIIAYTMSLGAENSVAYSNNSIAIPTNFTISVTTEILPVSMTKTSVDCTMYICGDSTECSNLLLQYGSFCTQLNRALTGIAVEQDKNTQEVFAQVKQIYKTPPIKDFGGFNFSQILPDPSKPSKRSFIEDLLFNKVTLADAGFIKQYGDCLGDIAARDLICAQKFNGLTVLPPLLTDEMIAQYTSALLAGTITSGWTFGAGAALQIPFAMQMAYRFNGIGVTQNVLYENQKLIANQFNSAIGKIQDSLSSTASALGKLQDVVNQNAQALNTLVKQLSSNFGAISSVLNDILSRLDPPEAEVQIDRLITGRLQSLQTYVTQQLIRAAEIRASANLAAIKMSECVLGQSKRVDFCGKGYHLMSFPQSAPHGVVFLHVTYVPAQEKNFTTAPAICHDGKAHFPREGVFVSNGTHWFVTQRNFYEPQIITTDNTFVSGNCDVVIGIVNNTVYDPLQPELDSFKEELDKYFKNHTSPDVDLGDISGINASVVNIQKEIDRLNEVAKNLNESLIDLQELGKYEQ

SEQ ID NO: 44 - protein, 1193 aa, synthetic construct
  source 1..1193: note; note (original language) = SARS-CoV-2 British variant B.1.1.7 spike protein extracellular domain without signal peptide; organism (original language) = Synthetic construct
QCVNLTTRTQLPPAYTNSFTRGVYYPDKVFRSSVLHSTQDLFLPFFSNVTWFHAISGTNGTKRFDNPVLPFNDGVYFASTEKSNIIRGWIFGTTLDSKTQSLLIVNNATNVVIKVCEFQFCNDPFLGVYYHKNNKSWMESEFRVYSSANNCTFEYVSQPFLMDLEGKQGNFKNLREFVFKNIDGYFKIYSKHTPINLVRDLPQGFSALEPLVDLPIGINITRFQTLLALHRSYLTPGDSSSGWTAGAAAYYVGYLQPRTFLLKYNENGTITDAVDCALDPLSETKCTLKSFTVEKGIYQTSNFRVQPTESIVRFPNITNLCPFGEVFNATRFASVYAWNRKRISNCVADYSVLYNSASFSTFKCYGVSPTKLNDLCFTNVYADSFVIRGDEVRQIAPGQTGKIADYNYKLPDDFTGCVIAWNSNNLDSKVGGNYNYLYRLFRKSNLKPFERDISTEIYQAGSTPCNGVEGFNCYFPLQSYGFQPTYGVGYQPYRVVVLSFELLHAPATVCGPKKSTNLVKNKCVNFNFNGLTGTGVLTESNKKFLPFQQFGRDIADTTDAVRDPQTLEILDITPCSFGGVSVITPGTNTSNQVAVLYQGVNCTEVPVAIHADQLTPTWRVYSTGSNVFQTRAGCLIGAEHVNNSYECDIPIGAGICASYQTQTNSHRRARSVASQSIIAYTMSLGAENSVAYSNNSIAIPTNFTISVTTEILPVSMTKTSVDCTMYICGDSTECSNLLLQYGSFCTQLNRALTGIAVEQDKNTQEVFAQVKQIYKTPPIKDFGGFNFSQILPDPSKPSKRSFIEDLLFNKVTLADAGFIKQYGDCLGDIAARDLICAQKFNGLTVLPPLLTDEMIAQYTSALLAGTITSGWTFGAGAALQIPFAMQMAYRFNGIGVTQNVLYENQKLIANQFNSAIGKIQDSLSSTASALGKLQDVVNQNAQALNTLVKQLSSNFGAISSVLNDILSRLDKVEAEVQIDRLITGRLQSLQTYVTQQLIRAAEIRASANLAATKMSECVLGQSKRVDFCGKGYHLMSFPQSAPHGVVFLHVTYVPAQEKNFTTAPAICHDGKAHFPREGVFVSNGTHWFVTQRNFYEPQIITTDNTFVSGNCDVVIGIVNNTVYDPLQPELDSFKEELDKYFKNHTSPDVDLGDISGINASVVNIQKEIDRLNEVAKNLNESLIDLQELGKYEQ

SEQ ID NO: 45 - protein, 1193 aa, synthetic construct
  source 1..1193: note; note (original language) = SARS-CoV-2 British variant B.1.1.7 spike protein extracellular domain without signal peptide, S1/S2 furin cleavage site 1 mutant (685R→685A); organism (original language) = Synthetic construct
QCVNLTTRTQLPPAYTNSFTRGVYYPDKVFRSSVLHSTQDLFLPFFSNVTWFHAISGTNGTKRFDNPVLPFNDGVYFASTEKSNIIRGWIFGTTLDSKTQSLLIVNNATNVVIKVCEFQFCNDPFLGVYYHKNNKSWMESEFRVYSSANNCTFEYVSQPFLMDLEGKQGNFKNLREFVFKNIDGYFKIYSKHTPINLVRDLPQGFSALEPLVDLPIGINITRFQTLLALHRSYLTPGDSSSGWTAGAAAYYVGYLQPRTFLLKYNENGTITDAVDCALDPLSETKCTLKSFTVEKGIYQTSNFRVQPTESIVRFPNITNLCPFGEVFNATRFASVYAWNRKRISNCVADYSVLYNSASFSTFKCYGVSPTKLNDLCFTNVYADSFVIRGDEVRQIAPGQTGKIADYNYKLPDDFTGCVIAWNSNNLDSKVGGNYNYLYRLFRKSNLKPFERDISTEIYQAGSTPCNGVEGFNCYFPLQSYGFQPTYGVGYQPYRVVVLSFELLHAPATVCGPKKSTNLVKNKCVNFNFNGLTGTGVLTESNKKFLPFQQFGRDIADTTDAVRDPQTLEILDITPCSFGGVSVITPGTNTSNQVAVLYQGVNCTEVPVAIHADQLTPTWRVYSTGSNVFQTRAGCLIGAEHVNNSYECDIPIGAGICASYQTQTNSHRRAASVASQSIIAYTMSLGAENSVAYSNNSIAIPTNFTISVTTEILPVSMTKTSVDCTMYICGDSTECSNLLLQYGSFCTQLNRALTGIAVEQDKNTQEVFAQVKQIYKTPPIKDFGGFNFSQILPDPSKPSKRSFIEDLLFNKVTLADAGFIKQYGDCLGDIAARDLICAQKFNGLTVLPPLLTDEMIAQYTSALLAGTITSGWTFGAGAALQIPFAMQMAYRFNGIGVTQNVLYENQKLIANQFNSAIGKIQDSLSSTASALGKLQDVVNQNAQALNTLVKQLSSNFGAISSVLNDILSRLDKVEAEVQIDRLITGRLQSLQTYVTQQLIRAAEIRASANLAATKMSECVLGQSKRVDFCGKGYHLMSFPQSAPHGVVFLHVTYVPAQEKNFTTAPAICHDGKAHFPREGVFVSNGTHWFVTQRNFYEPQIITTDNTFVSGNCDVVIGIVNNTVYDPLQPELDSFKEELDKYFKNHTSPDVDLGDISGINASVVNIQKEIDRLNEVAKNLNESLIDLQELGKYEQ

SEQ ID NO: 46 - protein, 1193 aa, synthetic construct
  source 1..1193: note; note (original language) = SARS-CoV-2 British variant B.1.1.7 spike protein extracellular domain without signal peptide, proline mutant (986K/987V→986P/987P); organism (original language) = Synthetic construct
QCVNLTTRTQLPPAYTNSFTRGVYYPDKVFRSSVLHSTQDLFLPFFSNVTWFHAISGTNGTKRFDNPVLPFNDGVYFASTEKSNIIRGWIFGTTLDSKTQSLLIVNNATNVVIKVCEFQFCNDPFLGVYYHKNNKSWMESEFRVYSSANNCTFEYVSQPFLMDLEGKQGNFKNLREFVFKNIDGYFKIYSKHTPINLVRDLPQGFSALEPLVDLPIGINITRFQTLLALHRSYLTPGDSSSGWTAGAAAYYVGYLQPRTFLLKYNENGTITDAVDCALDPLSETKCTLKSFTVEKGIYQTSNFRVQPTESIVRFPNITNLCPFGEVFNATRFASVYAWNRKRISNCVADYSVLYNSASFSTFKCYGVSPTKLNDLCFTNVYADSFVIRGDEVRQIAPGQTGKIADYNYKLPDDFTGCVIAWNSNNLDSKVGGNYNYLYRLFRKSNLKPFERDISTEIYQAGSTPCNGVEGFNCYFPLQSYGFQPTYGVGYQPYRVVVLSFELLHAPATVCGPKKSTNLVKNKCVNFNFNGLTGTGVLTESNKKFLPFQQFGRDIADTTDAVRDPQTLEILDITPCSFGGVSVITPGTNTSNQVAVLYQGVNCTEVPVAIHADQLTPTWRVYSTGSNVFQTRAGCLIGAEHVNNSYECDIPIGAGICASYQTQTNSHRRARSVASQSIIAYTMSLGAENSVAYSNNSIAIPTNFTISVTTEILPVSMTKTSVDCTMYICGDSTECSNLLLQYGSFCTQLNRALTGIAVEQDKNTQEVFAQVKQIYKTPPIKDFGGFNFSQILPDPSKPSKRSFIEDLLFNKVTLADAGFIKQYGDCLGDIAARDLICAQKFNGLTVLPPLLTDEMIAQYTSALLAGTITSGWTFGAGAALQIPFAMQMAYRFNGIGVTQNVLYENQKLIANQFNSAIGKIQDSLSSTASALGKLQDVVNQNAQALNTLVKQLSSNFGAISSVLNDILSRLDPPEAEVQIDRLITGRLQSLQTYVTQQLIRAAEIRASANLAATKMSECVLGQSKRVDFCGKGYHLMSFPQSAPHGVVFLHVTYVPAQEKNFTTAPAICHDGKAHFPREGVFVSNGTHWFVTQRNFYEPQIITTDNTFVSGNCDVVIGIVNNTVYDPLQPELDSFKEELDKYFKNHTSPDVDLGDISGINASVVNIQKEIDRLNEVAKNLNESLIDLQELGKYEQ

SEQ ID NO: 47 - protein, 1193 aa, synthetic construct
  source 1..1193: note; note (original language) = SARS-CoV-2 British variant B.1.1.7 spike protein extracellular domain without signal peptide, S1/S2 furin cleavage site and proline mutant (685R→685A, 986K/987V→986P/987P); organism (original language) = Synthetic construct
QCVNLTTRTQLPPAYTNSFTRGVYYPDKVFRSSVLHSTQDLFLPFFSNVTWFHAISGTNGTKRFDNPVLPFNDGVYFASTEKSNIIRGWIFGTTLDSKTQSLLIVNNATNVVIKVCEFQFCNDPFLGVYYHKNNKSWMESEFRVYSSANNCTFEYVSQPFLMDLEGKQGNFKNLREFVFKNIDGYFKIYSKHTPINLVRDLPQGFSALEPLVDLPIGINITRFQTLLALHRSYLTPGDSSSGWTAGAAAYYVGYLQPRTFLLKYNENGTITDAVDCALDPLSETKCTLKSFTVEKGIYQTSNFRVQPTESIVRFPNITNLCPFGEVFNATRFASVYAWNRKRISNCVADYSVLYNSASFSTFKCYGVSPTKLNDLCFTNVYADSFVIRGDEVRQIAPGQTGKIADYNYKLPDDFTGCVIAWNSNNLDSKVGGNYNYLYRLFRKSNLKPFERDISTEIYQAGSTPCNGVEGFNCYFPLQSYGFQPTYGVGYQPYRVVVLSFELLHAPATVCGPKKSTNLVKNKCVNFNFNGLTGTGVLTESNKKFLPFQQFGRDIADTTDAVRDPQTLEILDITPCSFGGVSVITPGTNTSNQVAVLYQGVNCTEVPVAIHADQLTPTWRVYSTGSNVFQTRAGCLIGAEHVNNSYECDIPIGAGICASYQTQTNSHRRAASVASQSIIAYTMSLGAENSVAYSNNSIAIPTNFTISVTTEILPVSMTKTSVDCTMYICGDSTECSNLLLQYGSFCTQLNRALTGIAVEQDKNTQEVFAQVKQIYKTPPIKDFGGFNFSQILPDPSKPSKRSFIEDLLFNKVTLADAGFIKQYGDCLGDIAARDLICAQKFNGLTVLPPLLTDEMIAQYTSALLAGTITSGWTFGAGAALQIPFAMQMAYRFNGIGVTQNVLYENQKLIANQFNSAIGKIQDSLSSTASALGKLQDVVNQNAQALNTLVKQLSSNFGAISSVLNDILSRLDPPEAEVQIDRLITGRLQSLQTYVTQQLIRAAEIRASANLAATKMSECVLGQSKRVDFCGKGYHLMSFPQSAPHGVVFLHVTYVPAQEKNFTTAPAICHDGKAHFPREGVFVSNGTHWFVTQRNFYEPQIITTDNTFVSGNCDVVIGIVNNTVYDPLQPELDSFKEELDKYFKNHTSPDVDLGDISGINASVVNIQKEIDRLNEVAKNLNESLIDLQELGKYEQ

SEQ ID NO: 48 - protein, 1195 aa, synthetic construct
  source 1..1195: note; note (original language) = SARS-CoV-2 variant D614G spike protein extracellular domain without signal peptide; organism (original language) = Synthetic construct
QCVNLTTRTQLPPAYTNSFTRGVYYPDKVFRSSVLHSTQDLFLPFFSNVTWFHAIHVSGTNGTKRFDNPVLPFNDGVYFASTEKSNIIRGWIFGTTLDSKTQSLLIVNNATNVVIKVCEFQFCNDPFLGVYYHKNNKSWMESEFRVYSSANNCTFEYVSQPFLMDLEGKQGNFKNLREFVFKNIDGYFKIYSKHTPINLVRDLPQGFSALEPLVDLPIGINITRFQTLLALHRSYLTPGDSSSGWTAGAAAYYVGYLQPRTFLLKYNENGTITDAVDCALDPLSETKCTLKSFTVEKGIYQTSNFRVQPTESIVRFPNITNLCPFGEVFNATRFASVYAWNRKRISNCVADYSVLYNSASFSTFKCYGVSPTKLNDLCFTNVYADSFVIRGDEVRQIAPGQTGKIADYNYKLPDDFTGCVIAWNSNNLDSKVGGNYNYLYRLFRKSNLKPFERDISTEIYQAGSTPCNGVEGFNCYFPLQSYGFQPTNGVGYQPYRVVVLSFELLHAPATVCGPKKSTNLVKNKCVNFNFNGLTGTGVLTESNKKFLPFQQFGRDIADTTDAVRDPQTLEILDITPCSFGGVSVITPGTNTSNQVAVLYQGVNCTEVPVAIHADQLTPTWRVYSTGSNVFQTRAGCLIGAEHVNNSYECDIPIGAGICASYQTQTNSPRRARSVASQSIIAYTMSLGAENSVAYSNNSIAIPTNFTISVTTEILPVSMTKTSVDCTMYICGDSTECSNLLLQYGSFCTQLNRALTGIAVEQDKNTQEVFAQVKQIYKTPPIKDFGGFNFSQILPDPSKPSKRSFIEDLLFNKVTLADAGFIKQYGDCLGDIAARDLICAQKFNGLTVLPPLLTDEMIAQYTSALLAGTITSGWTFGAGAALQIPFAMQMAYRFNGIGVTQNVLYENQKLIANQFNSAIGKIQDSLSSTASALGKLQDVVNQNAQALNTLVKQLSSNFGAISSVLNDILSRLDKVEAEVQIDRLITGRLQSLQTYVTQQLIRAAEIRASANLAATKMSECVLGQSKRVDFCGKGYHLMSFPQSAPHGVVFLHVTYVPAQEKNFTTAPAICHDGKAHFPREGVFVSNGTHWFVTQRNFYEPQIITTDNTFVSGNCDVVIGIVNNTVYDPLQPELDSFKEELDKYFKNHTSPDVDLGDISGINASVVNIQKEIDRLNEVAKNLNESLIDLQELGKYEQ

SEQ ID NO: 49 - protein, 1195 aa, synthetic construct
  source 1..1195: note; note (original language) = SARS-CoV-2 variant D614G spike protein extracellular domain without signal peptide, S1/S2 furin cleavage site 1 mutant (685R→685A); organism (original language) = Synthetic construct
QCVNLTTRTQLPPAYTNSFTRGVYYPDKVFRSSVLHSTQDLFLPFFSNVTWFHAIHVSGTNGTKRFDNPVLPFNDGVYFASTEKSNIIRGWIFGTTLDSKTQSLLIVNNATNVVIKVCEFQFCNDPFLGVYYHKNNKSWMESEFRVYSSANNCTFEYVSQPFLMDLEGKQGNFKNLREFVFKNIDGYFKIYSKHTPINLVRDLPQGFSALEPLVDLPIGINITRFQTLLALHRSYLTPGDSSSGWTAGAAAYYVGYLQPRTFLLKYNENGTITDAVDCALDPLSETKCTLKSFTVEKGIYQTSNFRVQPTESIVRFPNITNLCPFGEVFNATRFASVYAWNRKRISNCVADYSVLYNSASFSTFKCYGVSPTKLNDLCFTNVYADSFVIRGDEVRQIAPGQTGKIADYNYKLPDDFTGCVIAWNSNNLDSKVGGNYNYLYRLFRKSNLKPFERDISTEIYQAGSTPCNGVEGFNCYFPLQSYGFQPTNGVGYQPYRVVVLSFELLHAPATVCGPKKSTNLVKNKCVNFNFNGLTGTGVLTESNKKFLPFQQFGRDIADTTDAVRDPQTLEILDITPCSFGGVSVITPGTNTSNQVAVLYQGVNCTEVPVAIHADQLTPTWRVYSTGSNVFQTRAGCLIGAEHVNNSYECDIPIGAGICASYQTQTNSPRRAASVASQSIIAYTMSLGAENSVAYSNNSIAIPTNFTISVTTEILPVSMTKTSVDCTMYICGDSTECSNLLLQYGSFCTQLNRALTGIAVEQDKNTQEVFAQVKQIYKTPPIKDFGGFNFSQILPDPSKPSKRSFIEDLLFNKVTLADAGFIKQYGDCLGDIAARDLICAQKFNGLTVLPPLLTDEMIAQYTSALLAGTITSGWTFGAGAALQIPFAMQMAYRFNGIGVTQNVLYENQKLIANQFNSAIGKIQDSLSSTASALGKLQDVVNQNAQALNTLVKQLSSNFGAISSVLNDILSRLDKVEAEVQIDRLITGRLQSLQTYVTQQLIRAAEIRASANLAATKMSECVLGQSKRVDFCGKGYHLMSFPQSAPHGVVFLHVTYVPAQEKNFTTAPAICHDGKAHFPREGVFVSNGTHWFVTQRNFYEPQIITTDNTFVSGNCDVVIGIVNNTVYDPLQPELDSFKEELDKYFKNHTSPDVDLGDISGINASVVNIQKEIDRLNEVAKNLNESLIDLQELGKYEQ

SEQ ID NO: 50 - protein, 1195 aa, synthetic construct
  source 1..1195: note; note (original language) = SARS-CoV-2 variant D614G spike protein extracellular domain without signal peptide, proline mutant (986K/987V→986P/987P); organism (original language) = Synthetic construct
QCVNLTTRTQLPPAYTNSFTRGVYYPDKVFRSSVLHSTQDLFLPFFSNVTWFHAIHVSGTNGTKRFDNPVLPFNDGVYFASTEKSNIIRGWIFGTTLDSKTQSLLIVNNATNVVIKVCEFQFCNDPFLGVYYHKNNKSWMESEFRVYSSANNCTFEYVSQPFLMDLEGKQGNFKNLREFVFKNIDGYFKIYSKHTPINLVRDLPQGFSALEPLVDLPIGINITRFQTLLALHRSYLTPGDSSSGWTAGAAAYYVGYLQPRTFLLKYNENGTITDAVDCALDPLSETKCTLKSFTVEKGIYQTSNFRVQPTESIVRFPNITNLCPFGEVFNATRFASVYAWNRKRISNCVADYSVLYNSASFSTFKCYGVSPTKLNDLCFTNVYADSFVIRGDEVRQIAPGQTGKIADYNYKLPDDFTGCVIAWNSNNLDSKVGGNYNYLYRLFRKSNLKPFERDISTEIYQAGSTPCNGVEGFNCYFPLQSYGFQPTNGVGYQPYRVVVLSFELLHAPATVCGPKKSTNLVKNKCVNFNFNGLTGTGVLTESNKKFLPFQQFGRDIADTTDAVRDPQTLEILDITPCSFGGVSVITPGTNTSNQVAVLYQGVNCTEVPVAIHADQLTPTWRVYSTGSNVFQTRAGCLIGAEHVNNSYECDIPIGAGICASYQTQTNSPRRARSVASQSIIAYTMSLGAENSVAYSNNSIAIPTNFTISVTTEILPVSMTKTSVDCTMYICGDSTECSNLLLQYGSFCTQLNRALTGIAVEQDKNTQEVFAQVKQIYKTPPIKDFGGFNFSQILPDPSKPSKRSFIEDLLFNKVTLADAGFIKQYGDCLGDIAARDLICAQKFNGLTVLPPLLTDEMIAQYTSALLAGTITSGWTFGAGAALQIPFAMQMAYRFNGIGVTQNVLYENQKLIANQFNSAIGKIQDSLSSTASALGKLQDVVNQNAQALNTLVKQLSSNFGAISSVLNDILSRLDPPEAEVQIDRLITGRLQSLQTYVTQQLIRAAEIRASANLAATKMSECVLGQSKRVDFCGKGYHLMSFPQSAPHGVVFLHVTYVPAQEKNFTTAPAICHDGKAHFPREGVFVSNGTHWFVTQRNFYEPQIITTDNTFVSGNCDVVIGIVNNTVYDPLQPELDSFKEELDKYFKNHTSPDVDLGDISGINASVVNIQKEIDRLNEVAKNLNESLIDLQELGKYEQ

SEQ ID NO: 51 - protein, 1195 aa, synthetic construct
  source 1..1195: note; note (original language) = SARS-CoV-2 variant D614G spike protein extracellular domain without signal peptide, S1/S2 furin cleavage site 1 and proline mutant (685R→685A, 986K/987V→986P/987P); organism (original language) = Synthetic construct
QCVNLTTRTQLPPAYTNSFTRGVYYPDKVFRSSVLHSTQDLFLPFFSNVTWFHAIHVSGTNGTKRFDNPVLPFNDGVYFASTEKSNIIRGWIFGTTLDSKTQSLLIVNNATNVVIKVCEFQFCNDPFLGVYYHKNNKSWMESEFRVYSSANNCTFEYVSQPFLMDLEGKQGNFKNLREFVFKNIDGYFKIYSKHTPINLVRDLPQGFSALEPLVDLPIGINITRFQTLLALHRSYLTPGDSSSGWTAGAAAYYVGYLQPRTFLLKYNENGTITDAVDCALDPLSETKCTLKSFTVEKGIYQTSNFRVQPTESIVRFPNITNLCPFGEVFNATRFASVYAWNRKRISNCVADYSVLYNSASFSTFKCYGVSPTKLNDLCFTNVYADSFVIRGDEVRQIAPGQTGKIADYNYKLPDDFTGCVIAWNSNNLDSKVGGNYNYLYRLFRKSNLKPFERDISTEIYQAGSTPCNGVEGFNCYFPLQSYGFQPTNGVGYQPYRVVVLSFELLHAPATVCGPKKSTNLVKNKCVNFNFNGLTGTGVLTESNKKFLPFQQFGRDIADTTDAVRDPQTLEILDITPCSFGGVSVITPGTNTSNQVAVLYQGVNCTEVPVAIHADQLTPTWRVYSTGSNVFQTRAGCLIGAEHVNNSYECDIPIGAGICASYQTQTNSPRRAASVASQSIIAYTMSLGAENSVAYSNNSIAIPTNFTISVTTEILPVSMTKTSVDCTMYICGDSTECSNLLLQYGSFCTQLNRALTGIAVEQDKNTQEVFAQVKQIYKTPPIKDFGGFNFSQILPDPSKPSKRSFIEDLLFNKVTLADAGFIKQYGDCLGDIAARDLICAQKFNGLTVLPPLLTDEMIAQYTSALLAGTITSGWTFGAGAALQIPFAMQMAYRFNGIGVTQNVLYENQKLIANQFNSAIGKIQDSLSSTASALGKLQDVVNQNAQALNTLVKQLSSNFGAISSVLNDILSRLDPPEAEVQIDRLITGRLQSLQTYVTQQLIRAAEIRASANLAATKMSECVLGQSKRVDFCGKGYHLMSFPQSAPHGVVFLHVTYVPAQEKNFTTAPAICHDGKAHFPREGVFVSNGTHWFVTQRNFYEPQIITTDNTFVSGNCDVVIGIVNNTVYDPLQPELDSFKEELDKYFKNHTSPDVDLGDISGINASVVNIQKEIDRLNEVAKNLNESLIDLQELGKYEQ

SEQ ID NO: 52 - protein, 1177 aa, synthetic construct
  source 1..1177: note; note (original language) = SARS-CoV-1 spike protein extracellular domain without signal peptide; organism (original language) = Synthetic construct
SDLDRCTTFDDVQAPNYTQHTSSMRGVYYPDEIFRSDTLYLTQDLFLPFYSNVTGFHTINHTFDNPVIPFKDGIYFAATEKSNVVRGWVFGSTMNNKSQSVIIINNSTNVVIRACNFELCDNPFFAVSKPMGTQTHTMIFDNAFNCTFEYISDAFSLDVSEKSGNFKHLREFVFKNKDGFLYVYKGYQPIDVVRDLPSGFNTLKPIFKLPLGINITNFRAILTAFLPAQDTWGTSAAAYFVGYLKPTTFMLKYDENGTITDAVDCSQNPLAELKCSVKSFEIDKGIYQTSNFRVVPSRDVVRFPNITNLCPFGEVFNATKFPSVYAWERKRISNCVADYSVLYNSTFFSTFKCYGVSATKLNDLCFSNVYADSFVVKGDDVRQIAPGQTGVIADYNYKLPDDFMGCVLAWNTRNIDATSTGNYNYKYRYLRHGKLRPFERDISNVPFSPDGKPCTPPALNCYWPLNDYGFYTTTGIGYQPYRVVVLSFELLNAPATVCGPKLSTDLIKNQCVNFNFNGLTGTGVLTPSSKRFQPFQQFGRDVSDFTDSVRDPKTSEILDISPCSFGGVSVITPGTNASSEVAVLYQDVNCTDVSTAIHADQLTPAWRIYSTGNNVFQTQAGCLIGAEHVDTSYECDIPIGAGICASYHTVSLLRSTSQKSIVAYTMSLGADSSIAYSNNTIAIPTNFSISITTEVMPVSMAKTSVDCNMYICGDSTECANLLLQYGSFCTQLNRALSGIAAEQDRNTREVFAQVKQMYKTPTLKDFGGFNFSQILPDPLKPTKRSFIEDLLFNKVTLADAGFMKQYGECLGDINARDLICAQKFNGLTVLPPLLTDDMIAAYTAALVSGTATAGWTFGAGAALQIPFAMQMAYRFNGIGVTQNVLYENQKQIANQFNKAISQIQESLTTTSTALGKLQDVVNQNAQALNTLVKQLSSNFGAISSVLNDILSRLDKVEAEVQIDRLITGRLQSLQTYVTQQLIRAAEIRASANLAATKMSECVLGQSKRVDFCGKGYHLMSFPQAAPHGVVFLHVTYVPSQERNFTTAPAICHEGKAYFPREGVFVFNGTSWFITQRNFFSPQIITTDNTFVSGNCDVVIGIINNTVYDPLQPELDSFKEELDKYFKNHTSPDVDLGDISGINASVVNIQEEIDRLNEVAKNLNESLIDLQELGKYEQ

SEQ ID NO: 53 - protein, 13 aa, synthetic construct
  source 1..13: note; note (original language) = SARS-CoV-1 spike protein signal peptide; organism (original language) = Synthetic construct
MFIFLLFLTLTSG

SEQ ID NO: 54 - protein, 13 aa, synthetic construct
  source 1..13: note; note (original language) = Hu-1 SARS-CoV-2 spike protein signal peptide; organism (original language) = Synthetic construct
MFVFLVLLPLVSS

SEQ ID NO: 55 - protein, 1273 aa, synthetic construct
  source 1..1273: note; note (original language) = Hu-1 SARS-CoV-2 full-length spike protein, 1273 aa; organism (original language) = Synthetic construct
MFVFLVLLPLVSSQCVNLTTRTQLPPAYTNSFTRGVYYPDKVFRSSVLHSTQDLFLPFFSNVTWFHAIHVSGTNGTKRFDNPVLPFNDGVYFASTEKSNIIRGWIFGTTLDSKTQSLLIVNNATNVVIKVCEFQFCNDPFLGVYYHKNNKSWMESEFRVYSSANNCTFEYVSQPFLMDLEGKQGNFKNLREFVFKNIDGYFKIYSKHTPINLVRDLPQGFSALEPLVDLPIGINITRFQTLLALHRSYLTPGDSSSGWTAGAAAYYVGYLQPRTFLLKYNENGTITDAVDCALDPLSETKCTLKSFTVEKGIYQTSNFRVQPTESIVRFPNITNLCPFGEVFNATRFASVYAWNRKRISNCVADYSVLYNSASFSTFKCYGVSPTKLNDLCFTNVYADSFVIRGDEVRQIAPGQTGKIADYNYKLPDDFTGCVIAWNSNNLDSKVGGNYNYLYRLFRKSNLKPFERDISTEIYQAGSTPCNGVEGFNCYFPLQSYGFQPTNGVGYQPYRVVVLSFELLHAPATVCGPKKSTNLVKNKCVNFNFNGLTGTGVLTESNKKFLPFQQFGRDIADTTDAVRDPQTLEILDITPCSFGGVSVITPGTNTSNQVAVLYQDVNCTEVPVAIHADQLTPTWRVYSTGSNVFQTRAGCLIGAEHVNNSYECDIPIGAGICASYQTQTNSPRRARSVASQSIIAYTMSLGAENSVAYSNNSIAIPTNFTISVTTEILPVSMTKTSVDCTMYICGDSTECSNLLLQYGSFCTQLNRALTGIAVEQDKNTQEVFAQVKQIYKTPPIKDFGGFNFSQILPDPSKPSKRSFIEDLLFNKVTLADAGFIKQYGDCLGDIAARDLICAQKFNGLTVLPPLLTDEMIAQYTSALLAGTITSGWTFGAGAALQIPFAMQMAYRFNGIGVTQNVLYENQKLIANQFNSAIGKIQDSLSSTASALGKLQDVVNQNAQALNTLVKQLSSNFGAISSVLNDILSRLDKVEAEVQIDRLITGRLQSLQTYVTQQLIRAAEIRASANLAATKMSECVLGQSKRVDFCGKGYHLMSFPQSAPHGVVFLHVTYVPAQEKNFTTAPAICHDGKAHFPREGVFVSNGTHWFVTQRNFYEPQIITTDNTFVSGNCDVVIGIVNNTVYDPLQPELDSFKEELDKYFKNHTSPDVDLGDISGINASVVNIQKEIDRLNEVAKNLNESLIDLQELGKYEQYIKWPWYIWLGFIAGLIAIVMVTIMLCCMTSCCSCLKGCCSCGSCCKFDEDDSEPVLKGVKLHYT

SEQ ID NO: 56 - protein, 1208 aa, synthetic construct
  source 1..1208: note; note (original language) = Hu-1 SARS-CoV-2 spike protein extracellular domain with signal peptide; organism (original language) = Synthetic construct
MFVFLVLLPLVSSQCVNLTTRTQLPPAYTNSFTRGVYYPDKVFRSSVLHSTQDLFLPFFSNVTWFHAIHVSGTNGTKRFDNPVLPFNDGVYFASTEKSNIIRGWIFGTTLDSKTQSLLIVNNATNVVIKVCEFQFCNDPFLGVYYHKNNKSWMESEFRVYSSANNCTFEYVSQPFLMDLEGKQGNFKNLREFVFKNIDGYFKIYSKHTPINLVRDLPQGFSALEPLVDLPIGINITRFQTLLALHRSYLTPGDSSSGWTAGAAAYYVGYLQPRTFLLKYNENGTITDAVDCALDPLSETKCTLKSFTVEKGIYQTSNFRVQPTESIVRFPNITNLCPFGEVFNATRFASVYAWNRKRISNCVADYSVLYNSASFSTFKCYGVSPTKLNDLCFTNVYADSFVIRGDEVRQIAPGQTGKIADYNYKLPDDFTGCVIAWNSNNLDSKVGGNYNYLYRLFRKSNLKPFERDISTEIYQAGSTPCNGVEGFNCYFPLQSYGFQPTNGVGYQPYRVVVLSFELLHAPATVCGPKKSTNLVKNKCVNFNFNGLTGTGVLTESNKKFLPFQQFGRDIADTTDAVRDPQTLEILDITPCSFGGVSVITPGTNTSNQVAVLYQDVNCTEVPVAIHADQLTPTWRVYSTGSNVFQTRAGCLIGAEHVNNSYECDIPIGAGICASYQTQTNSPRRARSVASQSIIAYTMSLGAENSVAYSNNSIAIPTNFTISVTTEILPVSMTKTSVDCTMYICGDSTECSNLLLQYGSFCTQLNRALTGIAVEQDKNTQEVFAQVKQIYKTPPIKDFGGFNFSQILPDPSKPSKRSFIEDLLFNKVTLADAGFIKQYGDCLGDIAARDLICAQKFNGLTVLPPLLTDEMIAQYTSALLAGTITSGWTFGAGAALQIPFAMQMAYRFNGIGVTQNVLYENQKLIANQFNSAIGKIQDSLSSTASALGKLQDVVNQNAQALNTLVKQLSSNFGAISSVLNDILSRLDKVEAEVQIDRLITGRLQSLQTYVTQQLIRAAEIRASANLAATKMSECVLGQSKRVDFCGKGYHLMSFPQSAPHGVVFLHVTYVPAQEKNFTTAPAICHDGKAHFPREGVFVSNGTHWFVTQRNFYEPQIITTDNTFVSGNCDVVIGIVNNTVYDPLQPELDSFKEELDKYFKNHTSPDVDLGDISGINASVVNIQKEIDRLNEVAKNLNESLIDLQELGKYEQ

SEQ ID NO: 57 - protein, 290 aa, synthetic construct
  source 1..290: note; note (original language) = Hu-1 SARS-CoV-2 spike protein NTD without signal peptide, 290 aa; organism (original language) = Synthetic construct
VNLTTRTQLPPAYTNSFTRGVYYPDKVFRSSVLHSTQDLFLPFFSNVTWFHAIHVSGTNGTKRFDNPVLPFNDGVYFASTEKSNIIRGWIFGTTLDSKTQSLLIVNNATNVVIKVCEFQFCNDPFLGVYYHKNNKSWMESEFRVYSSANNCTFEYVSQPFLMDLEGKQGNFKNLREFVFKNIDGYFKIYSKHTPINLVRDLPQGFSALEPLVDLPIGINITRFQTLLALHRSYLTPGDSSSGWTAGAAAYYVGYLQPRTFLLKYNENGTITDAVDCALDPLSETKCTLKS

SEQ ID NO: 58 - protein, 192 aa, synthetic construct
  source 1..192: note; note (original language) = Hu-1 SARS-CoV-2 spike protein RBD, 192 aa; organism (original language) = Synthetic construct
PNITNLCPFGEVFNATRFASVYAWNRKRISNCVADYSVLYNSASFSTFKCYGVSPTKLNDLCFTNVYADSFVIRGDEVRQIAPGQTGKIADYNYKLPDDFTGCVIAWNSNNLDSKVGGNYNYLYRLFRKSNLKPFERDISTEIYQAGSTPCNGVEGFNCYFPLQSYGFQPTNGVGYQPYRVVVLSFELLHAP

SEQ ID NO: 59 - protein, 4 aa, synthetic construct
  source 1..4: note; note (original language) = Hu-1 SARS-CoV-2 spike protein S1/S2; organism (original language) = Synthetic construct
RRAR

SEQ ID NO: 60 - protein, 4 aa, synthetic construct
  source 1..4: note; note (original language) = Hu-1 SARS-CoV-2 spike protein S1/S2 mutant; organism (original language) = Synthetic construct
GSAG

SEQ ID NO: 61 - protein, 18 aa, synthetic construct
  source 1..18: note; note (original language) = Hu-1 SARS-CoV-2 spike protein fusion peptide (FP) sequence; organism (original language) = Synthetic construct
SFIEDLLFNKVTLADAGF

SEQ ID NO: 62 - protein, 78 aa, synthetic construct
  source 1..78: note; note (original language) = Hu-1 SARS-CoV-2 spike protein heptapeptide repeat 1 (HR1); organism (original language) = Synthetic construct
GIGVTQNVLYENQKLIANQFNSAIGKIQDSLSSTASALGKLQDVVNQNAQALNTLVKQLSSNFGAISSVLNDILSRLD

SEQ ID NO: 63 - protein, 50 aa, synthetic construct
  source 1..50: note; note (original language) = Hu-1 SARS-CoV-2 spike protein central helix (CH); organism (original language) = Synthetic construct
KVEAEVQIDRLITGRLQSLQTYVTQQLIRAAEIRASANLAATKMSECVLG

SEQ ID NO: 64 - protein, 66 aa, synthetic construct
  source 1..66: note; note (original language) = Hu-1 SARS-CoV-2 spike protein connector domain (CD); organism (original language) = Synthetic construct
TTAPAICHDGKAHFPREGVFVSNGTHWFVTQRNFYEPQIITTDNTFVSGNCDVVIGIVNNTVYDPL

SEQ ID NO: 65 - protein, 59 aa, synthetic construct
  source 1..59: note; note (original language) = Hu-1 SARS-CoV-2 spike protein heptapeptide repeat 2 (HR2); organism (original language) = Synthetic construct
EELDKYFKNHTSPDVDLGDISGINASVVNIQKEIDRLNEVAKNLNESLIDLQELGKYEQ

SEQ ID NO: 66 - protein, 23 aa, synthetic construct
  source 1..23: note; note (original language) = Hu-1 SARS-CoV-2 spike protein transmembrane (TM) domain; organism (original language) = Synthetic construct
WPWYIWLGFIAGLIAIVMVTIML

SEQ ID NO: 67 - protein, 244 aa, synthetic construct
  source 1..244: note; note (original language) = Trimeric peptide (type I), QT version; organism (original language) = Synthetic construct
ANVVRDRDLEVDTTLKSLSQQIENIRSPEGSRKNPARTCRDLKMCHSDWKSGEYWIDPNQGCNLDAIKVFCNMETGETCVYPTQPSVAQKNWYISKNPKDKRHVWFGESMTDGFQFEYGGQGSDPADVAIQLTFLRLMSTEASQNITYHCKNSVAYMDQQTGNLKKALLLQGSNEIEIRAEGNSRFTYSVTVDGCTSHTGAWGKTVIEYKTTKTSRLPIIDVAPLDVGAPDQEFGFDVGPVCFL

SEQ ID NO: 68 - protein, 309 aa, synthetic construct
  source 1..309: note; note (original language) = Trimerized peptide (type I) with glycine-X-Y repeat and D→N mutation at the BMP-1 site, QT version; organism (original language) = Synthetic construct
NGLPGPIGPPGPRGRTGDAGPVGPPGPPGPPGPPGPPSAGFDFSFLPQPPQEKAHDGGRYYRANDANVVRDRDLEVDTTLKSLSQQIENIRSPEGSRKNPARTCRDLKMCHSDWKSGEYWIDPNQGCNLDAIKVFCNMETGETCVYPTQPSVAQKNWYISKNPKDKRHVWFGESMTDGFQFEYGGQGSDPADVAIQLTFLRLMSTEASQNITYHCKNSVAYMDQQTGNLKKALLLQGSNEIEIRAEGNSRFTYSVTVDGCTSHTGAWGKTVIEYKTTKTSRLPIIDVAPLDVGAPDQEFGFDVGPVCFL

SEQ ID NO: 69 - protein, 309 aa, synthetic construct
  source 1..309: note; note (original language) = Trimerized peptide (type I) with glycine-X-Y repeat and A→N mutation at the BMP-1 site, QT version; organism (original language) = Synthetic construct
NGLPGPIGPPGPRGRTGDAGPVGPPGPPGPPGPPGPPSAGFDFSFLPQPPQEKAHDGGRYYRNDDANVVRDRDLEVDTTLKSLSQQIENIRSPEGSRKNPARTCRDLKMCHSDWKSGEYWIDPNQGCNLDAIKVFCNMETGETCVYPTQPSVAQKNWYISKNPKDKRHVWFGESMTDGFQFEYGGQGSDPADVAIQLTFLRLMSTEASQNITYHCKNSVAYMDQQTGNLKKALLLQGSNEIEIRAEGNSRFTYSVTVDGCTSHTGAWGKTVIEYKTTKTSRLPIIDVAPLDVGAPDQEFGFDVGPVCFL

SEQ ID NO: 70 - protein, 311 aa, synthetic construct
  source 1..311: note; note (original language) = Trimerized peptide (type I) with glycine-X-Y repeat and D→N mutation at the BMP-1 site, QT version; organism (original language) = Synthetic construct
RSNGLPGPIGPPGPRGRTGDAGPVGPPGPPGPPGPPGPPSAGFDFSFLPQPPQEKAHDGGRYYRANDANVVRDRDLEVDTTLKSLSQQIENIRSPEGSRKNPARTCRDLKMCHSDWKSGEYWIDPNQGCNLDAIKVFCNMETGETCVYPTQPSVAQKNWYISKNPKDKRHVWFGESMTDGFQFEYGGQGSDPADVAIQLTFLRLMSTEASQNITYHCKNSVAYMDQQTGNLKKALLLQGSNEIEIRAEGNSRFTYSVTVDGCTSHTGAWGKTVIEYKTTKTSRLPIIDVAPLDVGAPDQEFGFDVGPVCFL

SEQ ID NO: 71 - protein, 311 aa, synthetic construct
  source 1..311: note; note (original language) = Trimerized peptide (type I) with glycine-X-Y repeat and D→N mutation at the BMP-1 site, QT version; organism (original language) = Synthetic construct
GSNGLPGPIGPPGPRGRTGDAGPVGPPGPPGPPGPPGPPSAGFDFSFLPQPPQEKAHDGGRYYRANDANVVRDRDLEVDTTLKSLSQQIENIRSPEGSRKNPARTCRDLKMCHSDWKSGEYWIDPNQGCNLDAIKVFCNMETGETCVYPTQPSVAQKNWYISKNPKDKRHVWFGESMTDGFQFEYGGQGSDPADVAIQLTFLRLMSTEASQNITYHCKNSVAYMDQQTGNLKKALLLQGSNEIEIRAEGNSRFTYSVTVDGCTSHTGAWGKTVIEYKTTKTSRLPIIDVAPLDVGAPDQEFGFDVGPVCFL

SEQ ID NO: 72 - protein, 244 aa, synthetic construct
  source 1..244: note; note (original language) = Trimeric peptide (type I), KS version; organism (original language) = Synthetic construct
ANVVRDRDLEVDTTLKSLSQQIENIRSPEGSRKNPARTCRDLKMCHSDWKSGEYWIDPNQGCNLDAIKVFCNMETGETCVYPTQPSVAQKNWYISKNPKDKRHVWFGESMTDGFQFEYGGQGSDPADVAIQLTFLRLMSTEASQNITYHCKNSVAYMDQQTGNLKKALLLKGSNEIEIRAEGNSRFTYSVTVDGCTSHTGAWGKTVIEYKTTKSSRLPIIDVAPLDVGAPDQEFGFDVGPVCFL

SEQ ID NO: 73 - protein, 309 aa, synthetic construct
  source 1..309: note; note (original language) = Trimerized peptide (type I) with glycine-X-Y repeat and D→N mutation at the BMP-1 site, KS version; organism (original language) = Synthetic construct
NGLPGPIGPPGPRGRTGDAGPVGPPGPPGPPGPPGPPSAGFDFSFLPQPPQEKAHDGGRYYRANDANVVRDRDLEVDTTLKSLSQQIENIRSPEGSRKNPARTCRDLKMCHSDWKSGEYWIDPNQGCNLDAIKVFCNMETGETCVYPTQPSVAQKNWYISKNPKDKRHVWFGESMTDGFQFEYGGQGSDPADVAIQLTFLRLMSTEASQNITYHCKNSVAYMDQQTGNLKKALLLKGSNEIEIRAEGNSRFTYSVTVDGCTSHTGAWGKTVIEYKTTKSSRLPIIDVAPLDVGAPDQEFGFDVGPVCFL

SEQ ID NO: 74 - protein, 309 aa, synthetic construct
  source 1..309: note; note (original language) = Trimerized peptide (type I) with glycine-X-Y repeat and A→N mutation at the BMP-1 site, KS version; organism (original language) = Synthetic construct
NGLPGPIGPPGPRGRTGDAGPVGPPGPPGPPGPPGPPSAGFDFSFLPQPPQEKAHDGGRYYRNDDANVVRDRDLEVDTTLKSLSQQIENIRSPEGSRKNPARTCRDLKMCHSDWKSGEYWIDPNQGCNLDAIKVFCNMETGETCVYPTQPSVAQKNWYISKNPKDKRHVWFGESMTDGFQFEYGGQGSDPADVAIQLTFLRLMSTEASQNITYHCKNSVAYMDQQTGNLKKALLLKGSNEIEIRAEGNSRFTYSVTVDGCTSHTGAWGKTVIEYKTTKSSRLPIIDVAPLDVGAPDQEFGFDVGPVCFL

SEQ ID NO: 75 - protein, 311 aa, synthetic construct
  source 1..311: note; note (original language) = Trimerized peptide (type I) with glycine-X-Y repeat and D→N mutation at the BMP-1 site, KS version; organism (original language) = Synthetic construct
RSNGLPGPIGPPGPRGRTGDAGPVGPPGPPGPPGPPGPPSAGFDFSFLPQPPQEKAHDGGRYYRANDANVVRDRDLEVDTTLKSLSQQIENIRSPEGSRKNPARTCRDLKMCHSDWKSGEYWIDPNQGCNLDAIKVFCNMETGETCVYPTQPSVAQKNWYISKNPKDKRHVWFGESMTDGFQFEYGGQGSDPADVAIQLTFLRLMSTEASQNITYHCKNSVAYMDQQTGNLKKALLLKGSNEIEIRAEGNSRFTYSVTVDGCTSHTGAWGKTVIEYKTTKSSRLPIIDVAPLDVGAPDQEFGFDVGPVCFL

SEQ ID NO: 76 - protein, 311 aa, synthetic construct
  source 1..311: note; note (original language) = Trimerized peptide (type I) with glycine-X-Y repeat and D→N mutation at the BMP-1 site, KS version; organism (original language) = Synthetic construct
GSNGLPGPIGPPGPRGRTGDAGPVGPPGPPGPPGPPGPPSAGFDFSFLPQPPQEKAHDGGRYYRANDANVVRDRDLEVDTTLKSLSQQIENIRSPEGSRKNPARTCRDLKMCHSDWKSGEYWIDPNQGCNLDAIKVFCNMETGETCVYPTQPSVAQKNWYISKNPKDKRHVWFGESMTDGFQFEYGGQGSDPADVAIQLTFLRLMSTEASQNITYHCKNSVAYMDQQTGNLKKALLLKGSNEIEIRAEGNSRFTYSVTVDGCTSHTGAWGKTVIEYKTTKSSRLPIIDVAPLDVGAPDQEFGFDVGPVCFL

SEQ ID NO: 77 - protein, 234 aa, synthetic construct
  source 1..234: note; note (original language) = Trimeric peptide (type III); organism (original language) = Synthetic construct
DEIMTSLKSVNGQIESLISPDGSRKNPARNCRDLKFCHPELKSGEYWVDPNQGCKLDAIKVFCNMETGETCISANPLNVPRKHWWTDSSAEKKHVWFGESMDGGFQFSYGNPELPEDVLDVQLAFLRLLSSRASQNITYHCKNSIAYMDQASGNVKKALKLMGSNEGEFKAEGNSKFTYTVLEDGCTKHTGEWSKTVFEYRTRKAVRLPIVDIAPYDIGGPDQEFGVDVGPVCF

SEQ ID NO: 78 - protein, 244 aa, synthetic construct
  source 1..244: note; note (original language) = Trimeric peptide (type III); organism (original language) = Synthetic construct
EPMDFKINTDEIMTSLKSVNGQIESLISPDGSRKNPARNCRDLKFCHPELKSGEYWVDPNQGCKLDAIKVFCNMETGETCISANPLNVPRKHWWTDSSAEKKHVWFGESMDGGFQFSYGNPELPEDVLDVQLAFLRLLSSRASQNITYHCKNSIAYMDQASGNVKKALKLMGSNEGEFKAEGNSKFTYTVLEDGCTKHTGEWSKTVFEYRTRKAVRLPIVDIAPYDIGGPDQEFGVDVGPVCFL

SEQ ID NO: 79 - protein, 245 aa, synthetic construct
  source 1..245: note; note (original language) = Trimeric peptide (type III); organism (original language) = Synthetic construct
SEPMDFKINTDEIMTSLKSVNGQIESLISPDGSRKNPARNCRDLKFCHPELKSGEYWVDPNQGCKLDAIKVFCNMETGETCISANPLNVPRKHWWTDSSAEKKHVWFGESMDGGFQFSYGNPELPEDVLDVQLAFLRLLSSRASQNITYHCKNSIAYMDQASGNVKKALKLMGSNEGEFKAEGNSKFTYTVLEDGCTKHTGEWSKTVFEYRTRKAVRLPIVDIAPYDIGGPDQEFGVDVGPVCFL

SEQ ID NO: 80 - protein, 246 aa, synthetic construct
  source 1..246: note; note (original language) = Trimeric peptide (type III); organism (original language) = Synthetic construct
RSEPMDFKINTDEIMTSLKSVNGQIESLISPDGSRKNPARNCRDLKFCHPELKSGEYWVDPNQGCKLDAIKVFCNMETGETCISANPLNVPRKHWWTDSSAEKKHVWFGESMDGGFQFSYGNPELPEDVLDVQLAFLRLLSSRASQNITYHCKNSIAYMDQASGNVKKALKLMGSNEGEFKAEGNSKFTYTVLEDGCTKHTGEWSKTVFEYRTRKAVRLPIVDIAPYDIGGPDQEFGVDVGPVCFL

SEQ ID NO: 81 - protein, 1195 aa, synthetic construct
  source 1..1195: note; note (original language) = SARS-CoV-2 Omicron spike protein extracellular domain without signal peptide; organism (original language) = Synthetic construct
QCVNLTTRTQLPPAYTNSFTRGVYYPDKVFRSSVLHSTQDLFLPFFSNVTWFHVISGTNGTKRFDNPVLPFNDGVYFASIEKSNIIRGWIFGTTLDSKTQSLLIVNNATNVVIKVCEFQFCNDPFLDHKNNKSWMESEFRVYSSANNCTFEYVSQPFLMDLEGKQGNFKNLREFVFKNIDGYFKIYSKHTPIIVREPEDLPQGFSALEPLVDLPIGINITRFQTLLALHRSYLTPGDSSSGWTAGAAAYYVGYLQPRTFLLKYNENGTITDAVDCALDPLSETKCTLKSFTVEKGIYQTSNFRVQPTESIVRFPNITNLCPFDEVFNATKFASVYAWNRKRISNCVADYSVLYNLAPFFTFKCYGVSPTKLNDLCFTNVYADSFVIRGDEVRQIAPGQTGNIADYNYKLPDDFTGCVIAWNSNKLDSKVSGNYNYLYRLFRKSNLKPFERDISTEIYQAGNKPCNGVAGFNCYFPLRSYSFRPTYGVGHQPYRVVVLSFELLHAPATVCGPKKSTNLVKNKCVNFNFNGLKGTGVLTESNKKFLPFQQFGRDIADTTDAVRDPQTLEILDITPCSFGGVSVITPGTNTSNQVAVLYQGVNCTEVPVAIHADQLTPTWRVYSTGSNVFQTRAGCLIGAEYVNNSYECDIPIGAGICASYQTQTKSHRRARSVASQSIIAYTMSLGAENSVAYSNNSIAIPTNFTISVTTEILPVSMTKTSVDCTMYICGDSTECSNLLLQYGSFCTQLKRALTGIAVEQDKNTQEVFAQVKQIYKTPPIKYFGGFNFSQILPDPSKPSKRSFIEDLLFNKVTLADAGFIKQYGDCLGDIAARDLICAQKFKGLTVLPPLLTDEMIAQYTSALLAGTITSGWTFGAGAALQIPFAMQMAYRFNGIGVTQNVLYENQKLIANQFNSAIGKIQDSLSSTASALGKLQDVVNHNAQALNTLVKQLSSKFGAISSVLNDIFSRLDKVEAEVQIDRLITGRLQSLQTYVTQQLIRAAEIRASANLAATKMSECVLGQSKRVDFCGKGYHLMSFPQSAPHGVVFLHVTYVPAQEKNFTTAPAICHDGKAHFPREGVFVSNGTHWFVTQRNFYEPQIITTDNTFVSGNCDVVIGIVNNTVYDPLQPELDSFKEELDKYFKNHTSPDVDLGDISGINASVVNIQKEIDRLNEVAKNLNESLIDLQELGKYEQYIK

SEQ ID NO: 82 - protein, 1195 aa, synthetic construct
  source 1..1195: note; note (original language) = SARS-CoV-2 Omicron spike protein extracellular domain without signal peptide, S1/S2 furin cleavage site 1 mutant (685R→685A); organism (original language) = Synthetic construct
QCVNLTTRTQLPPAYTNSFTRGVYYPDKVFRSSVLHSTQDLFLPFFSNVTWFHVISGTNGTKRFDNPVLPFNDGVYFASIEKSNIIRGWIFGTTLDSKTQSLLIVNNATNVVIKVCEFQFCNDPFLDHKNNKSWMESEFRVYSSANNCTFEYVSQPFLMDLEGKQGNFKNLREFVFKNIDGYFKIYSKHTPIIVREPEDLPQGFSALEPLVDLPIGINITRFQTLLALHRSYLTPGDSSSGWTAGAAAYYVGYLQPRTFLLKYNENGTITDAVDCALDPLSETKCTLKSFTVEKGIYQTSNFRVQPTESIVRFPNITNLCPFDEVFNATKFASVYAWNRKRISNCVADYSVLYNLAPFFTFKCYGVSPTKLNDLCFTNVYADSFVIRGDEVRQIAPGQTGNIADYNYKLPDDFTGCVIAWNSNKLDSKVSGNYNYLYRLFRKSNLKPFERDISTEIYQAGNKPCNGVAGFNCYFPLRSYSFRPTYGVGHQPYRVVVLSFELLHAPATVCGPKKSTNLVKNKCVNFNFNGLKGTGVLTESNKKFLPFQQFGRDIADTTDAVRDPQTLEILDITPCSFGGVSVITPGTNTSNQVAVLYQGVNCTEVPVAIHADQLTPTWRVYSTGSNVFQTRAGCLIGAEYVNNSYECDIPIGAGICASYQTQTKSHRRAASVASQSIIAYTMSLGAENSVAYSNNSIAIPTNFTISVTTEILPVSMTKTSVDCTMYICGDSTECSNLLLQYGSFCTQLKRALTGIAVEQDKNTQEVFAQVKQIYKTPPIKYFGGFNFSQILPDPSKPSKRSFIEDLLFNKVTLADAGFIKQYGDCLGDIAARDLICAQKFKGLTVLPPLLTDEMIAQYTSALLAGTITSGWTFGAGAALQIPFAMQMAYRFNGIGVTQNVLYENQKLIANQFNSAIGKIQDSLSSTASALGKLQDVVNHNAQALNTLVKQLSSKFGAISSVLNDIFSRLDKVEAEVQIDRLITGRLQSLQTYVTQQLIRAAEIRASANLAATKMSECVLGQSKRVDFCGKGYHLMSFPQSAPHGVVFLHVTYVPAQEKNFTTAPAICHDGKAHFPREGVFVSNGTHWFVTQRNFYEPQIITTDNTFVSGNCDVVIGIVNNTVYDPLQPELDSFKEELDKYFKNHTSPDVDLGDISGINASVVNIQKEIDRLNEVAKNLNESLIDLQELGKYEQYIK

SEQ ID NO: 83 - protein, 1195 aa, synthetic construct
  source 1..1195: note; note (original language) = SARS-CoV-2 Omicron spike protein extracellular domain without signal peptide, S1/S2 furin cleavage site 1 and proline mutant (685R→685A, 986K/987V→986P/987P); organism (original language) = Synthetic construct
QCVNLTTRTQLPPAYTNSFTRGVYYPDKVFRSSVLHSTQDLFLPFFSNVTWFHVISGTNGTKRFDNPVLPFNDGVYFASIEKSNIIRGWIFGTTLDSKTQSLLIVNNATNVVIKVCEFQFCNDPFLDHKNNKSWMESEFRVYSSANNCTFEYVSQPFLMDLEGKQGNFKNLREFVFKNIDGYFKIYSKHTPIIVREPEDLPQGFSALEPLVDLPIGINITRFQTLLALHRSYLTPGDSSSGWTAGAAAYYVGYLQPRTFLLKYNENGTITDAVDCALDPLSETKCTLKSFTVEKGIYQTSNFRVQPTESIVRFPNITNLCPFDEVFNATKFASVYAWNRKRISNCVADYSVLYNLAPFFTFKCYGVSPTKLNDLCFTNVYADSFVIRGDEVRQIAPGQTGNIADYNYKLPDDFTGCVIAWNSNKLDSKVSGNYNYLYRLFRKSNLKPFERDISTEIYQAGNKPCNGVAGFNCYFPLRSYSFRPTYGVGHQPYRVVVLSFELLHAPATVCGPKKSTNLVKNKCVNFNFNGLKGTGVLTESNKKFLPFQQFGRDIADTTDAVRDPQTLEILDITPCSFGGVSVITPGTNTSNQVAVLYQGVNCTEVPVAIHADQLTPTWRVYSTGSNVFQTRAGCLIGAEYVNNSYECDIPIGAGICASYQTQTKSHRRAASVASQSIIAYTMSLGAENSVAYSNNSIAIPTNFTISVTTEILPVSMTKTSVDCTMYICGDSTECSNLLLQYGSFCTQLKRALTGIAVEQDKNTQEVFAQVKQIYKTPPIKYFGGFNFSQILPDPSKPSKRSFIEDLLFNKVTLADAGFIKQYGDCLGDIAARDLICAQKFKGLTVLPPLLTDEMIAQYTSALLAGTITSGWTFGAGAALQIPFAMQMAYRFNGIGVTQNVLYENQKLIANQFNSAIGKIQDSLSSTASALGKLQDVVNHNAQALNTLVKQLSSKFGAISSVLNDIFSRLDPPEAEVQIDRLITGRLQSLQTYVTQQLIRAAEIRASANLAATKMSECVLGQSKRVDFCGKGYHLMSFPQSAPHGVVFLHVTYVPAQEKNFTTAPAICHDGKAHFPREGVFVSNGTHWFVTQRNFYEPQIITTDNTFVSGNCDVVIGIVNNTVYDPLQPELDSFKEELDKYFKNHTSPDVDLGDISGINASVVNIQKEIDRLNEVAKNLNESLIDLQELGKYEQYIK

SEQ ID NO: 84 - protein, 1195 aa, synthetic construct
  source 1..1195: note; note (original language) = SARS-CoV-2 Omicron spike protein extracellular domain without signal peptide, proline mutant (986K/987V→986P/987P); organism (original language) = Synthetic construct
QCVNLTTRTQLPPAYTNSFTRGVYYPDKVFRSSVLHSTQDLFLPFFSNVTWFHVISGTNGTKRFDNPVLPFNDGVYFASIEKSNIIRGWIFGTTLDSKTQSLLIVNNATNVVIKVCEFQFCNDPFLDHKNNKSWMESEFRVYSSANNCTFEYVSQPFLMDLEGKQGNFKNLREFVFKNIDGYFKIYSKHTPIIVREPEDLPQGFSALEPLVDLPIGINITRFQTLLALHRSYLTPGDSSSGWTAGAAAYYVGYLQPRTFLLKYNENGTITDAVDCALDPLSETKCTLKSFTVEKGIYQTSNFRVQPTESIVRFPNITNLCPFDEVFNATKFASVYAWNRKRISNCVADYSVLYNLAPFFTFKCYGVSPTKLNDLCFTNVYADSFVIRGDEVRQIAPGQTGNIADYNYKLPDDFTGCVIAWNSNKLDSKVSGNYNYLYRLFRKSNLKPFERDISTEIYQAGNKPCNGVAGFNCYFPLRSYSFRPTYGVGHQPYRVVVLSFELLHAPATVCGPKKSTNLVKNKCVNFNFNGLKGTGVLTESNKKFLPFQQFGRDIADTTDAVRDPQTLEILDITPCSFGGVSVITPGTNTSNQVAVLYQGVNCTEVPVAIHADQLTPTWRVYSTGSNVFQTRAGCLIGAEYVNNSYECDIPIGAGICASYQTQTKSHRRARSVASQSIIAYTMSLGAENSVAYSNNSIAIPTNFTISVTTEILPVSMTKTSVDCTMYICGDSTECSNLLLQYGSFCTQLKRALTGIAVEQDKNTQEVFAQVKQIYKTPPIKYFGGFNFSQILPDPSKPSKRSFIEDLLFNKVTLADAGFIKQYGDCLGDIAARDLICAQKFKGLTVLPPLLTDEMIAQYTSALLAGTITSGWTFGAGAALQIPFAMQMAYRFNGIGVTQNVLYENQKLIANQFNSAIGKIQDSLSSTASALGKLQDVVNHNAQALNTLVKQLSSKFGAISSVLNDIFSRLDPPEAEVQIDRLITGRLQSLQTYVTQQLIRAAEIRASANLAATKMSECVLGQSKRVDFCGKGYHLMSFPQSAPHGVVFLHVTYVPAQEKNFTTAPAICHDGKAHFPREGVFVSNGTHWFVTQRNFYEPQIITTDNTFVSGNCDVVIGIVNNTVYDPLQPELDSFKEELDKYFKNHTSPDVDLGDISGINASVVNIQKEIDRLNEVAKNLNESLIDLQELGKYEQYIK

SEQ ID NO: 85 - protein, 1506 aa, synthetic construct
  source 1..1506: note; note (original language) = SARS-CoV-2 Omicron S-trimer fusion polypeptide without signal peptide; organism (original language) = Synthetic construct
QCVNLTTRTQLPPAYTNSFTRGVYYPDKVFRSSVLHSTQDLFLPFFSNVTWFHVISGTNGTKRFDNPVLPFNDGVYFASIEKSNIIRGWIFGTTLDSKTQSLLIVNNATNVVIKVCEFQFCNDPFLDHKNNKSWMESEFRVYSSANNCTFEYVSQPFLMDLEGKQGNFKNLREFVFKNIDGYFKIYSKHTPIIVREPEDLPQGFSALEPLVDLPIGINITRFQTLLALHRSYLTPGDSSSGWTAGAAAYYVGYLQPRTFLLKYNENGTITDAVDCALDPLSETKCTLKSFTVEKGIYQTSNFRVQPTESIVRFPNITNLCPFDEVFNATKFASVYAWNRKRISNCVADYSVLYNLAPFFTFKCYGVSPTKLNDLCFTNVYADSFVIRGDEVRQIAPGQTGNIADYNYKLPDDFTGCVIAWNSNKLDSKVSGNYNYLYRLFRKSNLKPFERDISTEIYQAGNKPCNGVAGFNCYFPLRSYSFRPTYGVGHQPYRVVVLSFELLHAPATVCGPKKSTNLVKNKCVNFNFNGLKGTGVLTESNKKFLPFQQFGRDIADTTDAVRDPQTLEILDITPCSFGGVSVITPGTNTSNQVAVLYQGVNCTEVPVAIHADQLTPTWRVYSTGSNVFQTRAGCLIGAEYVNNSYECDIPIGAGICASYQTQTKSHRRARSVASQSIIAYTMSLGAENSVAYSNNSIAIPTNFTISVTTEILPVSMTKTSVDCTMYICGDSTECSNLLLQYGSFCTQLKRALTGIAVEQDKNTQEVFAQVKQIYKTPPIKYFGGFNFSQILPDPSKPSKRSFIEDLLFNKVTLADAGFIKQYGDCLGDIAARDLICAQKFKGLTVLPPLLTDEMIAQYTSALLAGTITSGWTFGAGAALQIPFAMQMAYRFNGIGVTQNVLYENQKLIANQFNSAIGKIQDSLSSTASALGKLQDVVNHNAQALNTLVKQLSSKFGAISSVLNDIFSRLDKVEAEVQIDRLITGRLQSLQTYVTQQLIRAAEIRASANLAATKMSECVLGQSKRVDFCGKGYHLMSFPQSAPHGVVFLHVTYVPAQEKNFTTAPAICHDGKAHFPREGVFVSNGTHWFVTQRNFYEPQIITTDNTFVSGNCDVVIGIVNNTVYDPLQPELDSFKEELDKYFKNHTSPDVDLGDISGINASVVNIQKEIDRLNEVAKNLNESLIDLQELGKYEQYIKRSNGLPGPIGPPGPRGRTGDAGPVGPPGPPGPPGPPGPPSAGFDFSFLPQPPQEKAHDGGRYYRANDANVVRDRDLEVDTTLKSLSQQIENIRSPEGSRKNPARTCRDLKMCHSDWKSGEYWIDPNQGCNLDAIKVFCNMETGETCVYPTQPSVAQKNWYISKNPKDKRHVWFGESMTDGFQFEYGGQGSDPADVAIQLTFLRLMSTEASQNITYHCKNSVAYMDQQTGNLKKALLLQGSNEIEIRAEGNSRFTYSVTVDGCTSHTGAWGKTVIEYKTTKTSRLPIIDVAPLDVGAPDQEFGFDVGPVCFL

SEQ ID NO: 86 - protein, 1506 aa, synthetic construct
  source 1..1506: note; note (original language) = SARS-CoV-2 Omicron S-trimer fusion polypeptide without signal peptide, S1/S2 furin cleavage site 1 mutant (685R→685A); organism (original language) = Synthetic construct
QCVNLTTRTQLPPAYTNSFTRGVYYPDKVFRSSVLHSTQDLFLPFFSNVTWFHVISGTNGTKRFDNPVLPFNDGVYFASIEKSNIIRGWIFGTTLDSKTQSLLIVNNATNVVIKVCEFQFCNDPFLDHKNNKSWMESEFRVYSSANNCTFEYVSQPFLMDLEGKQGNFKNLREFVFKNIDGYFKIYSKHTPIIVREPEDLPQGFSALEPLVDLPIGINITRFQTLLALHRSYLTPGDSSSGWTAGAAAYYVGYLQPRTFLLKYNENGTITDAVDCALDPLSETKCTLKSFTVEKGIYQTSNFRVQPTESIVRFPNITNLCPFDEVFNATKFASVYAWNRKRISNCVADYSVLYNLAPFFTFKCYGVSPTKLNDLCFTNVYADSFVIRGDEVRQIAPGQTGNIADYNYKLPDDFTGCVIAWNSNKLDSKVSGNYNYLYRLFRKSNLKPFERDISTEIYQAGNKPCNGVAGFNCYFPLRSYSFRPTYGVGHQPYRVVVLSFELLHAPATVCGPKKSTNLVKNKCVNFNFNGLKGTGVLTESNKKFLPFQQFGRDIADTTDAVRDPQTLEILDITPCSFGGVSVITPGTNTSNQVAVLYQGVNCTEVPVAIHADQLTPTWRVYSTGSNVFQTRAGCLIGAEYVNNSYECDIPIGAGICASYQTQTKSHRRAASVASQSIIAYTMSLGAENSVAYSNNSIAIPTNFTISVTTEILPVSMTKTSVDCTMYICGDSTECSNLLLQYGSFCTQLKRALTGIAVEQDKNTQEVFAQVKQIYKTPPIKYFGGFNFSQILPDPSKPSKRSFIEDLLFNKVTLADAGFIKQYGDCLGDIAARDLICAQKFKGLTVLPPLLTDEMIAQYTSALLAGTITSGWTFGAGAALQIPFAMQMAYRFNGIGVTQNVLYENQKLIANQFNSAIGKIQDSLSSTASALGKLQDVVNHNAQALNTLVKQLSSKFGAISSVLNDIFSRLDKVEAEVQIDRLITGRLQSLQTYVTQQLIRAAEIRASANLAATKMSECVLGQSKRVDFCGKGYHLMSFPQSAPHGVVFLHVTYVPAQEKNFTTAPAICHDGKAHFPREGVFVSNGTHWFVTQRNFYEPQIITTDNTFVSGNCDVVIGIVNNTVYDPLQPELDSFKEELDKYFKNHTSPDVDLGDISGINASVVNIQKEIDRLNEVAKNLNESLIDLQELGKYEQYIKRSNGLPGPIGPPGPRGRTGDAGPVGPPGPPGPPGPPGPPSAGFDFSFLPQPPQEKAHDGGRYYRANDANVVRDRDLEVDTTLKSLSQQIENIRSPEGSRKNPARTCRDLKMCHSDWKSGEYWIDPNQGCNLDAIKVFCNMETGETCVYPTQPSVAQKNWYISKNPKDKRHVWFGESMTDGFQFEYGGQGSDPADVAIQLTFLRLMSTEASQNITYHCKNSVAYMDQQTGNLKKALLLQGSNEIEIRAEGNSRFTYSVTVDGCTSHTGAWGKTVIEYKTTKTSRLPIIDVAPLDVGAPDQEFGFDVGPVCFL

SEQ ID NO: 87 - protein, 1506 aa, synthetic construct
  source 1..1506: note; note (original language) = SARS-CoV-2 Omicron S-trimer fusion polypeptide without signal peptide, S1/S2 furin cleavage site 1 and proline mutant (685R→685A, 986K/987V→986P/987P); organism (original language) = Synthetic construct
QCVNLTTRTQLPPAYTNSFTRGVYYPDKVFRSSVLHSTQDLFLPFFSNVTWFHVISGTNGTKRFDNPVLPFNDGVYFASIEKSNIIRGWIFGTTLDSKTQSLLIVNNATNVVIKVCEFQFCNDPFLDHKNNKSWMESEFRVYSSANNCTFEYVSQPFLMDLEGKQGNFKNLREFVFKNIDGYFKIYSKHTPIIVREPEDLPQGFSALEPLVDLPIGINITRFQTLLALHRSYLTPGDSSSGWTAGAAAYYVGYLQPRTFLLKYNENGTITDAVDCALDPLSETKCTLKSFTVEKGIYQTSNFRVQPTESIVRFPNITNLCPFDEVFNATKFASVYAWNRKRISNCVADYSVLYNLAPFFTFKCYGVSPTKLNDLCFTNVYADSFVIRGDEVRQIAPGQTGNIADYNYKLPDDFTGCVIAWNSNKLDSKVSGNYNYLYRLFRKSNLKPFERDISTEIYQAGNKPCNGVAGFNCYFPLRSYSFRPTYGVGHQPYRVVVLSFELLHAPATVCGPKKSTNLVKNKCVNFNFNGLKGTGVLTESNKKFLPFQQFGRDIADTTDAVRDPQTLEILDITPCSFGGVSVITPGTNTSNQVAVLYQGVNCTEVPVAIHADQLTPTWRVYSTGSNVFQTRAGCLIGAEYVNNSYECDIPIGAGICASYQTQTKSHRRAASVASQSIIAYTMSLGAENSVAYSNNSIAIPTNFTISVTTEILPVSMTKTSVDCTMYICGDSTECSNLLLQYGSFCTQLKRALTGIAVEQDKNTQEVFAQVKQIYKTPPIKYFGGFNFSQILPDPSKPSKRSFIEDLLFNKVTLADAGFIKQYGDCLGDIAARDLICAQKFKGLTVLPPLLTDEMIAQYTSALLAGTITSGWTFGAGAALQIPFAMQMAYRFNGIGVTQNVLYENQKLIANQFNSAIGKIQDSLSSTASALGKLQDVVNHNAQALNTLVKQLSSKFGAISSVLNDIFSRLDPPEAEVQIDRLITGRLQSLQTYVTQQLIRAAEIRASANLAATKMSECVLGQSKRVDFCGKGYHLMSFPQSAPHGVVFLHVTYVPAQEKNFTTAPAICHDGKAHFPREGVFVSNGTHWFVTQRNFYEPQIITTDNTFVSGNCDVVIGIVNNTVYDPLQPELDSFKEELDKYFKNHTSPDVDLGDISGINASVVNIQKEIDRLNEVAKNLNESLIDLQELGKYEQYIKRSNGLPGPIGPPGPRGRTGDAGPVGPPGPPGPPGPPGPPSAGFDFSFLPQPPQEKAHDGGRYYRANDANVVRDRDLEVDTTLKSLSQQIENIRSPEGSRKNPARTCRDLKMCHSDWKSGEYWIDPNQGCNLDAIKVFCNMETGETCVYPTQPSVAQKNWYISKNPKDKRHVWFGESMTDGFQFEYGGQGSDPADVAIQLTFLRLMSTEASQNITYHCKNSVAYMDQQTGNLKKALLLQGSNEIEIRAEGNSRFTYSVTVDGCTSHTGAWGKTVIEYKTTKTSRLPIIDVAPLDVGAPDQEFGFDVGPVCFL

SEQ ID NO: 88 - protein, 1506 aa, synthetic construct
  source 1..1506: note; note (original language) = SARS-CoV-2 Omicron S-trimer fusion polypeptide without signal peptide, proline mutant (986K/987V→986P/987P); organism (original language) = Synthetic construct
QCVNLTTRTQLPPAYTNSFTRGVYYPDKVFRSSVLHSTQDLFLPFFSNVTWFHVISGTNGTKRFDNPVLPFNDGVYFASIEKSNIIRGWIFGTTLDSKTQSLLIVNNATNVVIKVCEFQFCNDPFLDHKNNKSWMESEFRVYSSANNCTFEYVSQPFLMDLEGKQGNFKNLREFVFKNIDGYFKIYSKHTPIIVREPEDLPQGFSALEPLVDLPIGINITRFQTLLALHRSYLTPGDSSSGWTAGAAAYYVGYLQPRTFLLKYNENGTITDAVDCALDPLSETKCTLKSFTVEKGIYQTSNFRVQPTESIVRFPNITNLCPFDEVFNATKFASVYAWNRKRISNCVADYSVLYNLAPFFTFKCYGVSPTKLNDLCFTNVYADSFVIRGDEVRQIAPGQTGNIADYNYKLPDDFTGCVIAWNSNKLDSKVSGNYNYLYRLFRKSNLKPFERDISTEIYQAGNKPCNGVAGFNCYFPLRSYSFRPTYGVGHQPYRVVVLSFELLHAPATVCGPKKSTNLVKNKCVNFNFNGLKGTGVLTESNKKFLPFQQFGRDIADTTDAVRDPQTLEILDITPCSFGGVSVITPGTNTSNQVAVLYQGVNCTEVPVAIHADQLTPTWRVYSTGSNVFQTRAGCLIGAEYVNNSYECDIPIGAGICASYQTQTKSHRRARSVASQSIIAYTMSLGAENSVAYSNNSIAIPTNFTISVTTEILPVSMTKTSVDCTMYICGDSTECSNLLLQYGSFCTQLKRALTGIAVEQDKNTQEVFAQVKQIYKTPPIKYFGGFNFSQILPDPSKPSKRSFIEDLLFNKVTLADAGFIKQYGDCLGDIAARDLICAQKFKGLTVLPPLLTDEMIAQYTSALLAGTITSGWTFGAGAALQIPFAMQMAYRFNGIGVTQNVLYENQKLIANQFNSAIGKIQDSLSSTASALGKLQDVVNHNAQALNTLVKQLSSKFGAISSVLNDIFSRLDPPEAEVQIDRLITGRLQSLQTYVTQQLIRAAEIRASANLAATKMSECVLGQSKRVDFCGKGYHLMSFPQSAPHGVVFLHVTYVPAQEKNFTTAPAICHDGKAHFPREGVFVSNGTHWFVTQRNFYEPQIITTDNTFVSGNCDVVIGIVNNTVYDPLQPELDSFKEELDKYFKNHTSPDVDLGDISGINASVVNIQKEIDRLNEVAKNLNESLIDLQELGKYEQYIKRSNGLPGPIGPPGPRGRTGDAGPVGPPGPPGPPGPPGPPSAGFDFSFLPQPPQEKAHDGGRYYRANDANVVRDRDLEVDTTLKSLSQQIENIRSPEGSRKNPARTCRDLKMCHSDWKSGEYWIDPNQGCNLDAIKVFCNMETGETCVYPTQPSVAQKNWYISKNPKDKRHVWFGESMTDGFQFEYGGQGSDPADVAIQLTFLRLMSTEASQNITYHCKNSVAYMDQQTGNLKKALLLQGSNEIEIRAEGNSRFTYSVTVDGCTSHTGAWGKTVIEYKTTKTSRLPIIDVAPLDVGAPDQEFGFDVGPVCFL

SEQ ID NO: 89 - protein, 1519 aa, synthetic construct
  source 1..1519: note; note (original language) = SARS-CoV-2 Omicron S-trimer fusion polypeptide with signal peptide; organism (original language) = Synthetic construct
MFVFLVLLPLVSSQCVNLTTRTQLPPAYTNSFTRGVYYPDKVFRSSVLHSTQDLFLPFFSNVTWFHVISGTNGTKRFDNPVLPFNDGVYFASIEKSNIIRGWIFGTTLDSKTQSLLIVNNATNVVIKVCEFQFCNDPFLDHKNNKSWMESEFRVYSSANNCTFEYVSQPFLMDLEGKQGNFKNLREFVFKNIDGYFKIYSKHTPIIVREPEDLPQGFSALEPLVDLPIGINITRFQTLLALHRSYLTPGDSSSGWTAGAAAYYVGYLQPRTFLLKYNENGTITDAVDCALDPLSETKCTLKSFTVEKGIYQTSNFRVQPTESIVRFPNITNLCPFDEVFNATKFASVYAWNRKRISNCVADYSVLYNLAPFFTFKCYGVSPTKLNDLCFTNVYADSFVIRGDEVRQIAPGQTGNIADYNYKLPDDFTGCVIAWNSNKLDSKVSGNYNYLYRLFRKSNLKPFERDISTEIYQAGNKPCNGVAGFNCYFPLRSYSFRPTYGVGHQPYRVVVLSFELLHAPATVCGPKKSTNLVKNKCVNFNFNGLKGTGVLTESNKKFLPFQQFGRDIADTTDAVRDPQTLEILDITPCSFGGVSVITPGTNTSNQVAVLYQGVNCTEVPVAIHADQLTPTWRVYSTGSNVFQTRAGCLIGAEYVNNSYECDIPIGAGICASYQTQTKSHRRARSVASQSIIAYTMSLGAENSVAYSNNSIAIPTNFTISVTTEILPVSMTKTSVDCTMYICGDSTECSNLLLQYGSFCTQLKRALTGIAVEQDKNTQEVFAQVKQIYKTPPIKYFGGFNFSQILPDPSKPSKRSFIEDLLFNKVTLADAGFIKQYGDCLGDIAARDLICAQKFKGLTVLPPLLTDEMIAQYTSALLAGTITSGWTFGAGAALQIPFAMQMAYRFNGIGVTQNVLYENQKLIANQFNSAIGKIQDSLSSTASALGKLQDVVNHNAQALNTLVKQLSSKFGAISSVLNDIFSRLDKVEAEVQIDRLITGRLQSLQTYVTQQLIRAAEIRASANLAATKMSECVLGQSKRVDFCGKGYHLMSFPQSAPHGVVFLHVTYVPAQEKNFTTAPAICHDGKAHFPREGVFVSNGTHWFVTQRNFYEPQIITTDNTFVSGNCDVVIGIVNNTVYDPLQPELDSFKEELDKYFKNHTSPDVDLGDISGINASVVNIQKEIDRLNEVAKNLNESLIDLQELGKYEQYIKRSNGLPGPIGPPGPRGRTGDAGPVGPPGPPGPPGPPGPPSAGFDFSFLPQPPQEKAHDGGRYYRANDANVVRDRDLEVDTTLKSLSQQIENIRSPEGSRKNPARTCRDLKMCHSDWKSGEYWIDPNQGCNLDAIKVFCNMETGETCVYPTQPSVAQKNWYISKNPKDKRHVWFGESMTDGFQFEYGGQGSDPADVAIQLTFLRLMSTEASQNITYHCKNSVAYMDQQTGNLKKALLLQGSNEIEIRAEGNSRFTYSVTVDGCTSHTGAWGKTVIEYKTTKTSRLPIIDVAPLDVGAPDQEFGFDVGPVCFL

SEQ ID NO: 90 - protein, 1519 aa, synthetic construct
  source 1..1519: note; note (original language) = SARS-CoV-2 Omicron S-trimer fusion polypeptide with signal peptide, S1/S2 furin cleavage site 1 mutant (685R→685A); organism (original language) = Synthetic construct
MFVFLVLLPLVSSQCVNLTTRTQLPPAYTNSFTRGVYYPDKVFRSSVLHSTQDLFLPFFSNVTWFHVISGTNGTKRFDNPVLPFNDGVYFASIEKSNIIRGWIFGTTLDSKTQSLLIVNNATNVVIKVCEFQFCNDPFLDHKNNKSWMESEFRVYSSANNCTFEYVSQPFLMDLEGKQGNFKNLREFVFKNIDGYFKIYSKHTPIIVREPEDLPQGFSALEPLVDLPIGINITRFQTLLALHRSYLTPGDSSSGWTAGAAAYYVGYLQPRTFLLKYNENGTITDAVDCALDPLSETKCTLKSFTVEKGIYQTSNFRVQPTESIVRFPNITNLCPFDEVFNATKFASVYAWNRKRISNCVADYSVLYNLAPFFTFKCYGVSPTKLNDLCFTNVYADSFVIRGDEVRQIAPGQTGNIADYNYKLPDDFTGCVIAWNSNKLDSKVSGNYNYLYRLFRKSNLKPFERDISTEIYQAGNKPCNGVAGFNCYFPLRSYSFRPTYGVGHQPYRVVVLSFELLHAPATVCGPKKSTNLVKNKCVNFNFNGLKGTGVLTESNKKFLPFQQFGRDIADTTDAVRDPQTLEILDITPCSFGGVSVITPGTNTSNQVAVLYQGVNCTEVPVAIHADQLTPTWRVYSTGSNVFQTRAGCLIGAEYVNNSYECDIPIGAGICASYQTQTKSHRRAASVASQSIIAYTMSLGAENSVAYSNNSIAIPTNFTISVTTEILPVSMTKTSVDCTMYICGDSTECSNLLLQYGSFCTQLKRALTGIAVEQDKNTQEVFAQVKQIYKTPPIKYFGGFNFSQILPDPSKPSKRSFIEDLLFNKVTLADAGFIKQYGDCLGDIAARDLICAQKFKGLTVLPPLLTDEMIAQYTSALLAGTITSGWTFGAGAALQIPFAMQMAYRFNGIGVTQNVLYENQKLIANQFNSAIGKIQDSLSSTASALGKLQDVVNHNAQALNTLVKQLSSKFGAISSVLNDIFSRLDKVEAEVQIDRLITGRLQSLQTYVTQQLIRAAEIRASANLAATKMSECVLGQSKRVDFCGKGYHLMSFPQSAPHGVVFLHVTYVPAQEKNFTTAPAICHDGKAHFPREGVFVSNGTHWFVTQRNFYEPQIITTDNTFVSGNCDVVIGIVNNTVYDPLQPELDSFKEELDKYFKNHTSPDVDLGDISGINASVVNIQKEIDRLNEVAKNLNESLIDLQELGKYEQYIKRSNGLPGPIGPPGPRGRTGDAGPVGPPGPPGPPGPPGPPSAGFDFSFLPQPPQEKAHDGGRYYRANDANVVRDRDLEVDTTLKSLSQQIENIRSPEGSRKNPARTCRDLKMCHSDWKSGEYWIDPNQGCNLDAIKVFCNMETGETCVYPTQPSVAQKNWYISKNPKDKRHVWFGESMTDGFQFEYGGQGSDPADVAIQLTFLRLMSTEASQNITYHCKNSVAYMDQQTGNLKKALLLQGSNEIEIRAEGNSRFTYSVTVDGCTSHTGAWGKTVIEYKTTKTSRLPIIDVAPLDVGAPDQEFGFDVGPVCFL

SEQ ID NO: 91 - protein, 1519 aa, synthetic construct
  source 1..1519: note; note (original language) = SARS-CoV-2 Omicron S-trimer fusion polypeptide with signal peptide, S1/S2 furin cleavage site 1 and proline mutant (685R→685A, 986K/987V→986P/987P); organism (original language) = Synthetic construct
MFVFLVLLPLVSSQCVNLTTRTQLPPAYTNSFTRGVYYPDKVFRSSVLHSTQDLFLPFFSNVTWFHVISGTNGTKRFDNPVLPFNDGVYFASIEKSNIIRGWIFGTTLDSKTQSLLIVNNATNVVIKVCEFQFCNDPFLDHKNNKSWMESEFRVYSSANNCTFEYVSQPFLMDLEGKQGNFKNLREFVFKNIDGYFKIYSKHTPIIVREPEDLPQGFSALEPLVDLPIGINITRFQTLLALHRSYLTPGDSSSGWTAGAAAYYVGYLQPRTFLLKYNENGTITDAVDCALDPLSETKCTLKSFTVEKGIYQTSNFRVQPTESIVRFPNITNLCPFDEVFNATKFASVYAWNRKRISNCVADYSVLYNLAPFFTFKCYGVSPTKLNDLCFTNVYADSFVIRGDEVRQIAPGQTGNIADYNYKLPDDFTGCVIAWNSNKLDSKVSGNYNYLYRLFRKSNLKPFERDISTEIYQAGNKPCNGVAGFNCYFPLRSYSFRPTYGVGHQPYRVVVLSFELLHAPATVCGPKKSTNLVKNKCVNFNFNGLKGTGVLTESNKKFLPFQQFGRDIADTTDAVRDPQTLEILDITPCSFGGVSVITPGTNTSNQVAVLYQGVNCTEVPVAIHADQLTPTWRVYSTGSNVFQTRAGCLIGAEYVNNSYECDIPIGAGICASYQTQTKSHRRAASVASQSIIAYTMSLGAENSVAYSNNSIAIPTNFTISVTTEILPVSMTKTSVDCTMYICGDSTECSNLLLQYGSFCTQLKRALTGIAVEQDKNTQEVFAQVKQIYKTPPIKYFGGFNFSQILPDPSKPSKRSFIEDLLFNKVTLADAGFIKQYGDCLGDIAARDLICAQKFKGLTVLPPLLTDEMIAQYTSALLAGTITSGWTFGAGAALQIPFAMQMAYRFNGIGVTQNVLYENQKLIANQFNSAIGKIQDSLSSTASALGKLQDVVNHNAQALNTLVKQLSSKFGAISSVLNDIFSRLDPPEAEVQIDRLITGRLQSLQTYVTQQLIRAAEIRASANLAATKMSECVLGQSKRVDFCGKGYHLMSFPQSAPHGVVFLHVTYVPAQEKNFTTAPAICHDGKAHFPREGVFVSNGTHWFVTQRNFYEPQIITTDNTFVSGNCDVVIGIVNNTVYDPLQPELDSFKEELDKYFKNHTSPDVDLGDISGINASVVNIQKEIDRLNEVAKNLNESLIDLQELGKYEQYIKRSNGLPGPIGPPGPRGRTGDAGPVGPPGPPGPPGPPGPPSAGFDFSFLPQPPQEKAHDGGRYYRANDANVVRDRDLEVDTTLKSLSQQIENIRSPEGSRKNPARTCRDLKMCHSDWKSGEYWIDPNQGCNLDAIKVFCNMETGETCVYPTQPSVAQKNWYISKNPKDKRHVWFGESMTDGFQFEYGGQGSDPADVAIQLTFLRLMSTEASQNITYHCKNSVAYMDQQTGNLKKALLLQGSNEIEIRAEGNSRFTYSVTVDGCTSHTGAWGKTVIEYKTTKTSRLPIIDVAPLDVGAPDQEFGFDVGPVCFL

SEQ ID NO: 92 - protein, 1519 aa, synthetic construct
  source 1..1519: note; note (original language) = SARS-CoV-2 Omicron S-trimer fusion polypeptide with signal peptide, proline mutant (986K/987V→986P/987P); organism (original language) = Synthetic construct
MFVFLVLLPLVSSQCVNLTTRTQLPPAYTNSFTRGVYYPDKVFRSSVLHSTQDLFLPFFSNVTWFHVISGTNGTKRFDNPVLPFNDGVYFASIEKSNIIRGWIFGTTLDSKTQSLLIVNNATNVVIKVCEFQFCNDPFLDHKNNKSWMESEFRVYSSANNCTFEYVSQPFLMDLEGKQGNFKNLREFVFKNIDGYFKIYSKHTPIIVREPEDLPQGFSALEPLVDLPIGINITRFQTLLALHRSYLTPGDSSSGWTAGAAAYYVGYLQPRTFLLKYNENGTITDAVDCALDPLSETKCTLKSFTVEKGIYQTSNFRVQPTESIVRFPNITNLCPFDEVFNATKFASVYAWNRKRISNCVADYSVLYNLAPFFTFKCYGVSPTKLNDLCFTNVYADSFVIRGDEVRQIAPGQTGNIADYNYKLPDDFTGCVIAWNSNKLDSKVSGNYNYLYRLFRKSNLKPFERDISTEIYQAGNKPCNGVAGFNCYFPLRSYSFRPTYGVGHQPYRVVVLSFELLHAPATVCGPKKSTNLVKNKCVNFNFNGLKGTGVLTESNKKFLPFQQFGRDIADTTDAVRDPQTLEILDITPCSFGGVSVITPGTNTSNQVAVLYQGVNCTEVPVAIHADQLTPTWRVYSTGSNVFQTRAGCLIGAEYVNNSYECDIPIGAGICASYQTQTKSHRRARSVASQSIIAYTMSLGAENSVAYSNNSIAIPTNFTISVTTEILPVSMTKTSVDCTMYICGDSTECSNLLLQYGSFCTQLKRALTGIAVEQDKNTQEVFAQVKQIYKTPPIKYFGGFNFSQILPDPSKPSKRSFIEDLLFNKVTLADAGFIKQYGDCLGDIAARDLICAQKFKGLTVLPPLLTDEMIAQYTSALLAGTITSGWTFGAGAALQIPFAMQMAYRFNGIGVTQNVLYENQKLIANQFNSAIGKIQDSLSSTASALGKLQDVVNHNAQALNTLVKQLSSKFGAISSVLNDIFSRLDPPEAEVQIDRLITGRLQSLQTYVTQQLIRAAEIRASANLAATKMSECVLGQSKRVDFCGKGYHLMSFPQSAPHGVVFLHVTYVPAQEKNFTTAPAICHDGKAHFPREGVFVSNGTHWFVTQRNFYEPQIITTDNTFVSGNCDVVIGIVNNTVYDPLQPELDSFKEELDKYFKNHTSPDVDLGDISGINASVVNIQKEIDRLNEVAKNLNESLIDLQELGKYEQYIKRSNGLPGPIGPPGPRGRTGDAGPVGPPGPPGPPGPPGPPSAGFDFSFLPQPPQEKAHDGGRYYRANDANVVRDRDLEVDTTLKSLSQQIENIRSPEGSRKNPARTCRDLKMCHSDWKSGEYWIDPNQGCNLDAIKVFCNMETGETCVYPTQPSVAQKNWYISKNPKDKRHVWFGESMTDGFQFEYGGQGSDPADVAIQLTFLRLMSTEASQNITYHCKNSVAYMDQQTGNLKKALLLQGSNEIEIRAEGNSRFTYSVTVDGCTSHTGAWGKTVIEYKTTKTSRLPIIDVAPLDVGAPDQEFGFDVGPVCFL

SEQ ID NO: 93 - protein, 1195 aa, synthetic construct
  source 1..1195: note; note (original language) = SARS-CoV-2 Beta spike protein extracellular domain without signal peptide; organism (original language) = Synthetic construct
QCVNFTTRTQLPPAYTNSFTRGVYYPDKVFRSSVLHSTQDLFLPFFSNVTWFHAIHVSGTNGTKRFANPVLPFNDGVYFASTEKSNIIRGWIFGTTLDSKTQSLLIVNNATNVVIKVCEFQFCNDPFLGVYYHKNNKSWMESEFRVYSSANNCTFEYVSQPFLMDLEGKQGNFKNLREFVFKNIDGYFKIYSKHTPINLVRGLPQGFSALEPLVDLPIGINITRFQTLHISYLTPGDSSSGWTAGAAAYYVGYLQPRTFLLKYNENGTITDAVDCALDPLSETKCTLKSFTVEKGIYQTSNFRVQPTESIVRFPNITNLCPFGEVFNATRFASVYAWNRKRISNCVADYSVLYNSASFSTFKCYGVSPTKLNDLCFTNVYADSFVIRGDEVRQIAPGQTGNIADYNYKLPDDFTGCVIAWNSNNLDSKVGGNYNYLYRLFRKSNLKPFERDISTEIYQAGSTPCNGVKGFNCYFPLQSYGFQPTYGVGYQPYRVVVLSFELLHAPATVCGPKKSTNLVKNKCVNFNFNGLTGTGVLTESNKKFLPFQQFGRDIADTTDAVRDPQTLEILDITPCSFGGVSVITPGTNTSNQVAVLYQGVNCTEVPVAIHADQLTPTWRVYSTGSNVFQTRAGCLIGAEHVNNSYECDIPIGAGICASYQTQTNSPRRARSVASQSIIAYTMSLGVENSVAYSNNSIAIPTNFTISVTTEILPVSMTKTSVDCTMYICGDSTECSNLLLQYGSFCTQLNRALTGIAVEQDKNTQEVFAQVKQIYKTPPIKDFGGFNFSQILPDPSKPSKRSFIEDLLFNKVTLADAGFIKQYGDCLGDIAARDLICAQKFNGLTVLPPLLTDEMIAQYTSALLAGTITSGWTFGAGAALQIPFAMQMAYRFNGIGVTQNVLYENQKLIANQFNSAIGKIQDSLSSTASALGKLQDVVNQNAQALNTLVKQLSSNFGAISSVLNDILSRLDKVEAEVQIDRLITGRLQSLQTYVTQQLIRAAEIRASANLAATKMSECVLGQSKRVDFCGKGYHLMSFPQSAPHGVVFLHVTYVPAQEKNFTTAPAICHDGKAHFPREGVFVSNGTHWFVTQRNFYEPQIITTDNTFVSGNCDVVIGIVNNTVYDPLQPELDSFKEELDKYFKNHTSPDVDLGDISGINASVVNIQKEIDRLNEVAKNLNESLIDLQELGKYEQYIK

SEQ ID NO: 94 - protein, 1195 aa, synthetic construct
  source 1..1195: note; note (original language) = SARS-CoV-2 Beta spike protein extracellular domain without signal peptide, S1/S2 furin cleavage site 1 mutant (685R→685A); organism (original language) = Synthetic construct
QCVNFTTRTQLPPAYTNSFTRGVYYPDKVFRSSVLHSTQDLFLPFFSNVTWFHAIHVSGTNGTKRFANPVLPFNDGVYFASTEKSNIIRGWIFGTTLDSKTQSLLIVNNATNVVIKVCEFQFCNDPFLGVYYHKNNKSWMESEFRVYSSANNCTFEYVSQPFLMDLEGKQGNFKNLREFVFKNIDGYFKIYSKHTPINLVRGLPQGFSALEPLVDLPIGINITRFQTLHISYLTPGDSSSGWTAGAAAYYVGYLQPRTFLLKYNENGTITDAVDCALDPLSETKCTLKSFTVEKGIYQTSNFRVQPTESIVRFPNITNLCPFGEVFNATRFASVYAWNRKRISNCVADYSVLYNSASFSTFKCYGVSPTKLNDLCFTNVYADSFVIRGDEVRQIAPGQTGNIADYNYKLPDDFTGCVIAWNSNNLDSKVGGNYNYLYRLFRKSNLKPFERDISTEIYQAGSTPCNGVKGFNCYFPLQSYGFQPTYGVGYQPYRVVVLSFELLHAPATVCGPKKSTNLVKNKCVNFNFNGLTGTGVLTESNKKFLPFQQFGRDIADTTDAVRDPQTLEILDITPCSFGGVSVITPGTNTSNQVAVLYQGVNCTEVPVAIHADQLTPTWRVYSTGSNVFQTRAGCLIGAEHVNNSYECDIPIGAGICASYQTQTNSPRRAASVASQSIIAYTMSLGVENSVAYSNNSIAIPTNFTISVTTEILPVSMTKTSVDCTMYICGDSTECSNLLLQYGSFCTQLNRALTGIAVEQDKNTQEVFAQVKQIYKTPPIKDFGGFNFSQILPDPSKPSKRSFIEDLLFNKVTLADAGFIKQYGDCLGDIAARDLICAQKFNGLTVLPPLLTDEMIAQYTSALLAGTITSGWTFGAGAALQIPFAMQMAYRFNGIGVTQNVLYENQKLIANQFNSAIGKIQDSLSSTASALGKLQDVVNQNAQALNTLVKQLSSNFGAISSVLNDILSRLDKVEAEVQIDRLITGRLQSLQTYVTQQLIRAAEIRASANLAATKMSECVLGQSKRVDFCGKGYHLMSFPQSAPHGVVFLHVTYVPAQEKNFTTAPAICHDGKAHFPREGVFVSNGTHWFVTQRNFYEPQIITTDNTFVSGNCDVVIGIVNNTVYDPLQPELDSFKEELDKYFKNHTSPDVDLGDISGINASVVNIQKEIDRLNEVAKNLNESLIDLQELGKYEQYIK

SEQ ID NO: 95 - protein, 1195 aa, synthetic construct
  source 1..1195: note; note (original language) = SARS-CoV-2 Beta spike protein extracellular domain without signal peptide, S1/S2 furin cleavage site 1 and proline mutant (685R→685A, 986K/987V→986P/987P); organism (original language) = Synthetic construct
QCVNFTTRTQLPPAYTNSFTRGVYYPDKVFRSSVLHSTQDLFLPFFSNVTWFHAIHVSGTNGTKRFANPVLPFNDGVYFASTEKSNIIRGWIFGTTLDSKTQSLLIVNNATNVVIKVCEFQFCNDPFLGVYYHKNNKSWMESEFRVYSSANNCTFEYVSQPFLMDLEGKQGNFKNLREFVFKNIDGYFKIYSKHTPINLVRGLPQGFSALEPLVDLPIGINITRFQTLHISYLTPGDSSSGWTAGAAAYYVGYLQPRTFLLKYNENGTITDAVDCALDPLSETKCTLKSFTVEKGIYQTSNFRVQPTESIVRFPNITNLCPFGEVFNATRFASVYAWNRKRISNCVADYSVLYNSASFSTFKCYGVSPTKLNDLCFTNVYADSFVIRGDEVRQIAPGQTGNIADYNYKLPDDFTGCVIAWNSNNLDSKVGGNYNYLYRLFRKSNLKPFERDISTEIYQAGSTPCNGVKGFNCYFPLQSYGFQPTYGVGYQPYRVVVLSFELLHAPATVCGPKKSTNLVKNKCVNFNFNGLTGTGVLTESNKKFLPFQQFGRDIADTTDAVRDPQTLEILDITPCSFGGVSVITPGTNTSNQVAVLYQGVNCTEVPVAIHADQLTPTWRVYSTGSNVFQTRAGCLIGAEHVNNSYECDIPIGAGICASYQTQTNSPRRAASVASQSIIAYTMSLGVENSVAYSNNSIAIPTNFTISVTTEILPVSMTKTSVDCTMYICGDSTECSNLLLQYGSFCTQLNRALTGIAVEQDKNTQEVFAQVKQIYKTPPIKDFGGFNFSQILPDPSKPSKRSFIEDLLFNKVTLADAGFIKQYGDCLGDIAARDLICAQKFNGLTVLPPLLTDEMIAQYTSALLAGTITSGWTFGAGAALQIPFAMQMAYRFNGIGVTQNVLYENQKLIANQFNSAIGKIQDSLSSTASALGKLQDVVNQNAQALNTLVKQLSSNFGAISSVLNDILSRLDPPEAEVQIDRLITGRLQSLQTYVTQQLIRAAEIRASANLAATKMSECVLGQSKRVDFCGKGYHLMSFPQSAPHGVVFLHVTYVPAQEKNFTTAPAICHDGKAHFPREGVFVSNGTHWFVTQRNFYEPQIITTDNTFVSGNCDVVIGIVNNTVYDPLQPELDSFKEELDKYFKNHTSPDVDLGDISGINASVVNIQKEIDRLNEVAKNLNESLIDLQELGKYEQYIK

SEQ ID NO: 96 - protein, 1195 aa, synthetic construct
  source 1..1195: note; note (original language) = SARS-CoV-2 Beta spike protein extracellular domain without signal peptide, proline mutant (986K/987V→986P/987P); organism (original language) = Synthetic construct
QCVNFTTRTQLPPAYTNSFTRGVYYPDKVFRSSVLHSTQDLFLPFFSNVTWFHAIHVSGTNGTKRFANPVLPFNDGVYFASTEKSNIIRGWIFGTTLDSKTQSLLIVNNATNVVIKVCEFQFCNDPFLGVYYHKNNKSWMESEFRVYSSANNCTFEYVSQPFLMDLEGKQGNFKNLREFVFKNIDGYFKIYSKHTPINLVRGLPQGFSALEPLVDLPIGINITRFQTLHISYLTPGDSSSGWTAGAAAYYVGYLQPRTFLLKYNENGTITDAVDCALDPLSETKCTLKSFTVEKGIYQTSNFRVQPTESIVRFPNITNLCPFGEVFNATRFASVYAWNRKRISNCVADYSVLYNSASFSTFKCYGVSPTKLNDLCFTNVYADSFVIRGDEVRQIAPGQTGNIADYNYKLPDDFTGCVIAWNSNNLDSKVGGNYNYLYRLFRKSNLKPFERDISTEIYQAGSTPCNGVKGFNCYFPLQSYGFQPTYGVGYQPYRVVVLSFELLHAPATVCGPKKSTNLVKNKCVNFNFNGLTGTGVLTESNKKFLPFQQFGRDIADTTDAVRDPQTLEILDITPCSFGGVSVITPGTNTSNQVAVLYQGVNCTEVPVAIHADQLTPTWRVYSTGSNVFQTRAGCLIGAEHVNNSYECDIPIGAGICASYQTQTNSPRRARSVASQSIIAYTMSLGVENSVAYSNNSIAIPTNFTISVTTEILPVSMTKTSVDCTMYICGDSTECSNLLLQYGSFCTQLNRALTGIAVEQDKNTQEVFAQVKQIYKTPPIKDFGGFNFSQILPDPSKPSKRSFIEDLLFNKVTLADAGFIKQYGDCLGDIAARDLICAQKFNGLTVLPPLLTDEMIAQYTSALLAGTITSGWTFGAGAALQIPFAMQMAYRFNGIGVTQNVLYENQKLIANQFNSAIGKIQDSLSSTASALGKLQDVVNQNAQALNTLVKQLSSNFGAISSVLNDILSRLDPPEAEVQIDRLITGRLQSLQTYVTQQLIRAAEIRASANLAATKMSECVLGQSKRVDFCGKGYHLMSFPQSAPHGVVFLHVTYVPAQEKNFTTAPAICHDGKAHFPREGVFVSNGTHWFVTQRNFYEPQIITTDNTFVSGNCDVVIGIVNNTVYDPLQPELDSFKEELDKYFKNHTSPDVDLGDISGINASVVNIQKEIDRLNEVAKNLNESLIDLQELGKYEQYIK

SEQ ID NO: 97 - protein, 1198 aa, synthetic construct
  source 1..1198: note; note (original language) = Chimeric prototype (Hu-1) spike protein extracellular domain containing SARS-CoV-2 Beta (South African) variant RBD without signal peptide, S1/S2 furin cleavage site 1 and proline mutant (685R→685A, 986K/987V→986P/987P); organism (original language) = Synthetic construct
QCVNLTTRTQLPPAYTNSFTRGVYYPDKVFRSSVLHSTQDLFLPFFSNVTWFHAIHVSGTNGTKRFDNPVLPFNDGVYFASTEKSNIIRGWIFGTTLDSKTQSLLIVNNATNVVIKVCEFQFCNDPFLGVYYHKNNKSWMESEFRVYSSANNCTFEYVSQPFLMDLEGKQGNFKNLREFVFKNIDGYFKIYSKHTPINLVRDLPQGFSALEPLVDLPIGINITRFQTLLALHRSYLTPGDSSSGWTAGAAAYYVGYLQPRTFLLKYNENGTITDAVDCALDPLSETKCTLKSFTVEKGIYQTSNFRVQPTESIVRFPNITNLCPFGEVFNATRFASVYAWNRKRISNCVADYSVLYNSASFSTFKCYGVSPTKLNDLCFTNVYADSFVIRGDEVRQIAPGQTGNIADYNYKLPDDFTGCVIAWNSNNLDSKVGGNYNYLYRLFRKSNLKPFERDISTEIYQAGSTPCNGVKGFNCYFPLQSYGFQPTYGVGYQPYRVVVLSFELLHAPATVCGPKKSTNLVKNKCVNFNFNGLTGTGVLTESNKKFLPFQQFGRDIADTTDAVRDPQTLEILDITPCSFGGVSVITPGTNTSNQVAVLYQGVNCTEVPVAIHADQLTPTWRVYSTGSNVFQTRAGCLIGAEHVNNSYECDIPIGAGICASYQTQTNSPRRAASVASQSIIAYTMSLGAENSVAYSNNSIAIPTNFTISVTTEILPVSMTKTSVDCTMYICGDSTECSNLLLQYGSFCTQLNRALTGIAVEQDKNTQEVFAQVKQIYKTPPIKDFGGFNFSQILPDPSKPSKRSFIEDLLFNKVTLADAGFIKQYGDCLGDIAARDLICAQKFNGLTVLPPLLTDEMIAQYTSALLAGTITSGWTFGAGAALQIPFAMQMAYRFNGIGVTQNVLYENQKLIANQFNSAIGKIQDSLSSTASALGKLQDVVNQNAQALNTLVKQLSSNFGAISSVLNDILSRLDPPEAEVQIDRLITGRLQSLQTYVTQQLIRAAEIRASANLAATKMSECVLGQSKRVDFCGKGYHLMSFPQSAPHGVVFLHVTYVPAQEKNFTTAPAICHDGKAHFPREGVFVSNGTHWFVTQRNFYEPQIITTDNTFVSGNCDVVIGIVNNTVYDPLQPELDSFKEELDKYFKNHTSPDVDLGDISGINASVVNIQKEIDRLNEVAKNLNESLIDLQELGKYEQYIK

SEQ ID NO: 98 - protein, 1506 aa, synthetic construct
  source 1..1506: note; note (original language) = SARS-CoV-2 Beta S-trimer fusion polypeptide without signal peptide; organism (original language) = Synthetic construct
QCVNFTTRTQLPPAYTNSFTRGVYYPDKVFRSSVLHSTQDLFLPFFSNVTWFHAIHVSGTNGTKRFANPVLPFNDGVYFASTEKSNIIRGWIFGTTLDSKTQSLLIVNNATNVVIKVCEFQFCNDPFLGVYYHKNNKSWMESEFRVYSSANNCTFEYVSQPFLMDLEGKQGNFKNLREFVFKNIDGYFKIYSKHTPINLVRGLPQGFSALEPLVDLPIGINITRFQTLHISYLTPGDSSSGWTAGAAAYYVGYLQPRTFLLKYNENGTITDAVDCALDPLSETKCTLKSFTVEKGIYQTSNFRVQPTESIVRFPNITNLCPFGEVFNATRFASVYAWNRKRISNCVADYSVLYNSASFSTFKCYGVSPTKLNDLCFTNVYADSFVIRGDEVRQIAPGQTGNIADYNYKLPDDFTGCVIAWNSNNLDSKVGGNYNYLYRLFRKSNLKPFERDISTEIYQAGSTPCNGVKGFNCYFPLQSYGFQPTYGVGYQPYRVVVLSFELLHAPATVCGPKKSTNLVKNKCVNFNFNGLTGTGVLTESNKKFLPFQQFGRDIADTTDAVRDPQTLEILDITPCSFGGVSVITPGTNTSNQVAVLYQGVNCTEVPVAIHADQLTPTWRVYSTGSNVFQTRAGCLIGAEHVNNSYECDIPIGAGICASYQTQTNSPRRARSVASQSIIAYTMSLGVENSVAYSNNSIAIPTNFTISVTTEILPVSMTKTSVDCTMYICGDSTECSNLLLQYGSFCTQLNRALTGIAVEQDKNTQEVFAQVKQIYKTPPIKDFGGFNFSQILPDPSKPSKRSFIEDLLFNKVTLADAGFIKQYGDCLGDIAARDLICAQKFNGLTVLPPLLTDEMIAQYTSALLAGTITSGWTFGAGAALQIPFAMQMAYRFNGIGVTQNVLYENQKLIANQFNSAIGKIQDSLSSTASALGKLQDVVNQNAQALNTLVKQLSSNFGAISSVLNDILSRLDKVEAEVQIDRLITGRLQSLQTYVTQQLIRAAEIRASANLAATKMSECVLGQSKRVDFCGKGYHLMSFPQSAPHGVVFLHVTYVPAQEKNFTTAPAICHDGKAHFPREGVFVSNGTHWFVTQRNFYEPQIITTDNTFVSGNCDVVIGIVNNTVYDPLQPELDSFKEELDKYFKNHTSPDVDLGDISGINASVVNIQKEIDRLNEVAKNLNESLIDLQELGKYEQYIKRSNGLPGPIGPPGPRGRTGDAGPVGPPGPPGPPGPPGPPSAGFDFSFLPQPPQEKAHDGGRYYRANDANVVRDRDLEVDTTLKSLSQQIENIRSPEGSRKNPARTCRDLKMCHSDWKSGEYWIDPNQGCNLDAIKVFCNMETGETCVYPTQPSVAQKNWYISKNPKDKRHVWFGESMTDGFQFEYGGQGSDPADVAIQLTFLRLMSTEASQNITYHCKNSVAYMDQQTGNLKKALLLQGSNEIEIRAEGNSRFTYSVTVDGCTSHTGAWGKTVIEYKTTKTSRLPIIDVAPLDVGAPDQEFGFDVGPVCFL

SEQ ID NO: 99 - protein, 1506 aa, synthetic construct
  source 1..1506: note; note (original language) = SARS-CoV-2 Beta S-trimer fusion polypeptide without signal peptide, S1/S2 furin cleavage site 1 mutant (685R→685A); organism (original language) = Synthetic construct
QCVNFTTRTQLPPAYTNSFTRGVYYPDKVFRSSVLHSTQDLFLPFFSNVTWFHAIHVSGTNGTKRFANPVLPFNDGVYFASTEKSNIIRGWIFGTTLDSKTQSLLIVNNATNVVIKVCEFQFCNDPFLGVYYHKNNKSWMESEFRVYSSANNCTFEYVSQPFLMDLEGKQGNFKNLREFVFKNIDGYFKIYSKHTPINLVRGLPQGFSALEPLVDLPIGINITRFQTLHISYLTPGDSSSGWTAGAAAYYVGYLQPRTFLLKYNENGTITDAVDCALDPLSETKCTLKSFTVEKGIYQTSNFRVQPTESIVRFPNITNLCPFGEVFNATRFASVYAWNRKRISNCVADYSVLYNSASFSTFKCYGVSPTKLNDLCFTNVYADSFVIRGDEVRQIAPGQTGNIADYNYKLPDDFTGCVIAWNSNNLDSKVGGNYNYLYRLFRKSNLKPFERDISTEIYQAGSTPCNGVKGFNCYFPLQSYGFQPTYGVGYQPYRVVVLSFELLHAPATVCGPKKSTNLVKNKCVNFNFNGLTGTGVLTESNKKFLPFQQFGRDIADTTDAVRDPQTLEILDITPCSFGGVSVITPGTNTSNQVAVLYQGVNCTEVPVAIHADQLTPTWRVYSTGSNVFQTRAGCLIGAEHVNNSYECDIPIGAGICASYQTQTNSPRRAASVASQSIIAYTMSLGVENSVAYSNNSIAIPTNFTISVTTEILPVSMTKTSVDCTMYICGDSTECSNLLLQYGSFCTQLNRALTGIAVEQDKNTQEVFAQVKQIYKTPPIKDFGGFNFSQILPDPSKPSKRSFIEDLLFNKVTLADAGFIKQYGDCLGDIAARDLICAQKFNGLTVLPPLLTDEMIAQYTSALLAGTITSGWTFGAGAALQIPFAMQMAYRFNGIGVTQNVLYENQKLIANQFNSAIGKIQDSLSSTASALGKLQDVVNQNAQALNTLVKQLSSNFGAISSVLNDILSRLDKVEAEVQIDRLITGRLQSLQTYVTQQLIRAAEIRASANLAATKMSECVLGQSKRVDFCGKGYHLMSFPQSAPHGVVFLHVTYVPAQEKNFTTAPAICHDGKAHFPREGVFVSNGTHWFVTQRNFYEPQIITTDNTFVSGNCDVVIGIVNNTVYDPLQPELDSFKEELDKYFKNHTSPDVDLGDISGINASVVNIQKEIDRLNEVAKNLNESLIDLQELGKYEQYIKRSNGLPGPIGPPGPRGRTGDAGPVGPPGPPGPPGPPGPPSAGFDFSFLPQPPQEKAHDGGRYYRANDANVVRDRDLEVDTTLKSLSQQIENIRSPEGSRKNPARTCRDLKMCHSDWKSGEYWIDPNQGCNLDAIKVFCNMETGETCVYPTQPSVAQKNWYISKNPKDKRHVWFGESMTDGFQFEYGGQGSDPADVAIQLTFLRLMSTEASQNITYHCKNSVAYMDQQTGNLKKALLLQGSNEIEIRAEGNSRFTYSVTVDGCTSHTGAWGKTVIEYKTTKTSRLPIIDVAPLDVGAPDQEFGFDVGPVCFL

SEQ ID NO: 100 - protein, 1506 aa, synthetic construct
  source 1..1506: note; note (original language) = SARS-CoV-2 Beta S-trimer fusion polypeptide without signal peptide, S1/S2 furin cleavage site 1 and proline mutant (685R→685A, 986K/987V→986P/987P); organism (original language) = Synthetic construct
QCVNFTTRTQLPPAYTNSFTRGVYYPDKVFRSSVLHSTQDLFLPFFSNVTWFHAIHVSGTNGTKRFANPVLPFNDGVYFASTEKSNIIRGWIFGTTLDSKTQSLLIVNNATNVVIKVCEFQFCNDPFLGVYYHKNNKSWMESEFRVYSSANNCTFEYVSQPFLMDLEGKQGNFKNLREFVFKNIDGYFKIYSKHTPINLVRGLPQGFSALEPLVDLPIGINITRFQTLHISYLTPGDSSSGWTAGAAAYYVGYLQPRTFLLKYNENGTITDAVDCALDPLSETKCTLKSFTVEKGIYQTSNFRVQPTESIVRFPNITNLCPFGEVFNATRFASVYAWNRKRISNCVADYSVLYNSASFSTFKCYGVSPTKLNDLCFTNVYADSFVIRGDEVRQIAPGQTGNIADYNYKLPDDFTGCVIAWNSNNLDSKVGGNYNYLYRLFRKSNLKPFERDISTEIYQAGSTPCNGVKGFNCYFPLQSYGFQPTYGVGYQPYRVVVLSFELLHAPATVCGPKKSTNLVKNKCVNFNFNGLTGTGVLTESNKKFLPFQQFGRDIADTTDAVRDPQTLEILDITPCSFGGVSVITPGTNTSNQVAVLYQGVNCTEVPVAIHADQLTPTWRVYSTGSNVFQTRAGCLIGAEHVNNSYECDIPIGAGICASYQTQTNSPRRAASVASQSIIAYTMSLGVENSVAYSNNSIAIPTNFTISVTTEILPVSMTKTSVDCTMYICGDSTECSNLLLQYGSFCTQLNRALTGIAVEQDKNTQEVFAQVKQIYKTPPIKDFGGFNFSQILPDPSKPSKRSFIEDLLFNKVTLADAGFIKQYGDCLGDIAARDLICAQKFNGLTVLPPLLTDEMIAQYTSALLAGTITSGWTFGAGAALQIPFAMQMAYRFNGIGVTQNVLYENQKLIANQFNSAIGKIQDSLSSTASALGKLQDVVNQNAQALNTLVKQLSSNFGAISSVLNDILSRLDPPEAEVQIDRLITGRLQSLQTYVTQQLIRAAEIRASANLAATKMSECVLGQSKRVDFCGKGYHLMSFPQSAPHGVVFLHVTYVPAQEKNFTTAPAICHDGKAHFPREGVFVSNGTHWFVTQRNFYEPQIITTDNTFVSGNCDVVIGIVNNTVYDPLQPELDSFKEELDKYFKNHTSPDVDLGDISGINASVVNIQKEIDRLNEVAKNLNESLIDLQELGKYEQYIKRSNGLPGPIGPPGPRGRTGDAGPVGPPGPPGPPGPPGPPSAGFDFSFLPQPPQEKAHDGGRYYRANDANVVRDRDLEVDTTLKSLSQQIENIRSPEGSRKNPARTCRDLKMCHSDWKSGEYWIDPNQGCNLDAIKVFCNMETGETCVYPTQPSVAQKNWYISKNPKDKRHVWFGESMTDGFQFEYGGQGSDPADVAIQLTFLRLMSTEASQNITYHCKNSVAYMDQQTGNLKKALLLQGSNEIEIRAEGNSRFTYSVTVDGCTSHTGAWGKTVIEYKTTKTSRLPIIDVAPLDVGAPDQEFGFDVGPVCFL

SEQ ID NO: 101 - protein, 1506 aa, synthetic construct
  source 1..1506: note; note (original language) = SARS-CoV-2 Beta S-trimer fusion polypeptide without signal peptide, proline mutant (986K/987V→986P/987P); organism (original language) = Synthetic construct
QCVNFTTRTQLPPAYTNSFTRGVYYPDKVFRSSVLHSTQDLFLPFFSNVTWFHAIHVSGTNGTKRFANPVLPFNDGVYFASTEKSNIIRGWIFGTTLDSKTQSLLIVNNATNVVIKVCEFQFCNDPFLGVYYHKNNKSWMESEFRVYSSANNCTFEYVSQPFLMDLEGKQGNFKNLREFVFKNIDGYFKIYSKHTPINLVRGLPQGFSALEPLVDLPIGINITRFQTLHISYLTPGDSSSGWTAGAAAYYVGYLQPRTFLLKYNENGTITDAVDCALDPLSETKCTLKSFTVEKGIYQTSNFRVQPTESIVRFPNITNLCPFGEVFNATRFASVYAWNRKRISNCVADYSVLYNSASFSTFKCYGVSPTKLNDLCFTNVYADSFVIRGDEVRQIAPGQTGNIADYNYKLPDDFTGCVIAWNSNNLDSKVGGNYNYLYRLFRKSNLKPFERDISTEIYQAGSTPCNGVKGFNCYFPLQSYGFQPTYGVGYQPYRVVVLSFELLHAPATVCGPKKSTNLVKNKCVNFNFNGLTGTGVLTESNKKFLPFQQFGRDIADTTDAVRDPQTLEILDITPCSFGGVSVITPGTNTSNQVAVLYQGVNCTEVPVAIHADQLTPTWRVYSTGSNVFQTRAGCLIGAEHVNNSYECDIPIGAGICASYQTQTNSPRRARSVASQSIIAYTMSLGVENSVAYSNNSIAIPTNFTISVTTEILPVSMTKTSVDCTMYICGDSTECSNLLLQYGSFCTQLNRALTGIAVEQDKNTQEVFAQVKQIYKTPPIKDFGGFNFSQILPDPSKPSKRSFIEDLLFNKVTLADAGFIKQYGDCLGDIAARDLICAQKFNGLTVLPPLLTDEMIAQYTSALLAGTITSGWTFGAGAALQIPFAMQMAYRFNGIGVTQNVLYENQKLIANQFNSAIGKIQDSLSSTASALGKLQDVVNQNAQALNTLVKQLSSNFGAISSVLNDILSRLDPPEAEVQIDRLITGRLQSLQTYVTQQLIRAAEIRASANLAATKMSECVLGQSKRVDFCGKGYHLMSFPQSAPHGVVFLHVTYVPAQEKNFTTAPAICHDGKAHFPREGVFVSNGTHWFVTQRNFYEPQIITTDNTFVSGNCDVVIGIVNNTVYDPLQPELDSFKEELDKYFKNHTSPDVDLGDISGINASVVNIQKEIDRLNEVAKNLNESLIDLQELGKYEQYIKRSNGLPGPIGPPGPRGRTGDAGPVGPPGPPGPPGPPGPPSAGFDFSFLPQPPQEKAHDGGRYYRANDANVVRDRDLEVDTTLKSLSQQIENIRSPEGSRKNPARTCRDLKMCHSDWKSGEYWIDPNQGCNLDAIKVFCNMETGETCVYPTQPSVAQKNWYISKNPKDKRHVWFGESMTDGFQFEYGGQGSDPADVAIQLTFLRLMSTEASQNITYHCKNSVAYMDQQTGNLKKALLLQGSNEIEIRAEGNSRFTYSVTVDGCTSHTGAWGKTVIEYKTTKTSRLPIIDVAPLDVGAPDQEFGFDVGPVCFL

SEQ ID NO: 102 - protein, 1509 aa, synthetic construct; identical to SEQ ID NO: 13
  source 1..1509: note; note (original language) = Chimeric prototype (Hu-1) S-trimer fusion polypeptide containing SARS-CoV-2 Beta (South African) variant RBD without signal peptide, S1/S2 furin cleavage site 1 and proline mutants (685R→685A, 986K/987V→986P/987P); organism (original language) = Synthetic construct

SEQ ID NO: 103 - protein, 1519 aa, synthetic construct
  source 1..1519: note; note (original language) = SARS-CoV-2 Beta S-trimer fusion polypeptide with signal peptide; organism (original language) = Synthetic construct
MFVFLVLLPLVSSQCVNFTTRTQLPPAYTNSFTRGVYYPDKVFRSSVLHSTQDLFLPFFSNVTWFHAIHVSGTNGTKRFANPVLPFNDGVYFASTEKSNIIRGWIFGTTLDSKTQSLLIVNNATNVVIKVCEFQFCNDPFLGVYYHKNNKSWMESEFRVYSSANNCTFEYVSQPFLMDLEGKQGNFKNLREFVFKNIDGYFKIYSKHTPINLVRGLPQGFSALEPLVDLPIGINITRFQTLHISYLTPGDSSSGWTAGAAAYYVGYLQPRTFLLKYNENGTITDAVDCALDPLSETKCTLKSFTVEKGIYQTSNFRVQPTESIVRFPNITNLCPFGEVFNATRFASVYAWNRKRISNCVADYSVLYNSASFSTFKCYGVSPTKLNDLCFTNVYADSFVIRGDEVRQIAPGQTGNIADYNYKLPDDFTGCVIAWNSNNLDSKVGGNYNYLYRLFRKSNLKPFERDISTEIYQAGSTPCNGVKGFNCYFPLQSYGFQPTYGVGYQPYRVVVLSFELLHAPATVCGPKKSTNLVKNKCVNFNFNGLTGTGVLTESNKKFLPFQQFGRDIADTTDAVRDPQTLEILDITPCSFGGVSVITPGTNTSNQVAVLYQGVNCTEVPVAIHADQLTPTWRVYSTGSNVFQTRAGCLIGAEHVNNSYECDIPIGAGICASYQTQTNSPRRARSVASQSIIAYTMSLGVENSVAYSNNSIAIPTNFTISVTTEILPVSMTKTSVDCTMYICGDSTECSNLLLQYGSFCTQLNRALTGIAVEQDKNTQEVFAQVKQIYKTPPIKDFGGFNFSQILPDPSKPSKRSFIEDLLFNKVTLADAGFIKQYGDCLGDIAARDLICAQKFNGLTVLPPLLTDEMIAQYTSALLAGTITSGWTFGAGAALQIPFAMQMAYRFNGIGVTQNVLYENQKLIANQFNSAIGKIQDSLSSTASALGKLQDVVNQNAQALNTLVKQLSSNFGAISSVLNDILSRLDKVEAEVQIDRLITGRLQSLQTYVTQQLIRAAEIRASANLAATKMSECVLGQSKRVDFCGKGYHLMSFPQSAPHGVVFLHVTYVPAQEKNFTTAPAICHDGKAHFPREGVFVSNGTHWFVTQRNFYEPQIITTDNTFVSGNCDVVIGIVNNTVYDPLQPELDSFKEELDKYFKNHTSPDVDLGDISGINASVVNIQKEIDRLNEVAKNLNESLIDLQELGKYEQYIKRSNGLPGPIGPPGPRGRTGDAGPVGPPGPPGPPGPPGPPSAGFDFSFLPQPPQEKAHDGGRYYRANDANVVRDRDLEVDTTLKSLSQQIENIRSPEGSRKNPARTCRDLKMCHSDWKSGEYWIDPNQGCNLDAIKVFCNMETGETCVYPTQPSVAQKNWYISKNPKDKRHVWFGESMTDGFQFEYGGQGSDPADVAIQLTFLRLMSTEASQNITYHCKNSVAYMDQQTGNLKKALLLQGSNEIEIRAEGNSRFTYSVTVDGCTSHTGAWGKTVIEYKTTKTSRLPIIDVAPLDVGAPDQEFGFDVGPVCFL

SEQ ID NO: 104 - protein, 1519 aa, synthetic construct
  source 1..1519: note; note (original language) = SARS-CoV-2 Beta S-trimer fusion polypeptide with signal peptide, S1/S2 furin cleavage site 1 mutant (685R→685A); organism (original language) = Synthetic construct
MFVFLVLLPLVSSQCVNFTTRTQLPPAYTNSFTRGVYYPDKVFRSSVLHSTQDLFLPFFSNVTWFHAIHVSGTNGTKRFANPVLPFNDGVYFASTEKSNIIRGWIFGTTLDSKTQSLLIVNNATNVVIKVCEFQFCNDPFLGVYYHKNNKSWMESEFRVYSSANNCTFEYVSQPFLMDLEGKQGNFKNLREFVFKNIDGYFKIYSKHTPINLVRGLPQGFSALEPLVDLPIGINITRFQTLHISYLTPGDSSSGWTAGAAAYYVGYLQPRTFLLKYNENGTITDAVDCALDPLSETKCTLKSFTVEKGIYQTSNFRVQPTESIVRFPNITNLCPFGEVFNATRFASVYAWNRKRISNCVADYSVLYNSASFSTFKCYGVSPTKLNDLCFTNVYADSFVIRGDEVRQIAPGQTGNIADYNYKLPDDFTGCVIAWNSNNLDSKVGGNYNYLYRLFRKSNLKPFERDISTEIYQAGSTPCNGVKGFNCYFPLQSYGFQPTYGVGYQPYRVVVLSFELLHAPATVCGPKKSTNLVKNKCVNFNFNGLTGTGVLTESNKKFLPFQQFGRDIADTTDAVRDPQTLEILDITPCSFGGVSVITPGTNTSNQVAVLYQGVNCTEVPVAIHADQLTPTWRVYSTGSNVFQTRAGCLIGAEHVNNSYECDIPIGAGICASYQTQTNSPRRAASVASQSIIAYTMSLGVENSVAYSNNSIAIPTNFTISVTTEILPVSMTKTSVDCTMYICGDSTECSNLLLQYGSFCTQLNRALTGIAVEQDKNTQEVFAQVKQIYKTPPIKDFGGFNFSQILPDPSKPSKRSFIEDLLFNKVTLADAGFIKQYGDCLGDIAARDLICAQKFNGLTVLPPLLTDEMIAQYTSALLAGTITSGWTFGAGAALQIPFAMQMAYRFNGIGVTQNVLYENQKLIANQFNSAIGKIQDSLSSTASALGKLQDVVNQNAQALNTLVKQLSSNFGAISSVLNDILSRLDKVEAEVQIDRLITGRLQSLQTYVTQQLIRAAEIRASANLAATKMSECVLGQSKRVDFCGKGYHLMSFPQSAPHGVVFLHVTYVPAQEKNFTTAPAICHDGKAHFPREGVFVSNGTHWFVTQRNFYEPQIITTDNTFVSGNCDVVIGIVNNTVYDPLQPELDSFKEELDKYFKNHTSPDVDLGDISGINASVVNIQKEIDRLNEVAKNLNESLIDLQELGKYEQYIKRSNGLPGPIGPPGPRGRTGDAGPVGPPGPPGPPGPPGPPSAGFDFSFLPQPPQEKAHDGGRYYRANDANVVRDRDLEVDTTLKSLSQQIENIRSPEGSRKNPARTCRDLKMCHSDWKSGEYWIDPNQGCNLDAIKVFCNMETGETCVYPTQPSVAQKNWYISKNPKDKRHVWFGESMTDGFQFEYGGQGSDPADVAIQLTFLRLMSTEASQNITYHCKNSVAYMDQQTGNLKKALLLQGSNEIEIRAEGNSRFTYSVTVDGCTSHTGAWGKTVIEYKTTKTSRLPIIDVAPLDVGAPDQEFGFDVGPVCFL

SEQ ID NO: 105 - protein, 1519 aa, synthetic construct
  source 1..1519: note; note (original language) = SARS-CoV-2 Beta S-trimer fusion polypeptide with signal peptide, S1/S2 furin cleavage site 1 and proline mutant (685R→685A, 986K/987V→986P/987P); organism (original language) = Synthetic construct
MFVFLVLLPLVSSQCVNFTTRTQLPPAYTNSFTRGVYYPDKVFRSSVLHSTQDLFLPFFSNVTWFHAIHVSGTNGTKRFANPVLPFNDGVYFASTEKSNIIRGWIFGTTLDSKTQSLLIVNNATNVVIKVCEFQFCNDPFLGVYYHKNNKSWMESEFRVYSSANNCTFEYVSQPFLMDLEGKQGNFKNLREFVFKNIDGYFKIYSKHTPINLVRGLPQGFSALEPLVDLPIGINITRFQTLHISYLTPGDSSSGWTAGAAAYYVGYLQPRTFLLKYNENGTITDAVDCALDPLSETKCTLKSFTVEKGIYQTSNFRVQPTESIVRFPNITNLCPFGEVFNATRFASVYAWNRKRISNCVADYSVLYNSASFSTFKCYGVSPTKLNDLCFTNVYADSFVIRGDEVRQIAPGQTGNIADYNYKLPDDFTGCVIAWNSNNLDSKVGGNYNYLYRLFRKSNLKPFERDISTEIYQAGSTPCNGVKGFNCYFPLQSYGFQPTYGVGYQPYRVVVLSFELLHAPATVCGPKKSTNLVKNKCVNFNFNGLTGTGVLTESNKKFLPFQQFGRDIADTTDAVRDPQTLEILDITPCSFGGVSVITPGTNTSNQVAVLYQGVNCTEVPVAIHADQLTPTWRVYSTGSNVFQTRAGCLIGAEHVNNSYECDIPIGAGICASYQTQTNSPRRAASVASQSIIAYTMSLGVENSVAYSNNSIAIPTNFTISVTTEILPVSMTKTSVDCTMYICGDSTECSNLLLQYGSFCTQLNRALTGIAVEQDKNTQEVFAQVKQIYKTPPIKDFGGFNFSQILPDPSKPSKRSFIEDLLFNKVTLADAGFIKQYGDCLGDIAARDLICAQKFNGLTVLPPLLTDEMIAQYTSALLAGTITSGWTFGAGAALQIPFAMQMAYRFNGIGVTQNVLYENQKLIANQFNSAIGKIQDSLSSTASALGKLQDVVNQNAQALNTLVKQLSSNFGAISSVLNDILSRLDPPEAEVQIDRLITGRLQSLQTYVTQQLIRAAEIRASANLAATKMSECVLGQSKRVDFCGKGYHLMSFPQSAPHGVVFLHVTYVPAQEKNFTTAPAICHDGKAHFPREGVFVSNGTHWFVTQRNFYEPQIITTDNTFVSGNCDVVIGIVNNTVYDPLQPELDSFKEELDKYFKNHTSPDVDLGDISGINASVVNIQKEIDRLNEVAKNLNESLIDLQELGKYEQYIKRSNGLPGPIGPPGPRGRTGDAGPVGPPGPPGPPGPPGPPSAGFDFSFLPQPPQEKAHDGGRYYRANDANVVRDRDLEVDTTLKSLSQQIENIRSPEGSRKNPARTCRDLKMCHSDWKSGEYWIDPNQGCNLDAIKVFCNMETGETCVYPTQPSVAQKNWYISKNPKDKRHVWFGESMTDGFQFEYGGQGSDPADVAIQLTFLRLMSTEASQNITYHCKNSVAYMDQQTGNLKKALLLQGSNEIEIRAEGNSRFTYSVTVDGCTSHTGAWGKTVIEYKTTKTSRLPIIDVAPLDVGAPDQEFGFDVGPVCFL

SEQ ID NO: 106 - protein, 1519 aa, synthetic construct
  source 1..1519: note; note (original language) = SARS-CoV-2 Beta S-trimer fusion polypeptide with signal peptide, proline mutant (986K/987V→986P/987P); organism (original language) = Synthetic construct
MFVFLVLLPLVSSQCVNFTTRTQLPPAYTNSFTRGVYYPDKVFRSSVLHSTQDLFLPFFSNVTWFHAIHVSGTNGTKRFANPVLPFNDGVYFASTEKSNIIRGWIFGTTLDSKTQSLLIVNNATNVVIKVCEFQFCNDPFLGVYYHKNNKSWMESEFRVYSSANNCTFEYVSQPFLMDLEGKQGNFKNLREFVFKNIDGYFKIYSKHTPINLVRGLPQGFSALEPLVDLPIGINITRFQTLHISYLTPGDSSSGWTAGAAAYYVGYLQPRTFLLKYNENGTITDAVDCALDPLSETKCTLKSFTVEKGIYQTSNFRVQPTESIVRFPNITNLCPFGEVFNATRFASVYAWNRKRISNCVADYSVLYNSASFSTFKCYGVSPTKLNDLCFTNVYADSFVIRGDEVRQIAPGQTGNIADYNYKLPDDFTGCVIAWNSNNLDSKVGGNYNYLYRLFRKSNLKPFERDISTEIYQAGSTPCNGVKGFNCYFPLQSYGFQPTYGVGYQPYRVVVLSFELLHAPATVCGPKKSTNLVKNKCVNFNFNGLTGTGVLTESNKKFLPFQQFGRDIADTTDAVRDPQTLEILDITPCSFGGVSVITPGTNTSNQVAVLYQGVNCTEVPVAIHADQLTPTWRVYSTGSNVFQTRAGCLIGAEHVNNSYECDIPIGAGICASYQTQTNSPRRARSVASQSIIAYTMSLGVENSVAYSNNSIAIPTNFTISVTTEILPVSMTKTSVDCTMYICGDSTECSNLLLQYGSFCTQLNRALTGIAVEQDKNTQEVFAQVKQIYKTPPIKDFGGFNFSQILPDPSKPSKRSFIEDLLFNKVTLADAGFIKQYGDCLGDIAARDLICAQKFNGLTVLPPLLTDEMIAQYTSALLAGTITSGWTFGAGAALQIPFAMQMAYRFNGIGVTQNVLYENQKLIANQFNSAIGKIQDSLSSTASALGKLQDVVNQNAQALNTLVKQLSSNFGAISSVLNDILSRLDPPEAEVQIDRLITGRLQSLQTYVTQQLIRAAEIRASANLAATKMSECVLGQSKRVDFCGKGYHLMSFPQSAPHGVVFLHVTYVPAQEKNFTTAPAICHDGKAHFPREGVFVSNGTHWFVTQRNFYEPQIITTDNTFVSGNCDVVIGIVNNTVYDPLQPELDSFKEELDKYFKNHTSPDVDLGDISGINASVVNIQKEIDRLNEVAKNLNESLIDLQELGKYEQYIKRSNGLPGPIGPPGPRGRTGDAGPVGPPGPPGPPGPPGPPSAGFDFSFLPQPPQEKAHDGGRYYRANDANVVRDRDLEVDTTLKSLSQQIENIRSPEGSRKNPARTCRDLKMCHSDWKSGEYWIDPNQGCNLDAIKVFCNMETGETCVYPTQPSVAQKNWYISKNPKDKRHVWFGESMTDGFQFEYGGQGSDPADVAIQLTFLRLMSTEASQNITYHCKNSVAYMDQQTGNLKKALLLQGSNEIEIRAEGNSRFTYSVTVDGCTSHTGAWGKTVIEYKTTKTSRLPIIDVAPLDVGAPDQEFGFDVGPVCFL

SEQ ID NO: 107 - protein, 1522 aa, synthetic construct
  source 1..1522: note; note (original language) = Chimeric prototype (Hu-1) S-trimer fusion polypeptide containing SARS-CoV-2 Beta (South African) variant RBD with signal peptide, S1/S2 furin cleavage site 1 and proline mutants (685R→685A, 986K/987V→986P/987P); organism (original language) = Synthetic construct
MFVFLVLLPLVSSQCVNLTTRTQLPPAYTNSFTRGVYYPDKVFRSSVLHSTQDLFLPFFSNVTWFHAIHVSGTNGTKRFDNPVLPFNDGVYFASTEKSNIIRGWIFGTTLDSKTQSLLIVNNATNVVIKVCEFQFCNDPFLGVYYHKNNKSWMESEFRVYSSANNCTFEYVSQPFLMDLEGKQGNFKNLREFVFKNIDGYFKIYSKHTPINLVRDLPQGFSALEPLVDLPIGINITRFQTLLALHRSYLTPGDSSSGWTAGAAAYYVGYLQPRTFLLKYNENGTITDAVDCALDPLSETKCTLKSFTVEKGIYQTSNFRVQPTESIVRFPNITNLCPFGEVFNATRFASVYAWNRKRISNCVADYSVLYNSASFSTFKCYGVSPTKLNDLCFTNVYADSFVIRGDEVRQIAPGQTGNIADYNYKLPDDFTGCVIAWNSNNLDSKVGGNYNYLYRLFRKSNLKPFERDISTEIYQAGSTPCNGVKGFNCYFPLQSYGFQPTYGVGYQPYRVVVLSFELLHAPATVCGPKKSTNLVKNKCVNFNFNGLTGTGVLTESNKKFLPFQQFGRDIADTTDAVRDPQTLEILDITPCSFGGVSVITPGTNTSNQVAVLYQGVNCTEVPVAIHADQLTPTWRVYSTGSNVFQTRAGCLIGAEHVNNSYECDIPIGAGICASYQTQTNSPRRAASVASQSIIAYTMSLGAENSVAYSNNSIAIPTNFTISVTTEILPVSMTKTSVDCTMYICGDSTECSNLLLQYGSFCTQLNRALTGIAVEQDKNTQEVFAQVKQIYKTPPIKDFGGFNFSQILPDPSKPSKRSFIEDLLFNKVTLADAGFIKQYGDCLGDIAARDLICAQKFNGLTVLPPLLTDEMIAQYTSALLAGTITSGWTFGAGAALQIPFAMQMAYRFNGIGVTQNVLYENQKLIANQFNSAIGKIQDSLSSTASALGKLQDVVNQNAQALNTLVKQLSSNFGAISSVLNDILSRLDPPEAEVQIDRLITGRLQSLQTYVTQQLIRAAEIRASANLAATKMSECVLGQSKRVDFCGKGYHLMSFPQSAPHGVVFLHVTYVPAQEKNFTTAPAICHDGKAHFPREGVFVSNGTHWFVTQRNFYEPQIITTDNTFVSGNCDVVIGIVNNTVYDPLQPELDSFKEELDKYFKNHTSPDVDLGDISGINASVVNIQKEIDRLNEVAKNLNESLIDLQELGKYEQYIKRSNGLPGPIGPPGPRGRTGDAGPVGPPGPPGPPGPPGPPSAGFDFSFLPQPPQEKAHDGGRYYRANDANVVRDRDLEVDTTLKSLSQQIENIRSPEGSRKNPARTCRDLKMCHSDWKSGEYWIDPNQGCNLDAIKVFCNMETGETCVYPTQPSVAQKNWYISKNPKDKRHVWFGESMTDGFQFEYGGQGSDPADVAIQLTFLRLMSTEASQNITYHCKNSVAYMDQQTGNLKKALLLQGSNEIEIRAEGNSRFTYSVTVDGCTSHTGAWGKTVIEYKTTKTSRLPIIDVAPLDVGAPDQEFGFDVGPVCFL

SEQ ID NO: 108 - protein, 1196 aa, synthetic construct
  source 1..1196: note; note (original language) = SARS-CoV-2 Delta spike protein extracellular domain without signal peptide; organism (original language) = Synthetic construct
QCVNLRTRTQLPPAYTNSFTRGVYYPDKVFRSSVLHSTQDLFLPFFSNVTWFHAIHVSGTNGTKRFDNPVLPFNDGVYFASTEKSNIIRGWIFGTTLDSKTQSLLIVNNATNVVIKVCEFQFCNDPFLDVYYHKNNKSWMESGVYSSANNCTFEYVSQPFLMDLEGKQGNFKNLREFVFKNIDGYFKIYSKHTPINLVRDLPQGFSALEPLVDLPIGINITRFQTLLALHRSYLTPGDSSSGWTAGAAAYYVGYLQPRTFLLKYNENGTITDAVDCALDPLSETKCTLKSFTVEKGIYQTSNFRVQPTESIVRFPNITNLCPFGEVFNATRFASVYAWNRKRISNCVADYSVLYNSASFSTFKCYGVSPTKLNDLCFTNVYADSFVIRGDEVRQIAPGQTGKIADYNYKLPDDFTGCVIAWNSNNLDSKVGGNYNYRYRLFRKSNLKPFERDISTEIYQAGSKPCNGVEGFNCYFPLQSYGFQPTNGVGYQPYRVVVLSFELLHAPATVCGPKKSTNLVKNKCVNFNFNGLTGTGVLTESNKKFLPFQQFGRDIADTTDAVRDPQTLEILDITPCSFGGVSVITPGTNTSNQVAVLYQGVNCTEVPVAIHADQLTPTWRVYSTGSNVFQTRAGCLIGAEHVNNSYECDIPIGAGICASYQTQTNSRRRARSVASQSIIAYTMSLGAENSVAYSNNSIAIPTNFTISVTTEILPVSMTKTSVDCTMYICGDSTECSNLLLQYGSFCTQLNRALTGIAVEQDKNTQEVFAQVKQIYKTPPIKDFGGFNFSQILPDPSKPSKRSFIEDLLFNKVTLADAGFIKQYGDCLGDIAARDLICAQKFNGLTVLPPLLTDEMIAQYTSALLAGTITSGWTFGAGAALQIPFAMQMAYRFNGIGVTQNVLYENQKLIANQFNSAIGKIQDSLSSTASALGKLQNVVNQNAQALNTLVKQLSSNFGAISSVLNDILSRLDKVEAEVQIDRLITGRLQSLQTYVTQQLIRAAEIRASANLAATKMSECVLGQSKRVDFCGKGYHLMSFPQSAPHGVVFLHVTYVPAQEKNFTTAPAICHDGKAHFPREGVFVSNGTHWFVTQRNFYEPQIITTDNTFVSGNCDVVIGIVNNTVYDPLQPELDSFKEELDKYFKNHTSPDVDLGDISGINASVVNIQKEIDRLNEVAKNLNESLIDLQELGKYEQYIK

SEQ ID NO: 109 - protein, 1196 aa, synthetic construct
  source 1..1196: note; note (original language) = SARS-CoV-2 Delta spike protein extracellular domain without signal peptide, S1/S2 furin cleavage site 1 mutant (685R→685A); organism (original language) = Synthetic construct
QCVNLRTRTQLPPAYTNSFTRGVYYPDKVFRSSVLHSTQDLFLPFFSNVTWFHAIHVSGTNGTKRFDNPVLPFNDGVYFASTEKSNIIRGWIFGTTLDSKTQSLLIVNNATNVVIKVCEFQFCNDPFLDVYYHKNNKSWMESGVYSSANNCTFEYVSQPFLMDLEGKQGNFKNLREFVFKNIDGYFKIYSKHTPINLVRDLPQGFSALEPLVDLPIGINITRFQTLLALHRSYLTPGDSSSGWTAGAAAYYVGYLQPRTFLLKYNENGTITDAVDCALDPLSETKCTLKSFTVEKGIYQTSNFRVQPTESIVRFPNITNLCPFGEVFNATRFASVYAWNRKRISNCVADYSVLYNSASFSTFKCYGVSPTKLNDLCFTNVYADSFVIRGDEVRQIAPGQTGKIADYNYKLPDDFTGCVIAWNSNNLDSKVGGNYNYRYRLFRKSNLKPFERDISTEIYQAGSKPCNGVEGFNCYFPLQSYGFQPTNGVGYQPYRVVVLSFELLHAPATVCGPKKSTNLVKNKCVNFNFNGLTGTGVLTESNKKFLPFQQFGRDIADTTDAVRDPQTLEILDITPCSFGGVSVITPGTNTSNQVAVLYQGVNCTEVPVAIHADQLTPTWRVYSTGSNVFQTRAGCLIGAEHVNNSYECDIPIGAGICASYQTQTNSRRRAASVASQSIIAYTMSLGAENSVAYSNNSIAIPTNFTISVTTEILPVSMTKTSVDCTMYICGDSTECSNLLLQYGSFCTQLNRALTGIAVEQDKNTQEVFAQVKQIYKTPPIKDFGGFNFSQILPDPSKPSKRSFIEDLLFNKVTLADAGFIKQYGDCLGDIAARDLICAQKFNGLTVLPPLLTDEMIAQYTSALLAGTITSGWTFGAGAALQIPFAMQMAYRFNGIGVTQNVLYENQKLIANQFNSAIGKIQDSLSSTASALGKLQNVVNQNAQALNTLVKQLSSNFGAISSVLNDILSRLDKVEAEVQIDRLITGRLQSLQTYVTQQLIRAAEIRASANLAATKMSECVLGQSKRVDFCGKGYHLMSFPQSAPHGVVFLHVTYVPAQEKNFTTAPAICHDGKAHFPREGVFVSNGTHWFVTQRNFYEPQIITTDNTFVSGNCDVVIGIVNNTVYDPLQPELDSFKEELDKYFKNHTSPDVDLGDISGINASVVNIQKEIDRLNEVAKNLNESLIDLQELGKYEQYIK

SEQ ID NO: 110 - protein, 1196 aa, synthetic construct
  source 1..1196: note; note (original language) = SARS-CoV-2 Delta spike protein extracellular domain without signal peptide, S1/S2 furin cleavage site 1 and proline mutant (685R→685A, 986K/987V→986P/987P); organism (original language) = Synthetic construct
QCVNLRTRTQLPPAYTNSFTRGVYYPDKVFRSSVLHSTQDLFLPFFSNVTWFHAIHVSGTNGTKRFDNPVLPFNDGVYFASTEKSNIIRGWIFGTTLDSKTQSLLIVNNATNVVIKVCEFQFCNDPFLDVYYHKNNKSWMESGVYSSANNCTFEYVSQPFLMDLEGKQGNFKNLREFVFKNIDGYFKIYSKHTPINLVRDLPQGFSALEPLVDLPIGINITRFQTLLALHRSYLTPGDSSSGWTAGAAAYYVGYLQPRTFLLKYNENGTITDAVDCALDPLSETKCTLKSFTVEKGIYQTSNFRVQPTESIVRFPNITNLCPFGEVFNATRFASVYAWNRKRISNCVADYSVLYNSASFSTFKCYGVSPTKLNDLCFTNVYADSFVIRGDEVRQIAPGQTGKIADYNYKLPDDFTGCVIAWNSNNLDSKVGGNYNYRYRLFRKSNLKPFERDISTEIYQAGSKPCNGVEGFNCYFPLQSYGFQPTNGVGYQPYRVVVLSFELLHAPATVCGPKKSTNLVKNKCVNFNFNGLTGTGVLTESNKKFLPFQQFGRDIADTTDAVRDPQTLEILDITPCSFGGVSVITPGTNTSNQVAVLYQGVNCTEVPVAIHADQLTPTWRVYSTGSNVFQTRAGCLIGAEHVNNSYECDIPIGAGICASYQTQTNSRRRAASVASQSIIAYTMSLGAENSVAYSNNSIAIPTNFTISVTTEILPVSMTKTSVDCTMYICGDSTECSNLLLQYGSFCTQLNRALTGIAVEQDKNTQEVFAQVKQIYKTPPIKDFGGFNFSQILPDPSKPSKRSFIEDLLFNKVTLADAGFIKQYGDCLGDIAARDLICAQKFNGLTVLPPLLTDEMIAQYTSALLAGTITSGWTFGAGAALQIPFAMQMAYRFNGIGVTQNVLYENQKLIANQFNSAIGKIQDSLSSTASALGKLQNVVNQNAQALNTLVKQLSSNFGAISSVLNDILSRLDPPEAEVQIDRLITGRLQSLQTYVTQQLIRAAEIRASANLAATKMSECVLGQSKRVDFCGKGYHLMSFPQSAPHGVVFLHVTYVPAQEKNFTTAPAICHDGKAHFPREGVFVSNGTHWFVTQRNFYEPQIITTDNTFVSGNCDVVIGIVNNTVYDPLQPELDSFKEELDKYFKNHTSPDVDLGDISGINASVVNIQKEIDRLNEVAKNLNESLIDLQELGKYEQYIK

SEQ ID NO: 111 - protein, 1196 aa, synthetic construct
  source 1..1196: note; note (original language) = SARS-CoV-2 Delta spike protein extracellular domain without signal peptide, proline mutant (986K/987V→986P/987P); organism (original language) = Synthetic construct
QCVNLRTRTQLPPAYTNSFTRGVYYPDKVFRSSVLHSTQDLFLPFFSNVTWFHAIHVSGTNGTKRFDNPVLPFNDGVYFASTEKSNIIRGWIFGTTLDSKTQSLLIVNNATNVVIKVCEFQFCNDPFLDVYYHKNNKSWMESGVYSSANNCTFEYVSQPFLMDLEGKQGNFKNLREFVFKNIDGYFKIYSKHTPINLVRDLPQGFSALEPLVDLPIGINITRFQTLLALHRSYLTPGDSSSGWTAGAAAYYVGYLQPRTFLLKYNENGTITDAVDCALDPLSETKCTLKSFTVEKGIYQTSNFRVQPTESIVRFPNITNLCPFGEVFNATRFASVYAWNRKRISNCVADYSVLYNSASFSTFKCYGVSPTKLNDLCFTNVYADSFVIRGDEVRQIAPGQTGKIADYNYKLPDDFTGCVIAWNSNNLDSKVGGNYNYRYRLFRKSNLKPFERDISTEIYQAGSKPCNGVEGFNCYFPLQSYGFQPTNGVGYQPYRVVVLSFELLHAPATVCGPKKSTNLVKNKCVNFNFNGLTGTGVLTESNKKFLPFQQFGRDIADTTDAVRDPQTLEILDITPCSFGGVSVITPGTNTSNQVAVLYQGVNCTEVPVAIHADQLTPTWRVYSTGSNVFQTRAGCLIGAEHVNNSYECDIPIGAGICASYQTQTNSRRRARSVASQSIIAYTMSLGAENSVAYSNNSIAIPTNFTISVTTEILPVSMTKTSVDCTMYICGDSTECSNLLLQYGSFCTQLNRALTGIAVEQDKNTQEVFAQVKQIYKTPPIKDFGGFNFSQILPDPSKPSKRSFIEDLLFNKVTLADAGFIKQYGDCLGDIAARDLICAQKFNGLTVLPPLLTDEMIAQYTSALLAGTITSGWTFGAGAALQIPFAMQMAYRFNGIGVTQNVLYENQKLIANQFNSAIGKIQDSLSSTASALGKLQNVVNQNAQALNTLVKQLSSNFGAISSVLNDILSRLDPPEAEVQIDRLITGRLQSLQTYVTQQLIRAAEIRASANLAATKMSECVLGQSKRVDFCGKGYHLMSFPQSAPHGVVFLHVTYVPAQEKNFTTAPAICHDGKAHFPREGVFVSNGTHWFVTQRNFYEPQIITTDNTFVSGNCDVVIGIVNNTVYDPLQPELDSFKEELDKYFKNHTSPDVDLGDISGINASVVNIQKEIDRLNEVAKNLNESLIDLQELGKYEQYIK

SEQ ID NO: 112 - protein, 1507 aa, synthetic construct
  source 1..1507: note; note (original language) = SARS-CoV-2 Delta S-trimer fusion polypeptide without signal peptide; organism (original language) = Synthetic construct
QCVNLRTRTQLPPAYTNSFTRGVYYPDKVFRSSVLHSTQDLFLPFFSNVTWFHAIHVSGTNGTKRFDNPVLPFNDGVYFASTEKSNIIRGWIFGTTLDSKTQSLLIVNNATNVVIKVCEFQFCNDPFLDVYYHKNNKSWMESGVYSSANNCTFEYVSQPFLMDLEGKQGNFKNLREFVFKNIDGYFKIYSKHTPINLVRDLPQGFSALEPLVDLPIGINITRFQTLLALHRSYLTPGDSSSGWTAGAAAYYVGYLQPRTFLLKYNENGTITDAVDCALDPLSETKCTLKSFTVEKGIYQTSNFRVQPTESIVRFPNITNLCPFGEVFNATRFASVYAWNRKRISNCVADYSVLYNSASFSTFKCYGVSPTKLNDLCFTNVYADSFVIRGDEVRQIAPGQTGKIADYNYKLPDDFTGCVIAWNSNNLDSKVGGNYNYRYRLFRKSNLKPFERDISTEIYQAGSKPCNGVEGFNCYFPLQSYGFQPTNGVGYQPYRVVVLSFELLHAPATVCGPKKSTNLVKNKCVNFNFNGLTGTGVLTESNKKFLPFQQFGRDIADTTDAVRDPQTLEILDITPCSFGGVSVITPGTNTSNQVAVLYQGVNCTEVPVAIHADQLTPTWRVYSTGSNVFQTRAGCLIGAEHVNNSYECDIPIGAGICASYQTQTNSRRRARSVASQSIIAYTMSLGAENSVAYSNNSIAIPTNFTISVTTEILPVSMTKTSVDCTMYICGDSTECSNLLLQYGSFCTQLNRALTGIAVEQDKNTQEVFAQVKQIYKTPPIKDFGGFNFSQILPDPSKPSKRSFIEDLLFNKVTLADAGFIKQYGDCLGDIAARDLICAQKFNGLTVLPPLLTDEMIAQYTSALLAGTITSGWTFGAGAALQIPFAMQMAYRFNGIGVTQNVLYENQKLIANQFNSAIGKIQDSLSSTASALGKLQNVVNQNAQALNTLVKQLSSNFGAISSVLNDILSRLDKVEAEVQIDRLITGRLQSLQTYVTQQLIRAAEIRASANLAATKMSECVLGQSKRVDFCGKGYHLMSFPQSAPHGVVFLHVTYVPAQEKNFTTAPAICHDGKAHFPREGVFVSNGTHWFVTQRNFYEPQIITTDNTFVSGNCDVVIGIVNNTVYDPLQPELDSFKEELDKYFKNHTSPDVDLGDISGINASVVNIQKEIDRLNEVAKNLNESLIDLQELGKYEQYIKRSNGLPGPIGPPGPRGRTGDAGPVGPPGPPGPPGPPGPPSAGFDFSFLPQPPQEKAHDGGRYYRANDANVVRDRDLEVDTTLKSLSQQIENIRSPEGSRKNPARTCRDLKMCHSDWKSGEYWIDPNQGCNLDAIKVFCNMETGETCVYPTQPSVAQKNWYISKNPKDKRHVWFGESMTDGFQFEYGGQGSDPADVAIQLTFLRLMSTEASQNITYHCKNSVAYMDQQTGNLKKALLLQGSNEIEIRAEGNSRFTYSVTVDGCTSHTGAWGKTVIEYKTTKTSRLPIIDVAPLDVGAPDQEFGFDVGPVCFL

SEQ ID NO: 113 - protein, 1507 aa, synthetic construct
  source 1..1507: note; note (original language) = SARS-CoV-2 Delta S-trimer fusion polypeptide without signal peptide, S1/S2 furin cleavage site 1 mutant (685R→685A); organism (original language) = Synthetic construct
QCVNLRTRTQLPPAYTNSFTRGVYYPDKVFRSSVLHSTQDLFLPFFSNVTWFHAIHVSGTNGTKRFDNPVLPFNDGVYFASTEKSNIIRGWIFGTTLDSKTQSLLIVNNATNVVIKVCEFQFCNDPFLDVYYHKNNKSWMESGVYSSANNCTFEYVSQPFLMDLEGKQGNFKNLREFVFKNIDGYFKIYSKHTPINLVRDLPQGFSALEPLVDLPIGINITRFQTLLALHRSYLTPGDSSSGWTAGAAAYYVGYLQPRTFLLKYNENGTITDAVDCALDPLSETKCTLKSFTVEKGIYQTSNFRVQPTESIVRFPNITNLCPFGEVFNATRFASVYAWNRKRISNCVADYSVLYNSASFSTFKCYGVSPTKLNDLCFTNVYADSFVIRGDEVRQIAPGQTGKIADYNYKLPDDFTGCVIAWNSNNLDSKVGGNYNYRYRLFRKSNLKPFERDISTEIYQAGSKPCNGVEGFNCYFPLQSYGFQPTNGVGYQPYRVVVLSFELLHAPATVCGPKKSTNLVKNKCVNFNFNGLTGTGVLTESNKKFLPFQQFGRDIADTTDAVRDPQTLEILDITPCSFGGVSVITPGTNTSNQVAVLYQGVNCTEVPVAIHADQLTPTWRVYSTGSNVFQTRAGCLIGAEHVNNSYECDIPIGAGICASYQTQTNSRRRAASVASQSIIAYTMSLGAENSVAYSNNSIAIPTNFTISVTTEILPVSMTKTSVDCTMYICGDSTECSNLLLQYGSFCTQLNRALTGIAVEQDKNTQEVFAQVKQIYKTPPIKDFGGFNFSQILPDPSKPSKRSFIEDLLFNKVTLADAGFIKQYGDCLGDIAARDLICAQKFNGLTVLPPLLTDEMIAQYTSALLAGTITSGWTFGAGAALQIPFAMQMAYRFNGIGVTQNVLYENQKLIANQFNSAIGKIQDSLSSTASALGKLQNVVNQNAQALNTLVKQLSSNFGAISSVLNDILSRLDKVEAEVQIDRLITGRLQSLQTYVTQQLIRAAEIRASANLAATKMSECVLGQSKRVDFCGKGYHLMSFPQSAPHGVVFLHVTYVPAQEKNFTTAPAICHDGKAHFPREGVFVSNGTHWFVTQRNFYEPQIITTDNTFVSGNCDVVIGIVNNTVYDPLQPELDSFKEELDKYFKNHTSPDVDLGDISGINASVVNIQKEIDRLNEVAKNLNESLIDLQELGKYEQYIKRSNGLPGPIGPPGPRGRTGDAGPVGPPGPPGPPGPPGPPSAGFDFSFLPQPPQEKAHDGGRYYRANDANVVRDRDLEVDTTLKSLSQQIENIRSPEGSRKNPARTCRDLKMCHSDWKSGEYWIDPNQGCNLDAIKVFCNMETGETCVYPTQPSVAQKNWYISKNPKDKRHVWFGESMTDGFQFEYGGQGSDPADVAIQLTFLRLMSTEASQNITYHCKNSVAYMDQQTGNLKKALLLQGSNEIEIRAEGNSRFTYSVTVDGCTSHTGAWGKTVIEYKTTKTSRLPIIDVAPLDVGAPDQEFGFDVGPVCFL

SEQ ID NO: 114 - protein, 1507 aa, synthetic construct
  source 1..1507: note; note (original language) = SARS-CoV-2 Delta S-trimer fusion polypeptide without signal peptide, S1/S2 furin cleavage site 1 and proline mutant (685R→685A, 986K/987V→986P/987P); organism (original language) = Synthetic construct
QCVNLRTRTQLPPAYTNSFTRGVYYPDKVFRSSVLHSTQDLFLPFFSNVTWFHAIHVSGTNGTKRFDNPVLPFNDGVYFASTEKSNIIRGWIFGTTLDSKTQSLLIVNNATNVVIKVCEFQFCNDPFLDVYYHKNNKSWMESGVYSSANNCTFEYVSQPFLMDLEGKQGNFKNLREFVFKNIDGYFKIYSKHTPINLVRDLPQGFSALEPLVDLPIGINITRFQTLLALHRSYLTPGDSSSGWTAGAAAYYVGYLQPRTFLLKYNENGTITDAVDCALDPLSETKCTLKSFTVEKGIYQTSNFRVQPTESIVRFPNITNLCPFGEVFNATRFASVYAWNRKRISNCVADYSVLYNSASFSTFKCYGVSPTKLNDLCFTNVYADSFVIRGDEVRQIAPGQTGKIADYNYKLPDDFTGCVIAWNSNNLDSKVGGNYNYRYRLFRKSNLKPFERDISTEIYQAGSKPCNGVEGFNCYFPLQSYGFQPTNGVGYQPYRVVVLSFELLHAPATVCGPKKSTNLVKNKCVNFNFNGLTGTGVLTESNKKFLPFQQFGRDIADTTDAVRDPQTLEILDITPCSFGGVSVITPGTNTSNQVAVLYQGVNCTEVPVAIHADQLTPTWRVYSTGSNVFQTRAGCLIGAEHVNNSYECDIPIGAGICASYQTQTNSRRRAASVASQSIIAYTMSLGAENSVAYSNNSIAIPTNFTISVTTEILPVSMTKTSVDCTMYICGDSTECSNLLLQYGSFCTQLNRALTGIAVEQDKNTQEVFAQVKQIYKTPPIKDFGGFNFSQILPDPSKPSKRSFIEDLLFNKVTLADAGFIKQYGDCLGDIAARDLICAQKFNGLTVLPPLLTDEMIAQYTSALLAGTITSGWTFGAGAALQIPFAMQMAYRFNGIGVTQNVLYENQKLIANQFNSAIGKIQDSLSSTASALGKLQNVVNQNAQALNTLVKQLSSNFGAISSVLNDILSRLDPPEAEVQIDRLITGRLQSLQTYVTQQLIRAAEIRASANLAATKMSECVLGQSKRVDFCGKGYHLMSFPQSAPHGVVFLHVTYVPAQEKNFTTAPAICHDGKAHFPREGVFVSNGTHWFVTQRNFYEPQIITTDNTFVSGNCDVVIGIVNNTVYDPLQPELDSFKEELDKYFKNHTSPDVDLGDISGINASVVNIQKEIDRLNEVAKNLNESLIDLQELGKYEQYIKRSNGLPGPIGPPGPRGRTGDAGPVGPPGPPGPPGPPGPPSAGFDFSFLPQPPQEKAHDGGRYYRANDANVVRDRDLEVDTTLKSLSQQIENIRSPEGSRKNPARTCRDLKMCHSDWKSGEYWIDPNQGCNLDAIKVFCNMETGETCVYPTQPSVAQKNWYISKNPKDKRHVWFGESMTDGFQFEYGGQGSDPADVAIQLTFLRLMSTEASQNITYHCKNSVAYMDQQTGNLKKALLLQGSNEIEIRAEGNSRFTYSVTVDGCTSHTGAWGKTVIEYKTTKTSRLPIIDVAPLDVGAPDQEFGFDVGPVCFL

SEQ ID NO: 115 - protein, 1507 aa, synthetic construct
  source 1..1507: note; note (original language) = SARS-CoV-2 Delta S-trimer fusion polypeptide without signal peptide, proline mutant (986K/987V→986P/987P); organism (original language) = Synthetic construct
QCVNLRTRTQLPPAYTNSFTRGVYYPDKVFRSSVLHSTQDLFLPFFSNVTWFHAIHVSGTNGTKRFDNPVLPFNDGVYFASTEKSNIIRGWIFGTTLDSKTQSLLIVNNATNVVIKVCEFQFCNDPFLDVYYHKNNKSWMESGVYSSANNCTFEYVSQPFLMDLEGKQGNFKNLREFVFKNIDGYFKIYSKHTPINLVRDLPQGFSALEPLVDLPIGINITRFQTLLALHRSYLTPGDSSSGWTAGAAAYYVGYLQPRTFLLKYNENGTITDAVDCALDPLSETKCTLKSFTVEKGIYQTSNFRVQPTESIVRFPNITNLCPFGEVFNATRFASVYAWNRKRISNCVADYSVLYNSASFSTFKCYGVSPTKLNDLCFTNVYADSFVIRGDEVRQIAPGQTGKIADYNYKLPDDFTGCVIAWNSNNLDSKVGGNYNYRYRLFRKSNLKPFERDISTEIYQAGSKPCNGVEGFNCYFPLQSYGFQPTNGVGYQPYRVVVLSFELLHAPATVCGPKKSTNLVKNKCVNFNFNGLTGTGVLTESNKKFLPFQQFGRDIADTTDAVRDPQTLEILDITPCSFGGVSVITPGTNTSNQVAVLYQGVNCTEVPVAIHADQLTPTWRVYSTGSNVFQTRAGCLIGAEHVNNSYECDIPIGAGICASYQTQTNSRRRARSVASQSIIAYTMSLGAENSVAYSNNSIAIPTNFTISVTTEILPVSMTKTSVDCTMYICGDSTECSNLLLQYGSFCTQLNRALTGIAVEQDKNTQEVFAQVKQIYKTPPIKDFGGFNFSQILPDPSKPSKRSFIEDLLFNKVTLADAGFIKQYGDCLGDIAARDLICAQKFNGLTVLPPLLTDEMIAQYTSALLAGTITSGWTFGAGAALQIPFAMQMAYRFNGIGVTQNVLYENQKLIANQFNSAIGKIQDSLSSTASALGKLQNVVNQNAQALNTLVKQLSSNFGAISSVLNDILSRLDPPEAEVQIDRLITGRLQSLQTYVTQQLIRAAEIRASANLAATKMSECVLGQSKRVDFCGKGYHLMSFPQSAPHGVVFLHVTYVPAQEKNFTTAPAICHDGKAHFPREGVFVSNGTHWFVTQRNFYEPQIITTDNTFVSGNCDVVIGIVNNTVYDPLQPELDSFKEELDKYFKNHTSPDVDLGDISGINASVVNIQKEIDRLNEVAKNLNESLIDLQELGKYEQYIKRSNGLPGPIGPPGPRGRTGDAGPVGPPGPPGPPGPPGPPSAGFDFSFLPQPPQEKAHDGGRYYRANDANVVRDRDLEVDTTLKSLSQQIENIRSPEGSRKNPARTCRDLKMCHSDWKSGEYWIDPNQGCNLDAIKVFCNMETGETCVYPTQPSVAQKNWYISKNPKDKRHVWFGESMTDGFQFEYGGQGSDPADVAIQLTFLRLMSTEASQNITYHCKNSVAYMDQQTGNLKKALLLQGSNEIEIRAEGNSRFTYSVTVDGCTSHTGAWGKTVIEYKTTKTSRLPIIDVAPLDVGAPDQEFGFDVGPVCFL

SEQ ID NO: 116 - protein, 1520 aa, synthetic construct
  source 1..1520: note; note (original language) = SARS-CoV-2 Delta S-trimer fusion polypeptide with signal peptide; organism (original language) = Synthetic construct
MFVFLVLLPLVSSQCVNLRTRTQLPPAYTNSFTRGVYYPDKVFRSSVLHSTQDLFLPFFSNVTWFHAIHVSGTNGTKRFDNPVLPFNDGVYFASTEKSNIIRGWIFGTTLDSKTQSLLIVNNATNVVIKVCEFQFCNDPFLDVYYHKNNKSWMESGVYSSANNCTFEYVSQPFLMDLEGKQGNFKNLREFVFKNIDGYFKIYSKHTPINLVRDLPQGFSALEPLVDLPIGINITRFQTLLALHRSYLTPGDSSSGWTAGAAAYYVGYLQPRTFLLKYNENGTITDAVDCALDPLSETKCTLKSFTVEKGIYQTSNFRVQPTESIVRFPNITNLCPFGEVFNATRFASVYAWNRKRISNCVADYSVLYNSASFSTFKCYGVSPTKLNDLCFTNVYADSFVIRGDEVRQIAPGQTGKIADYNYKLPDDFTGCVIAWNSNNLDSKVGGNYNYRYRLFRKSNLKPFERDISTEIYQAGSKPCNGVEGFNCYFPLQSYGFQPTNGVGYQPYRVVVLSFELLHAPATVCGPKKSTNLVKNKCVNFNFNGLTGTGVLTESNKKFLPFQQFGRDIADTTDAVRDPQTLEILDITPCSFGGVSVITPGTNTSNQVAVLYQGVNCTEVPVAIHADQLTPTWRVYSTGSNVFQTRAGCLIGAEHVNNSYECDIPIGAGICASYQTQTNSRRRARSVASQSIIAYTMSLGAENSVAYSNNSIAIPTNFTISVTTEILPVSMTKTSVDCTMYICGDSTECSNLLLQYGSFCTQLNRALTGIAVEQDKNTQEVFAQVKQIYKTPPIKDFGGFNFSQILPDPSKPSKRSFIEDLLFNKVTLADAGFIKQYGDCLGDIAARDLICAQKFNGLTVLPPLLTDEMIAQYTSALLAGTITSGWTFGAGAALQIPFAMQMAYRFNGIGVTQNVLYENQKLIANQFNSAIGKIQDSLSSTASALGKLQNVVNQNAQALNTLVKQLSSNFGAISSVLNDILSRLDKVEAEVQIDRLITGRLQSLQTYVTQQLIRAAEIRASANLAATKMSECVLGQSKRVDFCGKGYHLMSFPQSAPHGVVFLHVTYVPAQEKNFTTAPAICHDGKAHFPREGVFVSNGTHWFVTQRNFYEPQIITTDNTFVSGNCDVVIGIVNNTVYDPLQPELDSFKEELDKYFKNHTSPDVDLGDISGINASVVNIQKEIDRLNEVAKNLNESLIDLQELGKYEQYIKRSNGLPGPIGPPGPRGRTGDAGPVGPPGPPGPPGPPGPPSAGFDFSFLPQPPQEKAHDGGRYYRANDANVVRDRDLEVDTTLKSLSQQIENIRSPEGSRKNPARTCRDLKMCHSDWKSGEYWIDPNQGCNLDAIKVFCNMETGETCVYPTQPSVAQKNWYISKNPKDKRHVWFGESMTDGFQFEYGGQGSDPADVAIQLTFLRLMSTEASQNITYHCKNSVAYMDQQTGNLKKALLLQGSNEIEIRAEGNSRFTYSVTVDGCTSHTGAWGKTVIEYKTTKTSRLPIIDVAPLDVGAPDQEFGFDVGPVCFL

SEQ ID NO: 117 - protein, 1520 aa, synthetic construct
  source 1..1520: note; note (original language) = SARS-CoV-2 Delta S-trimer fusion polypeptide with signal peptide, S1/S2 furin cleavage site 1 mutant (685R→685A); organism (original language) = Synthetic construct
MFVFLVLLPLVSSQCVNLRTRTQLPPAYTNSFTRGVYYPDKVFRSSVLHSTQDLFLPFFSNVTWFHAIHVSGTNGTKRFDNPVLPFNDGVYFASTEKSNIIRGWIFGTTLDSKTQSLLIVNNATNVVIKVCEFQFCNDPFLDVYYHKNNKSWMESGVYSSANNCTFEYVSQPFLMDLEGKQGNFKNLREFVFKNIDGYFKIYSKHTPINLVRDLPQGFSALEPLVDLPIGINITRFQTLLALHRSYLTPGDSSSGWTAGAAAYYVGYLQPRTFLLKYNENGTITDAVDCALDPLSETKCTLKSFTVEKGIYQTSNFRVQPTESIVRFPNITNLCPFGEVFNATRFASVYAWNRKRISNCVADYSVLYNSASFSTFKCYGVSPTKLNDLCFTNVYADSFVIRGDEVRQIAPGQTGKIADYNYKLPDDFTGCVIAWNSNNLDSKVGGNYNYRYRLFRKSNLKPFERDISTEIYQAGSKPCNGVEGFNCYFPLQSYGFQPTNGVGYQPYRVVVLSFELLHAPATVCGPKKSTNLVKNKCVNFNFNGLTGTGVLTESNKKFLPFQQFGRDIADTTDAVRDPQTLEILDITPCSFGGVSVITPGTNTSNQVAVLYQGVNCTEVPVAIHADQLTPTWRVYSTGSNVFQTRAGCLIGAEHVNNSYECDIPIGAGICASYQTQTNSRRRAASVASQSIIAYTMSLGAENSVAYSNNSIAIPTNFTISVTTEILPVSMTKTSVDCTMYICGDSTECSNLLLQYGSFCTQLNRALTGIAVEQDKNTQEVFAQVKQIYKTPPIKDFGGFNFSQILPDPSKPSKRSFIEDLLFNKVTLADAGFIKQYGDCLGDIAARDLICAQKFNGLTVLPPLLTDEMIAQYTSALLAGTITSGWTFGAGAALQIPFAMQMAYRFNGIGVTQNVLYENQKLIANQFNSAIGKIQDSLSSTASALGKLQNVVNQNAQALNTLVKQLSSNFGAISSVLNDILSRLDKVEAEVQIDRLITGRLQSLQTYVTQQLIRAAEIRASANLAATKMSECVLGQSKRVDFCGKGYHLMSFPQSAPHGVVFLHVTYVPAQEKNFTTAPAICHDGKAHFPREGVFVSNGTHWFVTQRNFYEPQIITTDNTFVSGNCDVVIGIVNNTVYDPLQPELDSFKEELDKYFKNHTSPDVDLGDISGINASVVNIQKEIDRLNEVAKNLNESLIDLQELGKYEQYIKRSNGLPGPIGPPGPRGRTGDAGPVGPPGPPGPPGPPGPPSAGFDFSFLPQPPQEKAHDGGRYYRANDANVVRDRDLEVDTTLKSLSQQIENIRSPEGSRKNPARTCRDLKMCHSDWKSGEYWIDPNQGCNLDAIKVFCNMETGETCVYPTQPSVAQKNWYISKNPKDKRHVWFGESMTDGFQFEYGGQGSDPADVAIQLTFLRLMSTEASQNITYHCKNSVAYMDQQTGNLKKALLLQGSNEIEIRAEGNSRFTYSVTVDGCTSHTGAWGKTVIEYKTTKTSRLPIIDVAPLDVGAPDQEFGFDVGPVCFL

SEQ ID NO: 118 - protein, 1520 aa, synthetic construct
  source 1..1520: note; note (original language) = SARS-CoV-2 Delta S-trimer fusion polypeptide with signal peptide, S1/S2 furin cleavage site 1 and proline mutant (685R→685A, 986K/987V→986P/987P); organism (original language) = Synthetic construct
MFVFLVLLPLVSSQCVNLRTRTQLPPAYTNSFTRGVYYPDKVFRSSVLHSTQDLFLPFFSNVTWFHAIHVSGTNGTKRFDNPVLPFNDGVYFASTEKSNIIRGWIFGTTLDSKTQSLLIVNNATNVVIKVCEFQFCNDPFLDVYYHKNNKSWMESGVYSSANNCTFEYVSQPFLMDLEGKQGNFKNLREFVFKNIDGYFKIYSKHTPINLVRDLPQGFSALEPLVDLPIGINITRFQTLLALHRSYLTPGDSSSGWTAGAAAYYVGYLQPRTFLLKYNENGTITDAVDCALDPLSETKCTLKSFTVEKGIYQTSNFRVQPTESIVRFPNITNLCPFGEVFNATRFASVYAWNRKRISNCVADYSVLYNSASFSTFKCYGVSPTKLNDLCFTNVYADSFVIRGDEVRQIAPGQTGKIADYNYKLPDDFTGCVIAWNSNNLDSKVGGNYNYRYRLFRKSNLKPFERDISTEIYQAGSKPCNGVEGFNCYFPLQSYGFQPTNGVGYQPYRVVVLSFELLHAPATVCGPKKSTNLVKNKCVNFNFNGLTGTGVLTESNKKFLPFQQFGRDIADTTDAVRDPQTLEILDITPCSFGGVSVITPGTNTSNQVAVLYQGVNCTEVPVAIHADQLTPTWRVYSTGSNVFQTRAGCLIGAEHVNNSYECDIPIGAGICASYQTQTNSRRRAASVASQSIIAYTMSLGAENSVAYSNNSIAIPTNFTISVTTEILPVSMTKTSVDCTMYICGDSTECSNLLLQYGSFCTQLNRALTGIAVEQDKNTQEVFAQVKQIYKTPPIKDFGGFNFSQILPDPSKPSKRSFIEDLLFNKVTLADAGFIKQYGDCLGDIAARDLICAQKFNGLTVLPPLLTDEMIAQYTSALLAGTITSGWTFGAGAALQIPFAMQMAYRFNGIGVTQNVLYENQKLIANQFNSAIGKIQDSLSSTASALGKLQNVVNQNAQALNTLVKQLSSNFGAISSVLNDILSRLDPPEAEVQIDRLITGRLQSLQTYVTQQLIRAAEIRASANLAATKMSECVLGQSKRVDFCGKGYHLMSFPQSAPHGVVFLHVTYVPAQEKNFTTAPAICHDGKAHFPREGVFVSNGTHWFVTQRNFYEPQIITTDNTFVSGNCDVVIGIVNNTVYDPLQPELDSFKEELDKYFKNHTSPDVDLGDISGINASVVNIQKEIDRLNEVAKNLNESLIDLQELGKYEQYIKRSNGLPGPIGPPGPRGRTGDAGPVGPPGPPGPPGPPGPPSAGFDFSFLPQPPQEKAHDGGRYYRANDANVVRDRDLEVDTTLKSLSQQIENIRSPEGSRKNPARTCRDLKMCHSDWKSGEYWIDPNQGCNLDAIKVFCNMETGETCVYPTQPSVAQKNWYISKNPKDKRHVWFGESMTDGFQFEYGGQGSDPADVAIQLTFLRLMSTEASQNITYHCKNSVAYMDQQTGNLKKALLLQGSNEIEIRAEGNSRFTYSVTVDGCTSHTGAWGKTVIEYKTTKTSRLPIIDVAPLDVGAPDQEFGFDVGPVCFL

SEQ ID NO: 119 - protein, 1520 aa, synthetic construct
  source 1..1520: note; note (original language) = SARS-CoV-2 Delta S-trimer fusion polypeptide with signal peptide, proline mutant (986K/987V→986P/987P); organism (original language) = Synthetic construct
MFVFLVLLPLVSSQCVNLRTRTQLPPAYTNSFTRGVYYPDKVFRSSVLHSTQDLFLPFFSNVTWFHAIHVSGTNGTKRFDNPVLPFNDGVYFASTEKSNIIRGWIFGTTLDSKTQSLLIVNNATNVVIKVCEFQFCNDPFLDVYYHKNNKSWMESGVYSSANNCTFEYVSQPFLMDLEGKQGNFKNLREFVFKNIDGYFKIYSKHTPINLVRDLPQGFSALEPLVDLPIGINITRFQTLLALHRSYLTPGDSSSGWTAGAAAYYVGYLQPRTFLLKYNENGTITDAVDCALDPLSETKCTLKSFTVEKGIYQTSNFRVQPTESIVRFPNITNLCPFGEVFNATRFASVYAWNRKRISNCVADYSVLYNSASFSTFKCYGVSPTKLNDLCFTNVYADSFVIRGDEVRQIAPGQTGKIADYNYKLPDDFTGCVIAWNSNNLDSKVGGNYNYRYRLFRKSNLKPFERDISTEIYQAGSKPCNGVEGFNCYFPLQSYGFQPTNGVGYQPYRVVVLSFELLHAPATVCGPKKSTNLVKNKCVNFNFNGLTGTGVLTESNKKFLPFQQFGRDIADTTDAVRDPQTLEILDITPCSFGGVSVITPGTNTSNQVAVLYQGVNCTEVPVAIHADQLTPTWRVYSTGSNVFQTRAGCLIGAEHVNNSYECDIPIGAGICASYQTQTNSRRRARSVASQSIIAYTMSLGAENSVAYSNNSIAIPTNFTISVTTEILPVSMTKTSVDCTMYICGDSTECSNLLLQYGSFCTQLNRALTGIAVEQDKNTQEVFAQVKQIYKTPPIKDFGGFNFSQILPDPSKPSKRSFIEDLLFNKVTLADAGFIKQYGDCLGDIAARDLICAQKFNGLTVLPPLLTDEMIAQYTSALLAGTITSGWTFGAGAALQIPFAMQMAYRFNGIGVTQNVLYENQKLIANQFNSAIGKIQDSLSSTASALGKLQNVVNQNAQALNTLVKQLSSNFGAISSVLNDILSRLDPPEAEVQIDRLITGRLQSLQTYVTQQLIRAAEIRASANLAATKMSECVLGQSKRVDFCGKGYHLMSFPQSAPHGVVFLHVTYVPAQEKNFTTAPAICHDGKAHFPREGVFVSNGTHWFVTQRNFYEPQIITTDNTFVSGNCDVVIGIVNNTVYDPLQPELDSFKEELDKYFKNHTSPDVDLGDISGINASVVNIQKEIDRLNEVAKNLNESLIDLQELGKYEQYIKRSNGLPGPIGPPGPRGRTGDAGPVGPPGPPGPPGPPGPPSAGFDFSFLPQPPQEKAHDGGRYYRANDANVVRDRDLEVDTTLKSLSQQIENIRSPEGSRKNPARTCRDLKMCHSDWKSGEYWIDPNQGCNLDAIKVFCNMETGETCVYPTQPSVAQKNWYISKNPKDKRHVWFGESMTDGFQFEYGGQGSDPADVAIQLTFLRLMSTEASQNITYHCKNSVAYMDQQTGNLKKALLLQGSNEIEIRAEGNSRFTYSVTVDGCTSHTGAWGKTVIEYKTTKTSRLPIIDVAPLDVGAPDQEFGFDVGPVCFL

SEQ ID NO: 120 - protein, 1504 aa, synthetic construct
  source 1..1504: note; note (original language) = SARS-CoV-2 Omicron (BA.5) S-trimer fusion polypeptide without signal peptide, S1/S2 furin cleavage site 1 and proline mutant (685R→685A, 986K/987V→986P/987P); organism (original language) = Synthetic construct
QCVNLITRTQSYTNSFTRGVYYPDKVFRSSVLHSTQDLFLPFFSNVTWFHAISGTNGTKRFDNPVLPFNDGVYFASTEKSNIIRGWIFGTTLDSKTQSLLIVNNATNVVIKVCEFQFCNDPFLDVYYHKNNKSWMESEFRVYSSANNCTFEYVSQPFLMDLEGKQGNFKNLREFVFKNIDGYFKIYSKHTPINLGRDLPQGFSALEPLVDLPIGINITRFQTLLALHRSYLTPGDSSSGWTAGAAAYYVGYLQPRTFLLKYNENGTITDAVDCALDPLSETKCTLKSFTVEKGIYQTSNFRVQPTESIVRFPNITNLCPFDEVFNATRFASVYAWNRKRISNCVADYSVLYNFAPFFAFKCYGVSPTKLNDLCFTNVYADSFVIRGNEVSQIAPGQTGNIADYNYKLPDDFTGCVIAWNSNKLDSKVGGNYNYRYRLFRKSNLKPFERDISTEIYQAGNKPCNGVAGVNCYFPLQSYGFRPTYGVGHQPYRVVVLSFELLHAPATVCGPKKSTNLVKNKCVNFNFNGLTGTGVLTESNKKFLPFQQFGRDIADTTDAVRDPQTLEILDITPCSFGGVSVITPGTNTSNQVAVLYQGVNCTEVPVAIHADQLTPTWRVYSTGSNVFQTRAGCLIGAEYVNNSYECDIPIGAGICASYQTQTKSHRRAASVASQSIIAYTMSLGAENSVAYSNNSIAIPTNFTISVTTEILPVSMTKTSVDCTMYICGDSTECSNLLLQYGSFCTQLKRALTGIAVEQDKNTQEVFAQVKQIYKTPPIKYFGGFNFSQILPDPSKPSKRSFIEDLLFNKVTLADAGFIKQYGDCLGDIAARDLICAQKFNGLTVLPPLLTDEMIAQYTSALLAGTITSGWTFGAGAALQIPFAMQMAYRFNGIGVTQNVLYENQKLIANQFNSAIGKIQDSLSSTASALGKLQDVVNHNAQALNTLVKQLSSKFGAISSVLNDILSRLDPPEAEVQIDRLITGRLQSLQTYVTQQLIRAAEIRASANLAATKMSECVLGQSKRVDFCGKGYHLMSFPQSAPHGVVFLHVTYVPAQEKNFTTAPAICHDGKAHFPREGVFVSNGTHWFVTQRNFYEPQIITTDNTFVSGNCDVVIGIVNNTVYDPLQPELDSFKEELDKYFKNHTSPDVDLGDISGINASVVNIQKEIDRLNEVAKNLNESLIDLQELGKYEQYIKRSNGLPGPIGPPGPRGRTGDAGPVGPPGPPGPPGPPGPPSAGFDFSFLPQPPQEKAHDGGRYYRANDANVVRDRDLEVDTTLKSLSQQIENIRSPEGSRKNPARTCRDLKMCHSDWKSGEYWIDPNQGCNLDAIKVFCNMETGETCVYPTQPSVAQKNWYISKNPKDKRHVWFGESMTDGFQFEYGGQGSDPADVAIQLTFLRLMSTEASQNITYHCKNSVAYMDQQTGNLKKALLLQGSNEIEIRAEGNSRFTYSVTVDGCTSHTGAWGKTVIEYKTTKTSRLPIIDVAPLDVGAPDQEFGFDVGPVCFL

SEQ ID NO: 121 - protein, 1517 aa, synthetic construct
  source 1..1517: note; note (original language) = SARS-CoV-2 Omicron (BA.5) S-trimer fusion polypeptide with signal peptide, S1/S2 furin cleavage site 1 and proline mutant (685R→685A, 986K/987V→986P/987P); organism (original language) = Synthetic construct
MFVFLVLLPLVSSQCVNLITRTQSYTNSFTRGVYYPDKVFRSSVLHSTQDLFLPFFSNVTWFHAISGTNGTKRFDNPVLPFNDGVYFASTEKSNIIRGWIFGTTLDSKTQSLLIVNNATNVVIKVCEFQFCNDPFLDVYYHKNNKSWMESEFRVYSSANNCTFEYVSQPFLMDLEGKQGNFKNLREFVFKNIDGYFKIYSKHTPINLGRDLPQGFSALEPLVDLPIGINITRFQTLLALHRSYLTPGDSSSGWTAGAAAYYVGYLQPRTFLLKYNENGTITDAVDCALDPLSETKCTLKSFTVEKGIYQTSNFRVQPTESIVRFPNITNLCPFDEVFNATRFASVYAWNRKRISNCVADYSVLYNFAPFFAFKCYGVSPTKLNDLCFTNVYADSFVIRGNEVSQIAPGQTGNIADYNYKLPDDFTGCVIAWNSNKLDSKVGGNYNYRYRLFRKSNLKPFERDISTEIYQAGNKPCNGVAGVNCYFPLQSYGFRPTYGVGHQPYRVVVLSFELLHAPATVCGPKKSTNLVKNKCVNFNFNGLTGTGVLTESNKKFLPFQQFGRDIADTTDAVRDPQTLEILDITPCSFGGVSVITPGTNTSNQVAVLYQGVNCTEVPVAIHADQLTPTWRVYSTGSNVFQTRAGCLIGAEYVNNSYECDIPIGAGICASYQTQTKSHRRAASVASQSIIAYTMSLGAENSVAYSNNSIAIPTNFTISVTTEILPVSMTKTSVDCTMYICGDSTECSNLLLQYGSFCTQLKRALTGIAVEQDKNTQEVFAQVKQIYKTPPIKYFGGFNFSQILPDPSKPSKRSFIEDLLFNKVTLADAGFIKQYGDCLGDIAARDLICAQKFNGLTVLPPLLTDEMIAQYTSALLAGTITSGWTFGAGAALQIPFAMQMAYRFNGIGVTQNVLYENQKLIANQFNSAIGKIQDSLSSTASALGKLQDVVNHNAQALNTLVKQLSSKFGAISSVLNDILSRLDPPEAEVQIDRLITGRLQSLQTYVTQQLIRAAEIRASANLAATKMSECVLGQSKRVDFCGKGYHLMSFPQSAPHGVVFLHVTYVPAQEKNFTTAPAICHDGKAHFPREGVFVSNGTHWFVTQRNFYEPQIITTDNTFVSGNCDVVIGIVNNTVYDPLQPELDSFKEELDKYFKNHTSPDVDLGDISGINASVVNIQKEIDRLNEVAKNLNESLIDLQELGKYEQYIKRSNGLPGPIGPPGPRGRTGDAGPVGPPGPPGPPGPPGPPSAGFDFSFLPQPPQEKAHDGGRYYRANDANVVRDRDLEVDTTLKSLSQQIENIRSPEGSRKNPARTCRDLKMCHSDWKSGEYWIDPNQGCNLDAIKVFCNMETGETCVYPTQPSVAQKNWYISKNPKDKRHVWFGESMTDGFQFEYGGQGSDPADVAIQLTFLRLMSTEASQNITYHCKNSVAYMDQQTGNLKKALLLQGSNEIEIRAEGNSRFTYSVTVDGCTSHTGAWGKTVIEYKTTKTSRLPIIDVAPLDVGAPDQEFGFDVGPVCFL

SEQ ID NO: 122 - protein, 1016 aa, synthetic construct
  source 1..1016: note; note (original language) = SARS-CoV-2 Omicron (BA.5) spike protein extracellular domain without signal peptide, S1/S2 furin cleavage site 1 and proline mutant (685R→685A, 986K/987V→986P/987P); organism (original language) = Synthetic construct
NIDGYFKIYSKHTPINLGRDLPQGFSALEPLVDLPIGINITRFQTLLALHRSYLTPGDSSSGWTAGAAAYYVGYLQPRTFLLKYNENGTITDAVDCALDPLSETKCTLKSFTVEKGIYQTSNFRVQPTESIVRFPNITNLCPFDEVFNATRFASVYAWNRKRISNCVADYSVLYNFAPFFAFKCYGVSPTKLNDLCFTNVYADSFVIRGNEVSQIAPGQTGNIADYNYKLPDDFTGCVIAWNSNKLDSKVGGNYNYRYRLFRKSNLKPFERDISTEIYQAGNKPCNGVAGVNCYFPLQSYGFRPTYGVGHQPYRVVVLSFELLHAPATVCGPKKSTNLVKNKCVNFNFNGLTGTGVLTESNKKFLPFQQFGRDIADTTDAVRDPQTLEILDITPCSFGGVSVITPGTNTSNQVAVLYQGVNCTEVPVAIHADQLTPTWRVYSTGSNVFQTRAGCLIGAEYVNNSYECDIPIGAGICASYQTQTKSHRRAASVASQSIIAYTMSLGAENSVAYSNNSIAIPTNFTISVTTEILPVSMTKTSVDCTMYICGDSTECSNLLLQYGSFCTQLKRALTGIAVEQDKNTQEVFAQVKQIYKTPPIKYFGGFNFSQILPDPSKPSKRSFIEDLLFNKVTLADAGFIKQYGDCLGDIAARDLICAQKFNGLTVLPPLLTDEMIAQYTSALLAGTITSGWTFGAGAALQIPFAMQMAYRFNGIGVTQNVLYENQKLIANQFNSAIGKIQDSLSSTASALGKLQDVVNHNAQALNTLVKQLSSKFGAISSVLNDILSRLDPPEAEVQIDRLITGRLQSLQTYVTQQLIRAAEIRASANLAATKMSECVLGQSKRVDFCGKGYHLMSFPQSAPHGVVFLHVTYVPAQEKNFTTAPAICHDGKAHFPREGVFVSNGTHWFVTQRNFYEPQIITTDNTFVSGNCDVVIGIVNNTVYDPLQPELDSFKEELDKYFKNHTSPDVDLGDISGINASVVNIQKEIDRLNEVAKNLNESLIDLQELGKYEQYIK

SEQ ID NO: 123 - protein, 1029 aa, synthetic construct
  source 1..1029: note; note (original language) = SARS-CoV-2 Omicron (BA.5) spike protein extracellular domain with signal peptide, S1/S2 furin cleavage site 1 and proline mutant (685R→685A, 986K/987V→986P/987P); organism (original language) = Synthetic construct
MFVFLVLLPLVSSNIDGYFKIYSKHTPINLGRDLPQGFSALEPLVDLPIGINITRFQTLLALHRSYLTPGDSSSGWTAGAAAYYVGYLQPRTFLLKYNENGTITDAVDCALDPLSETKCTLKSFTVEKGIYQTSNFRVQPTESIVRFPNITNLCPFDEVFNATRFASVYAWNRKRISNCVADYSVLYNFAPFFAFKCYGVSPTKLNDLCFTNVYADSFVIRGNEVSQIAPGQTGNIADYNYKLPDDFTGCVIAWNSNKLDSKVGGNYNYRYRLFRKSNLKPFERDISTEIYQAGNKPCNGVAGVNCYFPLQSYGFRPTYGVGHQPYRVVVLSFELLHAPATVCGPKKSTNLVKNKCVNFNFNGLTGTGVLTESNKKFLPFQQFGRDIADTTDAVRDPQTLEILDITPCSFGGVSVITPGTNTSNQVAVLYQGVNCTEVPVAIHADQLTPTWRVYSTGSNVFQTRAGCLIGAEYVNNSYECDIPIGAGICASYQTQTKSHRRAASVASQSIIAYTMSLGAENSVAYSNNSIAIPTNFTISVTTEILPVSMTKTSVDCTMYICGDSTECSNLLLQYGSFCTQLKRALTGIAVEQDKNTQEVFAQVKQIYKTPPIKYFGGFNFSQILPDPSKPSKRSFIEDLLFNKVTLADAGFIKQYGDCLGDIAARDLICAQKFNGLTVLPPLLTDEMIAQYTSALLAGTITSGWTFGAGAALQIPFAMQMAYRFNGIGVTQNVLYENQKLIANQFNSAIGKIQDSLSSTASALGKLQDVVNHNAQALNTLVKQLSSKFGAISSVLNDILSRLDPPEAEVQIDRLITGRLQSLQTYVTQQLIRAAEIRASANLAATKMSECVLGQSKRVDFCGKGYHLMSFPQSAPHGVVFLHVTYVPAQEKNFTTAPAICHDGKAHFPREGVFVSNGTHWFVTQRNFYEPQIITTDNTFVSGNCDVVIGIVNNTVYDPLQPELDSFKEELDKYFKNHTSPDVDLGDISGINASVVNIQKEIDRLNEVAKNLNESLIDLQELGKYEQYIK

SEQ ID NO: 124 - protein, 1505 aa, synthetic construct
  source 1..1505: note; note (original language) = SARS-CoV-2 Omicron (XBB.1.5) S-trimer fusion polypeptide without signal peptide, S1/S2 furin cleavage site 1 and proline mutant (685R→685A, 986K/987V→986P/987P); organism (original language) = Synthetic construct
QCVNLITRTQSYTNSFTRGVYYPDKVFRSSVLHSTQDLFLPFFSNVTWFHAIHVSGTNGTKRFDNPALPFNDGVYFASTEKSNIIRGWIFGTTLDSKTQSLLIVNNATNVVIKVCEFQFCNDPFLDVYQKNNKSWMESEFRVYSSANNCTFEYVSQPFLMDLEGKEGNFKNLREFVFKNIDGYFKIYSKHTPINLERDLPQGFSALEPLVDLPIGINITRFQTLLALHRSYLTPVDSSSGWTAGAAAYYVGYLQPRTFLLKYNENGTITDAVDCALDPLSETKCTLKSFTVEKGIYQTSNFRVQPTESIVRFPNITNLCPFHEVFNATTFASVYAWNRKRISNCVADYSVIYNFAPFFAFKCYGVSPTKLNDLCFTNVYADSFVIRGNEVSQIAPGQTGNIADYNYKLPDDFTGCVIAWNSNKLDSKPSGNYNYLYRLFRKSKLKPFERDISTEIYQAGNKPCNGVAGPNCYSPLQSYGFRPTYGVGHQPYRVVVLSFELLHAPATVCGPKKSTNLVKNKCVNFNFNGLTGTGVLTESNKKFLPFQQFGRDIADTTDAVRDPQTLEILDITPCSFGGVSVITPGTNTSNQVAVLYQGVNCTEVPVAIHADQLTPTWRVYSTGSNVFQTRAGCLIGAEYVNNSYECDIPIGAGICASYQTQTKSHRRARSVASQSIIAYTMSLGAENSVAYSNNSIAIPTNFTISVTTEILPVSMTKTSVDCTMYICGDSTECSNLLLQYGSFCTQLKRALTGIAVEQDKNTQEVFAQVKQIYKTPPIKYFGGFNFSQILPDPSKPSKRSFIEDLLFNKVTLADAGFIKQYGDCLGDIAARDLICAQKFNGLTVLPPLLTDEMIAQYTSALLAGTITSGWTFGAGAALQIPFAMQMAYRFNGIGVTQNVLYENQKLIANQFNSAIGKIQDSLSSTASALGKLQDVVNHNAQALNTLVKQLSSKFGAISSVLNDILSRLDKVEAEVQIDRLITGRLQSLQTYVTQQLIRAAEIRASANLAATKMSECVLGQSKRVDFCGKGYHLMSFPQSAPHGVVFLHVTYVPAQEKNFTTAPAICHDGKAHFPREGVFVSNGTHWFVTQRNFYEPQIITTDNTFVSGNCDVVIGIVNNTVYDPLQPELDSFKEELDKYFKNHTSPDVDLGDISGINASVVNIQKEIDRLNEVAKNLNESLIDLQELGKYEQYIKRSNGLPGPIGPPGPRGRTGDAGPVGPPGPPGPPGPPGPPSAGFDFSFLPQPPQEKAHDGGRYYRANDANVVRDRDLEVDTTLKSLSQQIENIRSPEGSRKNPARTCRDLKMCHSDWKSGEYWIDPNQGCNLDAIKVFCNMETGETCVYPTQPSVAQKNWYISKNPKDKRHVWFGESMTDGFQFEYGGQGSDPADVAIQLTFLRLMSTEASQNITYHCKNSVAYMDQQTGNLKKALLLQGSNEIEIRAEGNSRFTYSVTVDGCTSHTGAWGKTVIEYKTTKTSRLPIIDVAPLDVGAPDQEFGFDVGPVCFL

SEQ ID NO: 125 - protein, 1518 aa, synthetic construct
  source 1..1518: note; note (original language) = SARS-CoV-2 Omicron (XBB.1.5) S-trimer fusion polypeptide with signal peptide, S1/S2 furin cleavage site 1 and proline mutant (685R→685A, 986K/987V→986P/987P); organism (original language) = Synthetic construct
MFVFLVLLPLVSSQCVNLITRTQSYTNSFTRGVYYPDKVFRSSVLHSTQDLFLPFFSNVTWFHAIHVSGTNGTKRFDNPALPFNDGVYFASTEKSNIIRGWIFGTTLDSKTQSLLIVNNATNVVIKVCEFQFCNDPFLDVYQKNNKSWMESEFRVYSSANNCTFEYVSQPFLMDLEGKEGNFKNLREFVFKNIDGYFKIYSKHTPINLERDLPQGFSALEPLVDLPIGINITRFQTLLALHRSYLTPVDSSSGWTAGAAAYYVGYLQPRTFLLKYNENGTITDAVDCALDPLSETKCTLKSFTVEKGIYQTSNFRVQPTESIVRFPNITNLCPFHEVFNATTFASVYAWNRKRISNCVADYSVIYNFAPFFAFKCYGVSPTKLNDLCFTNVYADSFVIRGNEVSQIAPGQTGNIADYNYKLPDDFTGCVIAWNSNKLDSKPSGNYNYLYRLFRKSKLKPFERDISTEIYQAGNKPCNGVAGPNCYSPLQSYGFRPTYGVGHQPYRVVVLSFELLHAPATVCGPKKSTNLVKNKCVNFNFNGLTGTGVLTESNKKFLPFQQFGRDIADTTDAVRDPQTLEILDITPCSFGGVSVITPGTNTSNQVAVLYQGVNCTEVPVAIHADQLTPTWRVYSTGSNVFQTRAGCLIGAEYVNNSYECDIPIGAGICASYQTQTKSHRRARSVASQSIIAYTMSLGAENSVAYSNNSIAIPTNFTISVTTEILPVSMTKTSVDCTMYICGDSTECSNLLLQYGSFCTQLKRALTGIAVEQDKNTQEVFAQVKQIYKTPPIKYFGGFNFSQILPDPSKPSKRSFIEDLLFNKVTLADAGFIKQYGDCLGDIAARDLICAQKFNGLTVLPPLLTDEMIAQYTSALLAGTITSGWTFGAGAALQIPFAMQMAYRFNGIGVTQNVLYENQKLIANQFNSAIGKIQDSLSSTASALGKLQDVVNHNAQALNTLVKQLSSKFGAISSVLNDILSRLDKVEAEVQIDRLITGRLQSLQTYVTQQLIRAAEIRASANLAATKMSECVLGQSKRVDFCGKGYHLMSFPQSAPHGVVFLHVTYVPAQEKNFTTAPAICHDGKAHFPREGVFVSNGTHWFVTQRNFYEPQIITTDNTFVSGNCDVVIGIVNNTVYDPLQPELDSFKEELDKYFKNHTSPDVDLGDISGINASVVNIQKEIDRLNEVAKNLNESLIDLQELGKYEQYIKRSNGLPGPIGPPGPRGRTGDAGPVGPPGPPGPPGPPGPPSAGFDFSFLPQPPQEKAHDGGRYYRANDANVVRDRDLEVDTTLKSLSQQIENIRSPEGSRKNPARTCRDLKMCHSDWKSGEYWIDPNQGCNLDAIKVFCNMETGETCVYPTQPSVAQKNWYISKNPKDKRHVWFGESMTDGFQFEYGGQGSDPADVAIQLTFLRLMSTEASQNITYHCKNSVAYMDQQTGNLKKALLLQGSNEIEIRAEGNSRFTYSVTVDGCTSHTGAWGKTVIEYKTTKTSRLPIIDVAPLDVGAPDQEFGFDVGPVCFL

SEQ ID NO: 126 - protein, 1194 aa, synthetic construct
  source 1..1194: note; note (original language) = SARS-CoV-2 Omicron (XBB.1.5) spike protein extracellular domain without signal peptide, S1/S2 furin cleavage site 1 and proline mutant (685R→685A, 986K/987V→986P/987P); organism (original language) = Synthetic construct
QCVNLITRTQSYTNSFTRGVYYPDKVFRSSVLHSTQDLFLPFFSNVTWFHAIHVSGTNGTKRFDNPALPFNDGVYFASTEKSNIIRGWIFGTTLDSKTQSLLIVNNATNVVIKVCEFQFCNDPFLDVYQKNNKSWMESEFRVYSSANNCTFEYVSQPFLMDLEGKEGNFKNLREFVFKNIDGYFKIYSKHTPINLERDLPQGFSALEPLVDLPIGINITRFQTLLALHRSYLTPVDSSSGWTAGAAAYYVGYLQPRTFLLKYNENGTITDAVDCALDPLSETKCTLKSFTVEKGIYQTSNFRVQPTESIVRFPNITNLCPFHEVFNATTFASVYAWNRKRISNCVADYSVIYNFAPFFAFKCYGVSPTKLNDLCFTNVYADSFVIRGNEVSQIAPGQTGNIADYNYKLPDDFTGCVIAWNSNKLDSKPSGNYNYLYRLFRKSKLKPFERDISTEIYQAGNKPCNGVAGPNCYSPLQSYGFRPTYGVGHQPYRVVVLSFELLHAPATVCGPKKSTNLVKNKCVNFNFNGLTGTGVLTESNKKFLPFQQFGRDIADTTDAVRDPQTLEILDITPCSFGGVSVITPGTNTSNQVAVLYQGVNCTEVPVAIHADQLTPTWRVYSTGSNVFQTRAGCLIGAEYVNNSYECDIPIGAGICASYQTQTKSHRRARSVASQSIIAYTMSLGAENSVAYSNNSIAIPTNFTISVTTEILPVSMTKTSVDCTMYICGDSTECSNLLLQYGSFCTQLKRALTGIAVEQDKNTQEVFAQVKQIYKTPPIKYFGGFNFSQILPDPSKPSKRSFIEDLLFNKVTLADAGFIKQYGDCLGDIAARDLICAQKFNGLTVLPPLLTDEMIAQYTSALLAGTITSGWTFGAGAALQIPFAMQMAYRFNGIGVTQNVLYENQKLIANQFNSAIGKIQDSLSSTASALGKLQDVVNHNAQALNTLVKQLSSKFGAISSVLNDILSRLDKVEAEVQIDRLITGRLQSLQTYVTQQLIRAAEIRASANLAATKMSECVLGQSKRVDFCGKGYHLMSFPQSAPHGVVFLHVTYVPAQEKNFTTAPAICHDGKAHFPREGVFVSNGTHWFVTQRNFYEPQIITTDNTFVSGNCDVVIGIVNNTVYDPLQPELDSFKEELDKYFKNHTSPDVDLGDISGINASVVNIQKEIDRLNEVAKNLNESLIDLQELGKYEQYIK

SEQ ID NO: 127 - protein, 1207 aa, synthetic construct
  source 1..1207: note; note (original language) = SARS-CoV-2 Omicron (XBB.1.5) spike protein extracellular domain with signal peptide, S1/S2 furin cleavage site 1 and proline mutant (685R→685A, 986K/987V→986P/987P); organism (original language) = Synthetic construct
MFVFLVLLPLVSSQCVNLITRTQSYTNSFTRGVYYPDKVFRSSVLHSTQDLFLPFFSNVTWFHAIHVSGTNGTKRFDNPALPFNDGVYFASTEKSNIIRGWIFGTTLDSKTQSLLIVNNATNVVIKVCEFQFCNDPFLDVYQKNNKSWMESEFRVYSSANNCTFEYVSQPFLMDLEGKEGNFKNLREFVFKNIDGYFKIYSKHTPINLERDLPQGFSALEPLVDLPIGINITRFQTLLALHRSYLTPVDSSSGWTAGAAAYYVGYLQPRTFLLKYNENGTITDAVDCALDPLSETKCTLKSFTVEKGIYQTSNFRVQPTESIVRFPNITNLCPFHEVFNATTFASVYAWNRKRISNCVADYSVIYNFAPFFAFKCYGVSPTKLNDLCFTNVYADSFVIRGNEVSQIAPGQTGNIADYNYKLPDDFTGCVIAWNSNKLDSKPSGNYNYLYRLFRKSKLKPFERDISTEIYQAGNKPCNGVAGPNCYSPLQSYGFRPTYGVGHQPYRVVVLSFELLHAPATVCGPKKSTNLVKNKCVNFNFNGLTGTGVLTESNKKFLPFQQFGRDIADTTDAVRDPQTLEILDITPCSFGGVSVITPGTNTSNQVAVLYQGVNCTEVPVAIHADQLTPTWRVYSTGSNVFQTRAGCLIGAEYVNNSYECDIPIGAGICASYQTQTKSHRRARSVASQSIIAYTMSLGAENSVAYSNNSIAIPTNFTISVTTEILPVSMTKTSVDCTMYICGDSTECSNLLLQYGSFCTQLKRALTGIAVEQDKNTQEVFAQVKQIYKTPPIKYFGGFNFSQILPDPSKPSKRSFIEDLLFNKVTLADAGFIKQYGDCLGDIAARDLICAQKFNGLTVLPPLLTDEMIAQYTSALLAGTITSGWTFGAGAALQIPFAMQMAYRFNGIGVTQNVLYENQKLIANQFNSAIGKIQDSLSSTASALGKLQDVVNHNAQALNTLVKQLSSKFGAISSVLNDILSRLDKVEAEVQIDRLITGRLQSLQTYVTQQLIRAAEIRASANLAATKMSECVLGQSKRVDFCGKGYHLMSFPQSAPHGVVFLHVTYVPAQEKNFTTAPAICHDGKAHFPREGVFVSNGTHWFVTQRNFYEPQIITTDNTFVSGNCDVVIGIVNNTVYDPLQPELDSFKEELDKYFKNHTSPDVDLGDISGINASVVNIQKEIDRLNEVAKNLNESLIDLQELGKYEQYIK